European Patent Application EP 4 477 230 A2, published December 18, 2024. Title: METHODS AND COMPOSITIONS FOR STABILIZED RECOMBINANT FLAVIVIRUS E PROTEIN DIMERS. Applicant: The University of North Carolina at Chapel Hill. Application EP. The sequence listing filed with the application follows.

SEQUENCE LISTING (192 sequences)

SEQ ID NO: 1 - DNA, 54 bp, synthetic construct
  misc_feature 1..54: note = Human Serum Albumin Signal Sequence
  source 1..54: mol_type = other DNA
atgaagtgggtaacctttatttcccttctttttctctttagctcggcttattcc

SEQ ID NO: 2 - DNA, 18 bp, synthetic construct
  misc_feature 1..18: note = Glycine-Serine Linker
  source 1..18: mol_type = other DNA
ggcagcagcggcggcagc

SEQ ID NO: 3 - DNA, 171 bp, synthetic construct
  misc_feature 1..171: note = MHC I-alpha Cytoplasmic and Transmembrane Domains
  source 1..171: mol_type = other DNA
gtaggaatcattgcgggacttgttctgctcggggccgtaataactggagcggtcgtggcggctgtgatgtggcgacggaaaagcagtgatcggaagggtggttcatatacccaagccgcttctagcgatagcgcacaaggatcagatgtttctcttaccgcatgtaaagta

SEQ ID NO: 4 - DNA, 24 bp, synthetic construct
  misc_feature 1..24: note = His Tag
  source 1..24: mol_type = other DNA
catcaccaccatcatcaccatcat

SEQ ID NO: 5 - DNA, 1182 bp, synthetic construct
  misc_feature 1..1182: note = DENV2 WT sE
  source 1..1182: mol_type = other DNA
atgaggtgtatcggcatgtccaacagggactttgtggagggagtgagcggcggcagctgggtggacattgtgctggagcatggaagctgcgtgaccacgatggcgaaaaacaagcccaccctggacttcgagctcatcaagacagaggctaaacagcccgccaccctcaggaagtactgcatcgaggccaagctgaccaacacaacaaccgagtccagatgccctacacagggcgaacccagcctcaacgaagagcaggacaagaggttcgtgtgcaaacacagcatggtggacaggggctggggcaatggatgcggactcttcggaaaaggcggcatcgtgacctgcgccatgttcaggtgtaaaaagaacatggaaggcaaggtggtgcagcccgaaaatctggagtataccatcgtgattaccccccacagcggagaggagcacgccgtgggcaatgacaccggcaagcacggcaaagagattaagatcaccccccagtcctccattaccgaagctgaactgacaggctacggcaccgtgacaatggagtgtagccccaggaccggactggatttcaacgagatggtcctgctacagatggagaacaaggcctggctcgtgcacaggcaatggtttctggatctgcctctgccttggctgcctggcgccgatacacagggctccaactggatacagaaagagaccctcgtcaccttcaagaatccccatgctaagaagcaggacgtggtggtgctgggcagccaagaaggcgccatgcacacagccctgaccggagctaccgagatccagatgagctccggcaacctgctgttcaccggccatctgaaatgtaggctgaggatggataagctgcaactcaaaggcatgtcctactccatgtgcaccggaaagttcaaggtggtgaaagaaatcgccgaaacacagcacggcaccatcgtgatcagggtgcagtatgagggcgacggctccccctgtaagatccccttcgaaatcatggacctggaaaagaggcacgtgctgggcaggctcatcaccgtgaaccccattgtcacagagaaagactcccccgtgaacatcgaggccgagcctccctttggcgactcctacatcatcattggcgtggagcccggacagctcaagctgaactggttcaagaag

SEQ ID NO: 6 - protein, 394 aa, synthetic construct
  REGION 1..394: note = DENV2 WT sE
MRCIGMSNRDFVEGVSGGSWVDIVLEHGSCVTTMAKNKPTLDFELIKTEAKQPATLRKYCIEAKLTNTTTESRCPTQGEPSLNEEQDKRFVCKHSMVDRGWGNGCGLFGKGGIVTCAMFRCKKNMEGKVVQPENLEYTIVITPHSGEEHAVGNDTGKHGKEIKITPQSSITEAELTGYGTVTMECSPRTGLDFNEMVLLQMENKAWLVHRQWFLDLPLPWLPGADTQGSNWIQKETLVTFKNPHAKKQDVVVLGSQEGAMHTALTGATEIQMSSGNLLFTGHLKCRLRMDKLQLKGMSYSMCTGKFKVVKEIAETQHGTIVIRVQYEGDGSPCKIPFEIMDLEKRHVLGRLITVNPIVTEKDSPVNIEAEPPFGDSYIIIGVEPGQLKLNWFKK

SEQ ID NO: 7 - DNA, 1182 bp, synthetic construct
  misc_feature 1..1182: note = DENV2 HCat1
  source 1..1182: mol_type = other DNA
atgaggtgtatcggcatgtccaacgtggactttgtggagggagtgagcggcggcagctgggtggacattgtgctggagcatggaagctgcgtggtgacgatggcgaaaaacaagcccaccctggacttcgagctcatcaagacagaggctaaacagcccgccaccctcaggaagtactgcatcgaggccaagctgaccaacacaacaaccgagtccagatgccctacacagggcgaacccagcctcaacgaagagcaggacaagaggttcgtgtgcaaacacagcatggtggacaggggctggggcaatggatgcggactcttcggaaaaggcggcatcgtgacctgcgccatgttcaggtgtaaaaagaacatggaaggcaaggtggtgcagcccgaaaatctggagtataccatcgtgattaccccctacagcggagaggagcacgccgtgggcaatgacaccggcaagcacggcaaagagattaagatcaccccccagtcctccattaccgaagctgaactgacaggctacggcaccgtgacaatggagtgtagccccaggaccggactggatttcaacgagatggtcctgctacagatggagaacaaggcctggctcgtgcacaggcaatggtttctggatctgcctctgccttggctgcctggcgccgatacacagggctccaactggatacagaaagagaccctcgtcaccttcaagaatccccatgctaagaagcaggacgtggtggtgctgggcagccaagaaggcgccatgcacacagccctgaccggagctaccgagatccagatgagctccggcaacctgctgttcaccggccatctgaaatgtaggctgaggatggataagctgcaactcaaaggcatgtcctactccatgtgcaccggaaagttcaaggtggtgaaagaaatcgccgaaacacagcacggcaccatcgtgatcagggtgcagtatgagggcgacggctccccctgtaagatccccttcgaaatcatggacctggaaaagaggcacgtgctgggcaggctcatcaccgtgaaccccattgtcacagagaaagactcccccgtgaacatcattgccgagcctccctttggcgactcctacatcatcattggcgtggagcccggacagctcaagctgaactggttcaagaag

SEQ ID NO: 8 - protein, 394 aa, synthetic construct
  REGION 1..394: note = DENV2 HCat1
MRCIGMSNVDFVEGVSGGSWVDIVLEHGSCVVTMAKNKPTLDFELIKTEAKQPATLRKYCIEAKLTNTTTESRCPTQGEPSLNEEQDKRFVCKHSMVDRGWGNGCGLFGKGGIVTCAMFRCKKNMEGKVVQPENLEYTIVITPYSGEEHAVGNDTGKHGKEIKITPQSSITEAELTGYGTVTMECSPRTGLDFNEMVLLQMENKAWLVHRQWFLDLPLPWLPGADTQGSNWIQKETLVTFKNPHAKKQDVVVLGSQEGAMHTALTGATEIQMSSGNLLFTGHLKCRLRMDKLQLKGMSYSMCTGKFKVVKEIAETQHGTIVIRVQYEGDGSPCKIPFEIMDLEKRHVLGRLITVNPIVTEKDSPVNIIAEPPFGDSYIIIGVEPGQLKLNWFKK

SEQ ID NO: 9 - DNA, 1182 bp, synthetic construct
  misc_feature 1..1182: note = DENV2 HCat2
  source 1..1182: mol_type = other DNA
atgatgtgtatcggcatgtccaacagggactttgtggagggagtgagcggcggcagctgggtggacattgtgctggagcatggaagctgcgtgaccacgatggcgaaaaacaagcccaccctggacttcatgctcatcaagacagaggctaaacagcccgccaccctcaggaagtactgcatcgaggccaagctgaccaacacaacaaccgagtccagatgccctacacagggcgaacccagcctcaacgaagagcaggacaagaggttcgtgtgcaaacacagcatggtggacaggggctggggcaatggatgcggactcttcggaaaaggcggcatcgtgacctgcgccatgttcaggtgtaaaaagaacatggaaggcaaggtggtgcagcccgaaaatctggagtataccatcgtgattaccccccacagcggagaggagcacgccgtgggcaatgacaccggcaagcacggcaaagagattaagatcaccccccagtcctccattaccgaagctgaactgacaggctacggcaccgtgacaatggagtgtagccccaggaccggactggatttcaacgagatggtcctgctacagatggagaacaaggcctggctcgtgcacaggcaatggtttctggatctgcctctgccttggctgcctggcgccgatacacagggctccaactggatacagaaagagaccctcgtcaccttcaagaatccccatgctaagaagcaggacgtggtggtgctgggcagccaagaaggcgccatgcacacagccctgaccggagctaccgagatccagatgagctccggcaacctgctgttcaccggccatctgaaatgtaggctgaggatggataagctgcaactcaaaggcatgtcctactccatgtgcaccggaaagttcaaggtggtgaaagaaatcgccgaaacacagcacggcaccatcgtgatcagggtgcagtatgagggcgacggctccccctgtaagatccccttcgaaatcatggacctggaaaagaggcacgtgctgggcaggctcatcaccgtgaaccccattgtcacagagaaagactcccccgtgaacatcgaggccgagcctccctttggcgactcctacatcatcattggcgtggagcccggacagctcaagctgaactggttcaagaag

SEQ ID NO: 10 - protein, 394 aa, synthetic construct
  REGION 1..394: note = DENV2 HCat2
MMCIGMSNRDFVEGVSGGSWVDIVLEHGSCVTTMAKNKPTLDFMLIKTEAKQPATLRKYCIEAKLTNTTTESRCPTQGEPSLNEEQDKRFVCKHSMVDRGWGNGCGLFGKGGIVTCAMFRCKKNMEGKVVQPENLEYTIVITPHSGEEHAVGNDTGKHGKEIKITPQSSITEAELTGYGTVTMECSPRTGLDFNEMVLLQMENKAWLVHRQWFLDLPLPWLPGADTQGSNWIQKETLVTFKNPHAKKQDVVVLGSQEGAMHTALTGATEIQMSSGNLLFTGHLKCRLRMDKLQLKGMSYSMCTGKFKVVKEIAETQHGTIVIRVQYEGDGSPCKIPFEIMDLEKRHVLGRLITVNPIVTEKDSPVNIEAEPPFGDSYIIIGVEPGQLKLNWFKK

SEQ ID NO: 11 - DNA, 1182 bp, synthetic construct
  misc_feature 1..1182: note = DENV2 HCat3
  source 1..1182: mol_type = other DNA
atgaggtgtatcggcatgtccaacagggactttgtggagggagtgagcggcggcagctgggtggacattgtgctggagcccggaagctgcgtgaccacgatggcgaaaaacaagcccaccctggacttcgagctcatcaagatcgaggctaaacagcccgccaccctcaggaagtactgcatcgaggccaagctgaccaacacaacaaccgagtccagatgccctacacagggcgaacccagcctcaacgaagagcaggacaagaggttcgtgtgcaaacacagcatggtggacaggggctggggcaatggatgcggactcttcggaaaaggcggcatcgtgacctgcgccatgttcaggtgtaaaaagaacatggaaggcaaggtggtgcagcccgaaaatctggagtataccatcgtgattaccccccacagcggagaggagcacgccgtgggcaatgacaccggcaagcacggcaaagagattaagatcaccccccagtcctccattaccgaagctgaactgacaggctacggcaccgtgacaatggagtgtagccccaggaccggactggatttcaacgagatggtcctgctacagatggagaacaaggcctggctcgtgcacaggcaatggtttctggatctgcctctgccttggctgcctggcgccgatacacagggctccaactggatacagaaagagaccctcgtcaccttcaagaatccccatgctaagaagcaggacgtggtggtgctgggcagccaagaaggcgccatgcacacagccctgaccggagctaccgagatccagatgagctccggcaacctgctgttcaccggccatctgaaatgtaggctgaggatggataagctgcaactcaaaggcatgtcctactccatgtgcaccggaaagttcaaggtggtgaaagaaatcgccgaaacacagcacggcaccatcgtgatcagggtgcagtatgagggcgacggctccccctgtaagatccccttcgaaatcatggacctggaaaagaggcacgtgctgggcaggctcatcaccgtgaaccccattgtcacagagaaagactcccccgtgaacatcgaggccgagcctccctttggcgactcctacatcatcattggcgtggagcccggacagctcaagctgaactggttcaagaag

SEQ ID NO: 12 - protein, 394 aa, synthetic construct
  REGION 1..394: note = DENV2 HCat3
MRCIGMSNRDFVEGVSGGSWVDIVLEPGSCVTTMAKNKPTLDFELIKIEAKQPATLRKYCIEAKLTNTTTESRCPTQGEPSLNEEQDKRFVCKHSMVDRGWGNGCGLFGKGGIVTCAMFRCKKNMEGKVVQPENLEYTIVITPHSGEEHAVGNDTGKHGKEIKITPQSSITEAELTGYGTVTMECSPRTGLDFNEMVLLQMENKAWLVHRQWFLDLPLPWLPGADTQGSNWIQKETLVTFKNPHAKKQDVVVLGSQEGAMHTALTGATEIQMSSGNLLFTGHLKCRLRMDKLQLKGMSYSMCTGKFKVVKEIAETQHGTIVIRVQYEGDGSPCKIPFEIMDLEKRHVLGRLITVNPIVTEKDSPVNIEAEPPFGDSYIIIGVEPGQLKLNWFKK

SEQ ID NO: 13 - DNA, 1182 bp, synthetic construct
  misc_feature 1..1182: note = DENV2 HCat4
  source 1..1182: mol_type = other DNA
atgatgtgtatcggcatgtccaacagggactttgtggagggagtgagcggcggcagctgggtggacattgtgctggagcatggaagctgcgtgaccacgatggcgaaaaacaagcccaccctggacttcctgctcatcaagacagaggctaaacagcccgccaccctcaggaagtactgcatcgaggccaagctgaccaacacaacaaccgagtccagatgccctacacagggcgaacccagcctcaacgaagagcaggacaagaggttcgtgtgcaaacacagcatggtggacaggggctggggcaatggatgcggactcttcggaaaaggcggcatcgtgacctgcgccatgttcaggtgtaaaaagaacatggaaggcaaggtggtgcagcccgaaaatctggagtataccatcgtgattaccccccacagcggagaggagcacgccgtgggcaatctgaccggcaagcacggcaaagagattaagatcaccccccagtcctccattaccgaagctgaactgacaggctacggcaccgtgacaatggagtgtagccccaggaccggactggatttcaacgagatggtcctgctacagatggagaacaaggcctggctcgtgcacaggcaatggtttctggatctgcctctgccttggctgcctggcgccgatacacagggctccaactggatacagaaagagaccctcgtcaccttcaagaatccccatgctatcaagcaggacgtggtggtgctgggcagccaagaaggcgccatgcacacagccctgaccggagctaccgagatccagatgagctccggcaacctgctgttcaccggccatctgaaatgtaggctgaggatggataagctgcaactcaaaggcatgtcctactccatgtgcaccggaaagttcaaggtggtgaaagaaatcgccgaaacacagcacggcaccatcgtgatcagggtgcagtatgagggcgacggctccccctgtaagatccccttcgaaatcatggacctggaaaagaggcacgtgctgggcaggctcatcaccgtgaaccccattgtcacagagaaagactcccccgtgaacatcgaggccgagcctccctttggcgactcctacatcatcattggcgtggagcccggacagctcaagctgaactggttcaagaag

SEQ ID NO: 14 - protein, 394 aa, synthetic construct
  REGION 1..394: note = DENV2 HCat4
MMCIGMSNRDFVEGVSGGSWVDIVLEHGSCVTTMAKNKPTLDFLLIKTEAKQPATLRKYCIEAKLTNTTTESRCPTQGEPSLNEEQDKRFVCKHSMVDRGWGNGCGLFGKGGIVTCAMFRCKKNMEGKVVQPENLEYTIVITPHSGEEHAVGNLTGKHGKEIKITPQSSITEAELTGYGTVTMECSPRTGLDFNEMVLLQMENKAWLVHRQWFLDLPLPWLPGADTQGSNWIQKETLVTFKNPHAIKQDVVVLGSQEGAMHTALTGATEIQMSSGNLLFTGHLKCRLRMDKLQLKGMSYSMCTGKFKVVKEIAETQHGTIVIRVQYEGDGSPCKIPFEIMDLEKRHVLGRLITVNPIVTEKDSPVNIEAEPPFGDSYIIIGVEPGQLKLNWFKK

SEQ ID NO: 15 - DNA, 1182 bp, synthetic construct
  misc_feature 1..1182: note = DENV2 HCat5
  source 1..1182: mol_type = other DNA
atgatgtgtatcggcatgtccaacagggactttgtggagggagtgagcggcggcagctgggtggacattgtgctggagcccggaagctgcgtgaccacgatggcgaaaaacaagcccaccctggacttcatgctcatcaagatcgaggctaaacagcccgccaccctcaggaagtactgcatcgaggccaagctgaccaacacaacaaccgagtccagatgccctacacagggcgaacccagcctcaacgaagagcaggacaagaggttcgtgtgcaaacacagcatggtggacaggggctggggcaatggatgcggactcttcggaaaaggcggcatcgtgacctgcgccatgttcaggtgtaaaaagaacatggaaggcaaggtggtgcagcccgaaaatctggagtataccatcgtgattaccccccacagcggagaggagcacgccgtgggcaatatgaccggcaagcacggcaaagagattaagatcaccccccagtcctccattaccgaagctgaactgacaggctacggcaccgtgacaatggagtgtagccccaggaccggactggatttcaacgagatggtcctgctacagatggagaacaaggcctggctcgtgcacaggcaatggtttctggatctgcctctgccttggctgcctggcgccgatacacagggctccaactggatacagaaagagaccctcgtcaccttcaagaatccccaggcttacaagcaggacgtggtggtgctgggcagccaagaaggcgccatgcacacagccctgaccggagctaccgagatccagatgagctccggcaacctgctgttcaccggccatctgaaatgtaggctgaggatggataagctgcaactcaaaggcatgtcctactccatgtgcaccggaaagttcaaggtggtgaaagaaatcgccgaaacacagcacggcaccatcgtgatcagggtgcagtatgagggcgacggctccccctgtaagatccccttcgaaatcatggacctggaaaagaggcacgtgctgggcaggctcatcaccgtgaaccccattgtcacagagaaagactcccccgtgaacatcgaggccgagcctccctttggcgactcctacatcatcattggcgtggagcccggacagctcaagctgaactggttcaagaag

SEQ ID NO: 16 - protein, 394 aa, synthetic construct
  REGION 1..394: note = DENV2 HCat5
MMCIGMSNRDFVEGVSGGSWVDIVLEPGSCVTTMAKNKPTLDFMLIKIEAKQPATLRKYCIEAKLTNTTTESRCPTQGEPSLNEEQDKRFVCKHSMVDRGWGNGCGLFGKGGIVTCAMFRCKKNMEGKVVQPENLEYTIVITPHSGEEHAVGNMTGKHGKEIKITPQSSITEAELTGYGTVTMECSPRTGLDFNEMVLLQMENKAWLVHRQWFLDLPLPWLPGADTQGSNWIQKETLVTFKNPQAYKQDVVVLGSQEGAMHTALTGATEIQMSSGNLLFTGHLKCRLRMDKLQLKGMSYSMCTGKFKVVKEIAETQHGTIVIRVQYEGDGSPCKIPFEIMDLEKRHVLGRLITVNPIVTEKDSPVNIEAEPPFGDSYIIIGVEPGQLKLNWFKK

SEQ ID NO: 17 - DNA, 1182 bp, synthetic construct
  misc_feature 1..1182: note = DENV2 HCat6
  source 1..1182: mol_type = other DNA
atgaggtgtatcggcatgtccaacagggactttgtggagggagtgagcggcggcagctgggtggacattgtgctggagcatggaagctgcgtgaccacgatggcgaaaaacaagcccaccctggacttcgagctcatcaagacagaggctaaacagcccgccaccctcaggaagtactgcatcgaggccaagctgaccaacacaacaaccgagtccagatgccctacacagggcgaacccagcctcaacgaagagcaggacaagaggttcgtgtgcaaacacagcatggtggacaggggctggggcaatggatgcggactcttcggaaaaggcggcatcgtgacctgcgccatgttcaggtgtaaaaagaacatggaaggcaaggtggtgcagcccgaaaatctggagtataccatcgtgattaccccccacagcggagaggagcacgccgtgggcaatgacaccggcaagcacggcaaagagattaagatcaccccccagtcctccattaccgaagctgaactgacaggctacggcaccgtgacaatggagtgtagccccaggaccggactggatttcaacgagatggtcctgctacagatggagaacttcgcctttctcgtgcacaggcaatggtttctggatctgcctctgccttggctgcctggcgccgatacacagggctccaactggatacagaaagagaccctcgtcaccttcaagaatccccatgctaagaagcaggacgtggtggtgctgggcagccaagaaggcgccatgctgacagccctgaccggagctaccgagatccagatgagctccggcaacctgctgttcaccggccatctgaaatgtaggctgaggatggataagctgcaactcaaaggcatgtcctactccatgtgcaccggaaagttcaaggtggtgaaagaaatcgccgaaacacagcacggcaccatcgtgatcagggtgcagtatgagggcgacggctccccctgtaagatccccttcgaaatcatggacctggaaaagaggcacgtgctgggcaggctcatcaccgtgaaccccattgtcacagagaaagactcccccgtgaacatcgaggccgagcctccctttggcgactcctacatcatcattggcgtggagcccggacagctcaagctgaactggttcaagaag

SEQ ID NO: 18 - protein, 394 aa, synthetic construct
  REGION 1..394: note = DENV2 HCat6
MRCIGMSNRDFVEGVSGGSWVDIVLEHGSCVTTMAKNKPTLDFELIKTEAKQPATLRKYCIEAKLTNTTTESRCPTQGEPSLNEEQDKRFVCKHSMVDRGWGNGCGLFGKGGIVTCAMFRCKKNMEGKVVQPENLEYTIVITPHSGEEHAVGNDTGKHGKEIKITPQSSITEAELTGYGTVTMECSPRTGLDFNEMVLLQMENFAFLVHRQWFLDLPLPWLPGADTQGSNWIQKETLVTFKNPHAKKQDVVVLGSQEGAMLTALTGATEIQMSSGNLLFTGHLKCRLRMDKLQLKGMSYSMCTGKFKVVKEIAETQHGTIVIRVQYEGDGSPCKIPFEIMDLEKRHVLGRLITVNPIVTEKDSPVNIEAEPPFGDSYIIIGVEPGQLKLNWFKK

SEQ ID NO: 19 - DNA, 1182 bp, synthetic construct
  misc_feature 1..1182: note = DENV2 HCat7
  source 1..1182: mol_type = other DNA
atgaggtgtatcggcatgtccaacagggactttgtggagggagtgagcggcggcagctgggtggacattgtgctggagcatggaagctgcgtgaccacgatggcgaaaaacaagcccaccctggacttcgagctcatcaagacagaggctaaacagcccgccaccctcaggaagtactgcatcgaggccaagctgaccaacacaacaaccgagtccagatgccctacacagggcgaacccagcctcaacgaagagcaggacaagaggttcgtgtgcaaacacagcatggtggacaggggctggggcaatggatgcggactcttcggaaaaggcggcatcgtgacctgcgccatgttcaggtgtaaaaagaacatggaaggcaaggtggtgcagcccgaaaatctggagtataccatcgtgattaccccccacagcggagaggagcacgccgtgggcaatgacaccggcaagcacggcaaagagattaagatcaccccccagtcctccattaccgaagctgaactgacaggctacggcaccgtgacaatggagtgtagccccaggaccggactggatttcaacgagatggtcctgctacagatggagaacttcgcctggctcgtgcacaggcaatggtttctggatctgcctctgccttggctgcctggcgccgatacacagggctccaactggatacagaaagagaccctcgtcaccttcaagaatccccatgctaagaagcaggacgtgttcgtgctgggcagccaagaaggcgccatgttcacagccctgaccggagctaccgagatccagatgagctccggcaacctgctgttcaccggccatctgaaatgtaggctgaggatggataagctgcaactcaaaggcatgtcctactccatgtgcaccggaaagttcaaggtggtgaaagaaatcgccgaaacacagcacggcaccatcgtgatcagggtgcagtatgagggcgacggctccccctgtaagatccccttcgaaatcatggacctggaaaagaggcacgtgctgggcaggctcatcaccgtgaaccccattgtcacagagaaagactcccccgtgaacatcgaggccgagcctccctttggcgactcctacatcatcattggcgtggagcccggacagctcaagctgaactggttcaagaag

SEQ ID NO: 20 - protein, 394 aa, synthetic construct
  REGION 1..394: note = DENV2 HCat7
MRCIGMSNRDFVEGVSGGSWVDIVLEHGSCVTTMAKNKPTLDFELIKTEAKQPATLRKYCIEAKLTNTTTESRCPTQGEPSLNEEQDKRFVCKHSMVDRGWGNGCGLFGKGGIVTCAMFRCKKNMEGKVVQPENLEYTIVITPHSGEEHAVGNDTGKHGKEIKITPQSSITEAELTGYGTVTMECSPRTGLDFNEMVLLQMENFAWLVHRQWFLDLPLPWLPGADTQGSNWIQKETLVTFKNPHAKKQDVFVLGSQEGAMFTALTGATEIQMSSGNLLFTGHLKCRLRMDKLQLKGMSYSMCTGKFKVVKEIAETQHGTIVIRVQYEGDGSPCKIPFEIMDLEKRHVLGRLITVNPIVTEKDSPVNIEAEPPFGDSYIIIGVEPGQLKLNWFKK

SEQ ID NO: 21 - DNA, 1182 bp, synthetic construct
  misc_feature 1..1182: note = DENV2 HCat8
  source 1..1182: mol_type = other DNA
atgaggtgtatcggcatgtccaacagggactttgtggagggagtgagcggcggcagctgggtggacattgtgctggagcatggaagctgcgtgaccacgatggcgaaaaacaagcccaccctggacttcgagctcatcaagacagaggctaaacagcccgccaccctcaggaagtactgcatcgaggccaagctgaccaacacaacaaccgagtccagatgccctacacagggcgaacccagcctcaacgaagagcaggacaagaggttcgtgtgcaaacacagcatggtggacaggggctggggcaatggatgcggactcttcggaaaaggcggcatcgtgacctgcgccatgttcaggtgtaaaaagaacatggaaggcaaggtggtgcagcccgaaaatctggagtataccatcgtgattaccccccacagcggagaggagcacgccgtgggcaatgacaccggcaagcacggcaaagagattaagatcaccccccagtcctccattaccgaagctgaactgacaggctacggcaccgtgacaatggagtgtagccccaggaccggactggatttcaacgagatggtcctgctacagatggagaacttcgcctggctcgtgcacaggcaatggtttctggatctgcctctgccttggctgcctggcgccgatacacagggctccaactggatacagaaagagaccctcgtcaccttcaagaatccccatgctaagaagcaggacgtggtggtgctgggcagccaagaaggcgccatgctgacagccctgaccggagctaccgagatccagatgagctccggcaacctgctgttcaccggccatctgaaatgtaggctgaggatggataagctgcaactcaaaggcatgtcctactccatgtgcaccggaaagttcaaggtggtgaaagaaatcgccgaaacacagcacggcaccatcgtgatcagggtgcagtatgagggcgacggctccccctgtaagatccccttcgaaatcatggacctggaaaagaggcacgtgctgggcaggctcatcaccgtgaaccccattgtcacagagaaagactcccccgtgaacatcgaggccgagcctccctttggcgactcctacatcatcattggcgtggagcccggacagctcaagctgaactggttcaagaag

SEQ ID NO: 22 - protein, 394 aa, synthetic construct
  REGION 1..394: note = DENV2 HCat8
MRCIGMSNRDFVEGVSGGSWVDIVLEHGSCVTTMAKNKPTLDFELIKTEAKQPATLRKYCIEAKLTNTTTESRCPTQGEPSLNEEQDKRFVCKHSMVDRGWGNGCGLFGKGGIVTCAMFRCKKNMEGKVVQPENLEYTIVITPHSGEEHAVGNDTGKHGKEIKITPQSSITEAELTGYGTVTMECSPRTGLDFNEMVLLQMENFAWLVHRQWFLDLPLPWLPGADTQGSNWIQKETLVTFKNPHAKKQDVVVLGSQEGAMLTALTGATEIQMSSGNLLFTGHLKCRLRMDKLQLKGMSYSMCTGKFKVVKEIAETQHGTIVIRVQYEGDGSPCKIPFEIMDLEKRHVLGRLITVNPIVTEKDSPVNIEAEPPFGDSYIIIGVEPGQLKLNWFKK

SEQ ID NO: 23 - DNA, 1182 bp, synthetic construct
  misc_feature 1..1182: note = DENV2 IntFc1
  source 1..1182: mol_type = other DNA
atgaggtgtatcggcatgtccaacagggactttgtggagggagtgagcggcggcagctgggtggacattgtgctggagcatggaagctgcgtgaccacgatggcgaaaaacaagcccaccctggacttcgagctcatcaagacagaggctaaacagcccgccaccctcaggaagtactgcatcgaggccaagctgaccaacacaacaaccgagtccagatgccctacacagggcgaacccagcctcaacgaagagcaggacaagaggttcgtgtgcaaacacagcatggtggacaggggctggggcaatggatgcggactcttcggaaaaggcggcatcgtgacctgcgccatgttcaggtgtaaaaagaacatggaaggcaaggtggtgcagcccgaaaatctggagtataccatcgtgattaccccccacagcggagaggagcacgccgtgggcaatgacaccggcaagcacggcaaagagattaagatcaccccccagtcctccattaccgaagctgaactgacaggctacggcaccgtgacaatggagtgtagccccaggaccggactggatttcaacgagatggtcctgctacagatggagaacaaggcctggctcgtgcacaggcaatggtttctggatctgcctctgccttggctgcctggcgccgatacacagggctccaactggatacagaaagagaccctcgtcaccttcaagaatccccatgctaagaagcaggacgtggtggtgctgggcagccaagaaggcgtgatgcaccacgccctgaccggagctaccgagatccagatgagctccggcaacctgctgttcaccggccatctgaaatgtaggctgaggatggataagctgcaactcaaaggcatgtcctactccatgtgcaccggaaagttcaaggtggtgaaagaaatcgccgaaacacagcacggcaccatcgtgatcagggtgcagtatgagggcgacggctccccctgtaagatccccttcgaaatcatggacctggaaaagaggcacgtgctgggcaggctcatcaccgtgaaccccattgtcacagagaaagactcccccgtgaacatcgaggccgagcctccctttggcgactcctacatcatcattggcgtggagcccggacagctcaagctgaactggttcaagaag

SEQ ID NO: 24 - protein, 394 aa, synthetic construct
  REGION 1..394: note = DENV2 IntFc1
MRCIGMSNRDFVEGVSGGSWVDIVLEHGSCVTTMAKNKPTLDFELIKTEAKQPATLRKYCIEAKLTNTTTESRCPTQGEPSLNEEQDKRFVCKHSMVDRGWGNGCGLFGKGGIVTCAMFRCKKNMEGKVVQPENLEYTIVITPHSGEEHAVGNDTGKHGKEIKITPQSSITEAELTGYGTVTMECSPRTGLDFNEMVLLQMENKAWLVHRQWFLDLPLPWLPGADTQGSNWIQKETLVTFKNPHAKKQDVVVLGSQEGVMHHALTGATEIQMSSGNLLFTGHLKCRLRMDKLQLKGMSYSMCTGKFKVVKEIAETQHGTIVIRVQYEGDGSPCKIPFEIMDLEKRHVLGRLITVNPIVTEKDSPVNIEAEPPFGDSYIIIGVEPGQLKLNWFKK

SEQ ID NO: 25 - DNA, 1182 bp, synthetic construct
  misc_feature 1..1182: note = DENV2 IntFc2
  source 1..1182: mol_type = other DNA
atgaggtgtatcggcatgtccaacagggactttgtggagggagtgagcggcggcagctgggtggacattgtgctggagcatggaagctgcgtgaccacgatggcgaaaaacaagcccaccctggacttcgagctcatcaagacagaggctaaacagcccgccaccctcaggaagtactgcatcgaggccaagctgaccaacacaacaaccgagtccagatgccctacacagggcgaacccagcctcaacgaagagcaggacaagaggttcgtgtgcaaacacagcatggtggacaggggctggggcaatggatgcggactcttcggaaaaggcggcatcgtgacctgcgccatgttcaggtgtaaaaagaacatggaaggcaaggtggtgcagcccgaaaatctggagtataccatcgtgattaccccccacagcggagaggagcacgccgtgggcaatgacaccggcaagcacggcaaagagattaagatcaccccccagtcctccattaccgaagctgaactgacaggctacggcaccgtgacaatggagtgtagccccaggaccggactggatttcaacgagatggtcctgctacagatggagaacaaggcctggctcgtgcacaggcaatggtttctggatctgcctctgccttggctgcctggcgccgatacacagggctccaactggatacagaaagagaccctcgtcaccttcaagaatccccatgctaagaagcaggacgtggtggtgctgggcagccaagaaggctggatgcaccgggccctgaccggagctaccgagatccagatgagctccggcaacctgctgttcaccggccatctgaaatgtaggctgaggatggataagctgcaactcaaaggcatgtcctactccatgtgcaccggaaagttcaaggtggtgaaagaaatcgccgaaacacagcacggcaccatcgtgatcagggtgcagtatgagggcgacggctccccctgtaagatccccttcgaaatcatggacctggaaaagaggcacgtgctgggcaggctcatcaccgtgaaccccattgtcacagagaaagactcccccgtgaacatcgaggccgagcctccctttggcgactcctacatcatcattggcgtggagcccggacagctcaagctgaactggttcaagaag

SEQ ID NO: 26 - protein, 394 aa, synthetic construct
  REGION 1..394: note = DENV2 IntFc2
MRCIGMSNRDFVEGVSGGSWVDIVLEHGSCVTTMAKNKPTLDFELIKTEAKQPATLRKYCIEAKLTNTTTESRCPTQGEPSLNEEQDKRFVCKHSMVDRGWGNGCGLFGKGGIVTCAMFRCKKNMEGKVVQPENLEYTIVITPHSGEEHAVGNDTGKHGKEIKITPQSSITEAELTGYGTVTMECSPRTGLDFNEMVLLQMENKAWLVHRQWFLDLPLPWLPGADTQGSNWIQKETLVTFKNPHAKKQDVVVLGSQEGWMHRALTGATEIQMSSGNLLFTGHLKCRLRMDKLQLKGMSYSMCTGKFKVVKEIAETQHGTIVIRVQYEGDGSPCKIPFEIMDLEKRHVLGRLITVNPIVTEKDSPVNIEAEPPFGDSYIIIGVEPGQLKLNWFKK

SEQ ID NO: 27 - DNA, 1182 bp, synthetic construct
  misc_feature 1..1182: note = DENV2 IntFc3
  source 1..1182: mol_type = other DNA
atgaggtgtatcggcatgtccaacagggactttgtggagggagtgagcggcggcagctgggtggacattgtgctggagcatggaagctgcgtgaccacgatggcgaaaaacaagcccaccctggacttcgagctcatcaagacagaggctaaacagcccgccaccctcaggaagtactgcatcgaggccaagctgaccaacacaacaaccgagtccagatgccctacacagggcgaacccagcctcaacgaagagcaggacaagaggttcgtgtgcaaacacagcatggtggacaggggctggggcaatggatgcggactcttcggaaaaggcggcatcgtgacctgcgccatgttcaggtgtaaaaagaacatggaaggcaaggtggtgcagcccgaaaatctggagtataccatcgtgattaccccccacagcggagaggagcacgccgtgggcaatgacaccggcaagcacggcaaagagattaagatcaccccccagtcctccattaccgaagctgaactgacaggctacggcaccgtgacaatggagtgtagccccaggaccggactggatttcaacgagatggtcctgctacagatggagaacaaggcctggctcgtgcacaggcaatggtttctggatctgcctctgccttggctgcctggcgccgatacacagggctccaactggatacagaaagagaccctcgtcaccttcaagaatccccatgctaagaagcaggacgtggtggtgctgggcagccaagaaggcgtgatgcaccggtggctgaccggagctaccgagatccagatgagctccggcaacctgctgttcaccggccatctgaaatgtaggctgaggatggataagctgcaactcaaaggcatgtcctactccatgtgcaccggaaagttcaaggtggtgaaagaaatcgccgaaacacagcacggcaccatcgtgatcagggtgcagtatgagggcgacggctccccctgtaagatccccttcgaaatcatggacctggaaaagaggcacgtgctgggcaggctcatcaccgtgaaccccattgtcacagagaaagactcccccgtgaacatcgaggccgagcctccctttggcgactcctacatcatcattggcgtggagcccggacagctcaagctgaactggttcaagaag

SEQ ID NO: 28 - protein, 394 aa, synthetic construct
  REGION 1..394: note = DENV2 IntFc3
MRCIGMSNRDFVEGVSGGSWVDIVLEHGSCVTTMAKNKPTLDFELIKTEAKQPATLRKYCIEAKLTNTTTESRCPTQGEPSLNEEQDKRFVCKHSMVDRGWGNGCGLFGKGGIVTCAMFRCKKNMEGKVVQPENLEYTIVITPHSGEEHAVGNDTGKHGKEIKITPQSSITEAELTGYGTVTMECSPRTGLDFNEMVLLQMENKAWLVHRQWFLDLPLPWLPGADTQGSNWIQKETLVTFKNPHAKKQDVVVLGSQEGVMHRWLTGATEIQMSSGNLLFTGHLKCRLRMDKLQLKGMSYSMCTGKFKVVKEIAETQHGTIVIRVQYEGDGSPCKIPFEIMDLEKRHVLGRLITVNPIVTEKDSPVNIEAEPPFGDSYIIIGVEPGQLKLNWFKK

SEQ ID NO: 29 - DNA, 1182 bp, synthetic construct
  misc_feature 1..1182: note = DENV2 IntFc4
  source 1..1182: mol_type = other DNA
atgaggtgtatcggcatgtccaacagggactttgtggagggagtgagcggcggcagctgggtggacattgtgctggagcatggaagctgcgtgaccacgatggcgaaaaacaagcccaccctggacttcgagctcatcaagacagaggctaaacagcccgccaccctcaggaagtactgcatcgaggccaagctgaccaacacaacaaccgagtccagatgccctacacagggcgaacccagcctcaacgaagagcaggacaagaggttcgtgtgcaaacacagcatggtggacaggggctggggcaatggatgcggactcttcggaaaaggcggcatcgtgacctgcgccatgttcaggtgtaaaaagaacatggaaggcaaggtggtgcagcccgaaaatctggagtataccatcgtgattaccccccacagcggagaggagcacgccgtgggcaatgacaccggcaagcacggcaaagagattaagatcaccccccagtcctccattaccgaagctgaactgacaggctacggcaccgtgacaatggagtgtagccccaggaccggactggatttcaacgagatggtcctgctacagatggagaacaaggcctggctcgtgcacaggcaatggtttctggatctgcctctgccttggctgcctggcgccgatacacagggctccaactggatacagaaagagaccctcgtcaccttcaagaatccccatgctaagaagcaggacgtggtggtgctgggcagccaagaaggctggatgcactacctcctgaccggagctaccgagatccagatgagctccggcaacctgctgttcaccggccatctgaaatgtaggctgaggatggataagctgcaactcaaaggcatgtcctactccatgtgcaccggaaagttcaaggtggtgaaagaaatcgccgaaacacagcacggcaccatcgtgatcagggtgcagtatgagggcgacggctccccctgtaagatccccttcgaaatcatggacctggaaaagaggcacgtgctgggcaggctcatcaccgtgaaccccattgtcacagagaaagactcccccgtgaacatcgaggccgagcctccctttggcgactcctacatcatcattggcgtggagcccggacagctcaagctgaactggttcaagaag

SEQ ID NO: 30 - protein, 394 aa, synthetic construct
  REGION 1..394: note = DENV2 IntFc4
MRCIGMSNRDFVEGVSGGSWVDIVLEHGSCVTTMAKNKPTLDFELIKTEAKQPATLRKYCIEAKLTNTTTESRCPTQGEPSLNEEQDKRFVCKHSMVDRGWGNGCGLFGKGGIVTCAMFRCKKNMEGKVVQPENLEYTIVITPHSGEEHAVGNDTGKHGKEIKITPQSSITEAELTGYGTVTMECSPRTGLDFNEMVLLQMENKAWLVHRQWFLDLPLPWLPGADTQGSNWIQKETLVTFKNPHAKKQDVVVLGSQEGWMHYLLTGATEIQMSSGNLLFTGHLKCRLRMDKLQLKGMSYSMCTGKFKVVKEIAETQHGTIVIRVQYEGDGSPCKIPFEIMDLEKRHVLGRLITVNPIVTEKDSPVNIEAEPPFGDSYIIIGVEPGQLKLNWFKK

SEQ ID NO: 31 - DNA, 1182 bp, synthetic construct
  misc_feature 1..1182: note = DENV2 IntFc5
  source 1..1182: mol_type = other DNA
atgaggtgtatcggcatgtccaacagggactttgtggagggagtgagcggcggcagctgggtggacattgtgctggagcatggaagctgcgtgaccacgatggcgaaaaacaagcccaccctggacttcgagctcatcaagacagaggctaaacagcccgccaccctcaggaagtactgcatcgaggccaagctgaccaacacaacaaccgagtccagatgccctacacagggcgaacccagcctcaacgaagagcaggacaagaggttcgtgtgcaaacacagcatggtggacaggggctggggcaatggatgcggactcttcggaaaaggcggcatcgtgacctgcgccatgttcaggtgtaaaaagaacatggaaggcaaggtggtgcagcccgaaaatctggagtataccatcgtgattaccccccacagcggagaggagcacgccgtgggcaatgacaccggcaagcacggcaaagagattaagatcaccccccagtcctccattaccgaagctgaactgacaggctacggcaccgtgacaatggagtgtagccccaggaccggactggatttcaacgagatggtcctgctacagatggagaacaaggcctggctcgtgcacaggcaatggtttctggatctgcctctgccttggctgcctggcgccgatacacagggctccaactggatacagaaagagaccctcgtcaccttcaagaatccccatgctaagaagcaggacgtggtggtgctgggcagccaagaaggcgccatgcaccggtggctgaccggagctaccgagatccagatgagctccggcaacctgctgttcaccggccatctgaaatgtaggctgaggatggataagctgcaactcaaaggcatgtcctactccatgtgcaccggaaagttcaaggtggtgaaagaaatcgccgaaacacagcacggcaccatcgtgatcagggtgcagtatgagggcgacggctccccctgtaagatccccttcgaaatcatggacctggaaaagaggcacgtgctgggcaggctcatcaccgtgaaccccattgtcacagagaaagactcccccgtgaacatcgaggccgagcctccctttggcgactcctacatcatcattggcgtggagcccggacagctcaagctgaactggttcaagaag

SEQ ID NO: 32 - protein, 394 aa, synthetic construct
  REGION 1..394: note = DENV2 IntFc5
MRCIGMSNRDFVEGVSGGSWVDIVLEHGSCVTTMAKNKPTLDFELIKTEAKQPATLRKYCIEAKLTNTTTESRCPTQGEPSLNEEQDKRFVCKHSMVDRGWGNGCGLFGKGGIVTCAMFRCKKNMEGKVVQPENLEYTIVITPHSGEEHAVGNDTGKHGKEIKITPQSSITEAELTGYGTVTMECSPRTGLDFNEMVLLQMENKAWLVHRQWFLDLPLPWLPGADTQGSNWIQKETLVTFKNPHAKKQDVVVLGSQEGAMHRWLTGATEIQMSSGNLLFTGHLKCRLRMDKLQLKGMSYSMCTGKFKVVKEIAETQHGTIVIRVQYEGDGSPCKIPFEIMDLEKRHVLGRLITVNPIVTEKDSPVNIEAEPPFGDSYIIIGVEPGQLKLNWFKK

SEQ ID NO: 33 - DNA, 1182 bp, synthetic construct
  misc_feature 1..1182: note = DENV2 IntFc6
  source 1..1182: mol_type = other DNA
atgaggtgtatcggcatgtccctgagggactttgtggagggagtgagcggcggcagctgggtggacattgtgctggagcatggatactgcgtgaccacgatggcgaaaaacaagcccaccctggacttcgagctcatcaagacagaggctaaacagcccgccaccctcaggaagtactgcatcgaggccaagctgaccaacacaacaaccgagtccagatgccctacacagggcgaacccagcctcaacgaagagcaggacaagaggttcgtgtgcaaacacagcatggtggacaggggctggggcaatggatgcggactcttcggaaaaggcggcatcgtgacctgcgccatgttcaggtgtaaaaagaacatggaaggcaaggtggtgcagcccgaaaatctggagtataccatcgtgattaccccccacagcggagaggagcacgccgtgggcaatgacaccggcaagcacggcaaagagattaagatcaccccccagtcctccattaccgaagctgaactgacaggctacggcaccgtgacaatggagtgtagccccaggaccggactggatttcaacgagatggtcctgctacagatggagaacaaggcctggctcgtgcacaggcaatggtttctggatctgcctctgccttggctgcctggcgccgatacacagggctccaactggatacagaaagagaccctcgtcaccttcaagaatcccttcgctaagaagcaggacgtggtggtgctgggcagccaagaaggcgccatgcacacagccctgaccggagctaccgagatccagatgagctccggcaacctgctgttcaccggccatctgaaatgtaggctgaggatggataagctgcaactcaaaggcatgtcctactccatgtgcaccggaaagttcaaggtggtgaaagaaatcgccgaaacacagcacggcaccatcgtgatcagggtgcagtatgagggcgacggctccccctgtaagatccccttcgaaatcatggacctggaaaagaggcacgtgctgggcaggctcatcaccgtgaaccccattgtcacagagaaagactcccccgtgaacatcgaggccgagcctccctttggcgactcctacatcatcattggcgtggagcccggacagctcaagctgaactggttcaagaag

SEQ ID NO: 34 - protein, 394 aa, synthetic construct
  REGION 1..394: note = DENV2 IntFc6
MRCIGMSLRDFVEGVSGGSWVDIVLEHGYCVTTMAKNKPTLDFELIKTEAKQPATLRKYCIEAKLTNTTTESRCPTQGEPSLNEEQDKRFVCKHSMVDRGWGNGCGLFGKGGIVTCAMFRCKKNMEGKVVQPENLEYTIVITPHSGEEHAVGNDTGKHGKEIKITPQSSITEAELTGYGTVTMECSPRTGLDFNEMVLLQMENKAWLVHRQWFLDLPLPWLPGADTQGSNWIQKETLVTFKNPFAKKQDVVVLGSQEGAMHTALTGATEIQMSSGNLLFTGHLKCRLRMDKLQLKGMSYSMCTGKFKVVKEIAETQHGTIVIRVQYEGDGSPCKIPFEIMDLEKRHVLGRLITVNPIVTEKDSPVNIEAEPPFGDSYIIIGVEPGQLKLNWFKK

SEQ ID NO: 35 - DNA, 1182 bp, synthetic construct
  misc_feature 1..1182: note = DENV2 IntFc7
  source 1..1182: mol_type = other DNA
atgaggtgtatcggcatgtccaacagggactttgtggagggagtgagcggcggcagctgggtggacattgtgctggagcatggaagctgcgtgaccacgatggcgaaaaacaagcccaccctggacttcgagctcatcaagacagaggctaaacagcccgccaccctcaggaagtactgcatcgaggccaagctgaccaacacaacaaccgagtccagatgccctacacagggcgaacccagcctcaacgaagagcaggacaagaggttcgtgtgcaaacacagcatggtggacaggggctggggcaatggatgcggactcttcggaaaaggcggcatcgtgacctgcgccatgttcaggtgtaaaaagaacatggaaggcaaggtggtgcagcccgaaaatctggagtataccatcgtgattaccccccacagcggagaggagcacgccgtgggcaatgacaccggcaagcacggcaaagagattaagatcaccccccagtcctccattaccgaagctgaactgacaggctacggcaccgtgacaatggagtgtagccccaggaccggactggatttcaacgagatggtcctgctacagatggagaacaaggcctggctcgtgcacaggcaatggtttctggatctgcctctgccttggctgcctggcgccgatacacagggctccaactggatacagaaagagaccctcgtcaccttcaagaatccccatgctaagaagcaggacgtggtggtgctgggcagccaagaaggcgccatgcaccgggccctgaccggagctaccgagatccagatgagctccggcaacctgctgttcaccggccatctgaaatgtaggctgaggatggataagctgcaactcaaaggcatgtcctactccatgtgcaccggaaagttcaaggtggtgaaagaaatcgccgaaacacagcacggcaccatcgtgatcagggtgcagtatgagggcgacggctccccctgtaagatccccttcgaaatcatggacctggaaaagaggcacgtgctgggcaggctcatcaccgtgaaccccattgtcacagagaaagactcccccgtgaacatcgaggccgagcctccctttggcgactcctacatcatcattggcgtggagcccggacagctcaagctgaactggttcaagaag

SEQ ID NO: 36 - protein, 394 aa, synthetic construct
  REGION 1..394: note = DENV2 IntFc7
MRCIGMSNRDFVEGVSGGSWVDIVLEHGSCVTTMAKNKPTLDFELIKTEAKQPATLRKYCIEAKLTNTTTESRCPTQGEPSLNEEQDKRFVCKHSMVDRGWGNGCGLFGKGGIVTCAMFRCKKNMEGKVVQPENLEYTIVITPHSGEEHAVGNDTGKHGKEIKITPQSSITEAELTGYGTVTMECSPRTGLDFNEMVLLQMENKAWLVHRQWFLDLPLPWLPGADTQGSNWIQKETLVTFKNPHAKKQDVVVLGSQEGAMHRALTGATEIQMSSGNLLFTGHLKCRLRMDKLQLKGMSYSMCTGKFKVVKEIAETQHGTIVIRVQYEGDGSPCKIPFEIMDLEKRHVLGRLITVNPIVTEKDSPVNIEAEPPFGDSYIIIGVEPGQLKLNWFKK

SEQ ID NO: 37 - DNA, 1182 bp, synthetic construct
  misc_feature 1..1182: note = DENV2 IntFc8
  source 1..1182: mol_type = other DNA
atgaggtgtatcggcatgtccaacagggactttgtggagggagtgagcggcggcagctgggtggacattgtgctggagcatggaagctgcgtgaccacgatggcgaaaaacaagcccaccctggacttcgagctcatcaagacagaggctaaacagcccgccaccctcaggaagtactgcatcgaggccaagctgaccaacacaacaaccgagtccagatgccctacacagggcgaacccagcctcaacgaagagcaggacaagaggttcgtgtgcaaacacagcatggtggacaggggctggggcaatggatgcgacctcttcggaaaaggcggcatcgtgacctgcgccatgttcaggtgtaaaaagaacatggaaggcaaggtggtgcagcccgaaaatctggagtataccatcgtgattaccccccacagcggagaggagcacgccgtgggcaatgacaccggcaagcacggcaaagagattaagatcaccccccagtcctccattaccgaagctgaactgacaggctacggcaccgtgacaatggagtgtagccccaggaccggactggatttcaacgagatggtcctgctacagatggagaacaaggcctggctcgtgcacaggcaatggtttctggatctgcctctgccttggctgcctggcgccgatacacagggctccaactggatacagaaagagaccctcgtcaccttcaagaatccccatgctaagaagcaggacgtggtggtgctgggcagccaagaaggcgccatgcacacagccctgaccggagctaccgagatccagatgagctccggcaacctgctgttcaccggccatctgaaatgtaggctgaggatggataagctgcaactcaaaggcatgtcctactccatgtgcaccggaaagttcaaggtggtgaaagaaatcgccgaaacacagcacggcaccatcgtgatcagggtgcagtatgagggcgacggctccccctgtaagatccccttcgaaatcatggacctggaaaagaggcacgtgctgggcaggctcatcaccgtgaaccccattgtcacagagaaagactcccccgtgaacatcgaggccgagcctccctttggcgactcctacatcatcattggcgtggagcccggacagctcaagctgaactggttcaagaag

SEQ ID NO: 38 - protein, 394 aa, synthetic construct
  REGION 1..394: note = DENV2 IntFc8
MRCIGMSNRDFVEGVSGGSWVDIVLEHGSCVTTMAKNKPTLDFELIKTEAKQPATLRKYCIEAKLTNTTTESRCPTQGEPSLNEEQDKRFVCKHSMVDRGWGNGCDLFGKGGIVTCAMFRCKKNMEGKVVQPENLEYTIVITPHSGEEHAVGNDTGKHGKEIKITPQSSITEAELTGYGTVTMECSPRTGLDFNEMVLLQMENKAWLVHRQWFLDLPLPWLPGADTQGSNWIQKETLVTFKNPHAKKQDVVVLGSQEGAMHTALTGATEIQMSSGNLLFTGHLKCRLRMDKLQLKGMSYSMCTGKFKVVKEIAETQHGTIVIRVQYEGDGSPCKIPFEIMDLEKRHVLGRLITVNPIVTEKDSPVNIEAEPPFGDSYIIIGVEPGQLKLNWFKK

SEQ ID NO: 39 - DNA, 1182 bp, synthetic construct
  misc_feature 1..1182: note = DENV2 Mnmer1
  source 1..1182: mol_type = other DNA
atgaggtgtatcggcatgtccaacagggactttgtggagggagtgagcggcggcagctgggtggacattgtgctggagcatggaagctgcgtgaccacgatggcgaaaaacaagcccaccctggacttcgagctcatcaagacagaggctaaacagcccgccaccctcaggaagtactgcatcgaggccaagctgaccaacacaacaaccgagtccagatgccctacacagggcgaacccagcctcaacgaagagcaggacaagaggttcgtgtgcaaacacagcatggtggacaggggctggggcaatggatgcggactcttcggaaaaggcggcatcgtgacctgcgccatgttcaggtgtaaaaagaacatggaaggcaaggtggtgcagcccgaaaatctggagtataccatcgtgattaccccccacagcggagaggagcacgccgtgggcaatgacaccggcaagcacggcaaagagattaagatcaccccccagtcctccattaccgaagctgaactgacaggctacggcaccgtgacaatggagtgtagccccaggaccggactggatttcaacgagatggtcctgctacagatggagaacaaggcctggctcgtgcacaggcaatggtttctggatctgcctctgccttggctgcctggcgccgatacacagggctccaactggatacagaaagagaccctcgtcaccttcaagaatccccatgctaagaagcaggacgtggtggtgctgggcgaacaagaaggcgccatgcacacagccctgaccggagctaccgagatccagatgagctccggcaacctgctgttcaccggccatctgaaatgtaggctgaggatggataagctgcaactcaaaggcatgtcctactccatgtgcaccggaaagttcaaggtggtgaaagaaatcgccgaaacacagcacggcaccatcgtgatcagggtgcagtatgagggcgacggctccccctgtaagatccccttcgaaatcatggacctggaaaagaggcacgtgctgggcaggctcatcaccgtgaaccccattgtcacagagaaagactcccccgtgaacatcgaggccgagcctccctttggcgactcctacatcatcattggcgtggagcccggacagctcaagctgaactggttcaagaag

SEQ ID NO: 40 - protein, 394 aa, synthetic construct
  REGION 1..394: note = DENV2 Mnmer1
MRCIGMSNRDFVEGVSGGSWVDIVLEHGSCVTTMAKNKPTLDFELIKTEAKQPATLRKYCIEAKLTNTTTESRCPTQGEPSLNEEQDKRFVCKHSMVDRGWGNGCGLFGKGGIVTCAMFRCKKNMEGKVVQPENLEYTIVITPHSGEEHAVGNDTGKHGKEIKITPQSSITEAELTGYGTVTMECSPRTGLDFNEMVLLQMENKAWLVHRQWFLDLPLPWLPGADTQGSNWIQKETLVTFKNPHAKKQDVVVLGEQEGAMHTALTGATEIQMSSGNLLFTGHLKCRLRMDKLQLKGMSYSMCTGKFKVVKEIAETQHGTIVIRVQYEGDGSPCKIPFEIMDLEKRHVLGRLITVNPIVTEKDSPVNIEAEPPFGDSYIIIGVEPGQLKLNWFKK

SEQ ID NO: 41 - DNA, 1182 bp, synthetic construct
  misc_feature 1..1182: note = DENV2 Mnmer2
  source 1..1182: mol_type = other DNA
atgaggtgtatcggcatgtccaacagggactttgtggagggagtgagcggcggcagctgggtggacattgtgctggagcatggaagctgcgtgaccacgatggcgaaaaacaagcccaccctggacttcgagctcatcaagacagaggctaaacagcccgccaccctcaggaagtactgcatcgaggccaagctgaccaacacaacaaccgagtccagatgccctacacagggcgaacccagcctcaacgaagagcaggacaagaggttcgtgtgcaaacacagcatggtggacaggggctggggcaatggatgcggactcttcggaaaaggcggcatcgtgacctgcgccatgttcaggtgtaaaaagaacatggaaggcaaggtggtgcagcccgaaaatctggagtataccatcgtgattaccccccacagcggagaggagcacgccgtgggcaatgacaccggcaagcacggcaaagagattaagatcaccccccagtcctccattaccgaagctgaactgacaggctacggcaccgtgacaatggagtgtagccccaggaccggactggatttcaacgagatggtcctgctacagatggagaacaaggcctggctcgtgcacaggcaatggtttctggatctgcctctgccttggctgcctggcgccgatacacagggctccaactggatacagaaagagaccctcgtcaccttcaagaatccccatgctaagaagcaggacgtggtggtgctgggcagccaagaagaggccatgcacacagccctgaccggagctaccgagatccagatgagctccggcaacctgctgttcaccggccatctgaaatgtaggctgaggatggataagctgcaactcaaaggcatgtcctactccatgtgcaccggaaagttcaaggtggtgaaagaaatcgccgaaacacagcacggcaccatcgtgatcagggtgcagtatgagggcgacggctccccctgtaagatccccttcgaaatcatggacctggaaaagaggcacgtgctgggcaggctcatcaccgtgaaccccattgtcacagagaaagactcccccgtgaacatcgaggccgagcctccctttggcgactcctacatcatcattggcgtggagcccggacagctcaagctgaactggttcaagaag

SEQ ID NO: 42 - protein, 394 aa, synthetic construct
  REGION 1..394: note = DENV2 Mnmer2
MRCIGMSNRDFVEGVSGGSWVDIVLEHGSCVTTMAKNKPTLDFELIKTEAKQPATLRKYCIEAKLTNTTTESRCPTQGEPSLNEEQDKRFVCKHSMVDRGWGNGCGLFGKGGIVTCAMFRCKKNMEGKVVQPENLEYTIVITPHSGEEHAVGNDTGKHGKEIKITPQSSITEAELTGYGTVTMECSPRTGLDFNEMVLLQMENKAWLVHRQWFLDLPLPWLPGADTQGSNWIQKETLVTFKNPHAKKQDVVVLGSQEEAMHTALTGATEIQMSSGNLLFTGHLKCRLRMDKLQLKGMSYSMCTGKFKVVKEIAETQHGTIVIRVQYEGDGSPCKIPFEIMDLEKRHVLGRLITVNPIVTEKDSPVNIEAEPPFGDSYIIIGVEPGQLKLNWFKK

SEQ ID NO: 43 - DNA, 1182 bp, synthetic construct
  misc_feature 1..1182: note = DENV2 PM1
  source 1..1182: mol_type = other DNA
atgaggtgtatcggcctgtccaacagggactttgtggagggagtgagcggcggcagctgggtggacattgtgctggagcatggaagctgcgtgaccacgatggcgaaaaacaagcccaccctggacttcgagctcatcaagacagaggctaaacagcccgccaccctcaggaagtactgcatcgaggccaagctgaccaacacaacaaccgagtccagatgccctacacagggcgaacccagcctcaacgaagagcaggacaagaggttcgtgtgcaaacacagcatggtggacaggggctggggcaatggatgcggactcttcggaaaaggcggcatcgtgacctgcgccatgttcaggtgtaaaaagaacatggaaggcaaggtggtgcagcccgaaaatctggagtataccatcgtgattaccccccacagcggagaggagcacgccgtgggcaatgacaccggcaagcacggcaaagagattaagatcaccccccagtcctccattaccgaagctgaactgacaggctacggcaccgtgacaatggagtgtagccccaggaccggactggatttcaacgagatggtcctgctacagatggagaacaaggcctggctcgtgcacaggcaatggtttctggatctgcctctgccttggctgcctggcgccgatacacagggctccaactggatacagaaagagaccctcgtcaccttcaagaatccccatgctaagaagcaggacgtggtggtgctgggcagccaagaaggcgccatgcacacagccctgaccggagctaccgagatccagatgagctccggcaacctgctgttcaccggccatctgaaatgtaggctgaggatggataagctgcaactcaaaggcatgtcctactccatgtgcaccggaaagttcaaggtggtgaaagaaatcgccgaaacaatgcacggcaccatcgtgatcagggtgcagtatgagggcgacggctccccctgtaagatccccttcgaaatcatggacctggaaaagaggcacgtgctgggcaggctcatcaccgtgaaccccattgtcacagagaaagactcccccgtgaacatcgaggccgagcctccctttggcgactcctacatcatcattggcgtggagcccggacagctcaagctgaactggttcaagaag

SEQ ID NO: 44 - protein, 394 aa, synthetic construct
  REGION 1..394: note = DENV2 PM1
MRCIGLSNRDFVEGVSGGSWVDIVLEHGSCVTTMAKNKPTLDFELIKTEAKQPATLRKYCIEAKLTNTTTESRCPTQGEPSLNEEQDKRFVCKHSMVDRGWGNGCGLFGKGGIVTCAMFRCKKNMEGKVVQPENLEYTIVITPHSGEEHAVGNDTGKHGKEIKITPQSSITEAELTGYGTVTMECSPRTGLDFNEMVLLQMENKAWLVHRQWFLDLPLPWLPGADTQGSNWIQKETLVTFKNPHAKKQDVVVLGSQEGAMHTALTGATEIQMSSGNLLFTGHLKCRLRMDKLQLKGMSYSMCTGKFKVVKEIAETMHGTIVIRVQYEGDGSPCKIPFEIMDLEKRHVLGRLITVNPIVTEKDSPVNIEAEPPFGDSYIIIGVEPGQLKLNWFKK

SEQ ID NO: 45 - DNA, 1182 bp, synthetic construct
  misc_feature 1..1182: note = DENV2 PM2
  source 1..1182: mol_type = other DNA
atgaggtgtatcggcatgtccaacagggactttgtggagggagtgagcggcggcagctgggtggacattgtgctggagcatggaagctgcgtgaccacgatggcgaaaaacaagcccaccctggacttcgagctcatcaagacagaggctaaacagcccgccaccctcaggaagtactgcatcgaggccaagctgaccaacacaacaaccgagtccagatgccctacacagggcgaacccagcctcaacgaagagcaggacaagaggttcgtgtgcaaacacagcatggtggacaggggctggggcaatggatgcggactcttcggaaaaggcggcatcgtgacctgcgccatgttcaggtgtaaaaagaacatggaaggcaaggtggtgatccccgaaaatctggagtataccatcgtgattaccccccacagcggagaggagcacgccgtgggcaatgacaccggcaagcacggcaaagagattaagatcaccccccagtcctccattaccgaagctgaactgacaggctacggcaccgtgacaatggagtgtagccccaggaccggactggatttcaacgagatggtcctgctacagatggagaacaaggcctggctcgtgcacaggcaatggtttctggatctgcctctgccttggctgcctggcgccgatacacagggctccaactggatacagaaagagaccctcgtcaccttcaagaatccccatgctaagaagcaggacgtggtggtgctgggcagccaagaaggcgccatgcacacagccctgaccggagctaccgagatccagatgagctccggcaacctgctgttcaccggccatctgaaatgtaggctgaggatggataagctgcaactcaaaggcatgtccctgtccatgtgcaccggaaagttcaaggtggtgaaagaaatcgccgaaacacagcacggcaccatcgtgatcagggtgcagtatgagggcgacggctccccctgtaagatccccttcgaaatcatggacctggaaaagaggcacgtgctgggcaggctcatcaccgtgaaccccattgtcacagagaaagactcccccgtgaacatcgaggccgagcctccctttggcgactcctacatcatcattggcgtggagcccggacagctcaagctgaactggttcaagaag

SEQ ID NO: 46 - protein, 394 aa, synthetic construct
  REGION 1..394: note = DENV2 PM2
MRCIGMSNRDFVEGVSGGSWVDIVLEHGSCVTTMAKNKPTLDFELIKTEAKQPATLRKYCIEAKLTNTTTESRCPTQGEPSLNEEQDKRFVCKHSMVDRGWGNGCGLFGKGGIVTCAMFRCKKNMEGKVVIPENLEYTIVITPHSGEEHAVGNDTGKHGKEIKITPQSSITEAELTGYGTVTMECSPRTGLDFNEMVLLQMENKAWLVHRQWFLDLPLPWLPGADTQGSNWIQKETLVTFKNPHAKKQDVVVLGSQEGAMHTALTGATEIQMSSGNLLFTGHLKCRLRMDKLQLKGMSLSMCTGKFKVVKEIAETQHGTIVIRVQYEGDGSPCKIPFEIMDLEKRHVLGRLITVNPIVTEKDSPVNIEAEPPFGDSYIIIGVEPGQLKLNWFKK

SEQ ID NO: 47 - DNA, 1182 bp, synthetic construct
  misc_feature 1..1182: note = DENV2 PM3
  source 1..1182: mol_type = other DNA
atgaggtgtatcggcatgtccaacagggactttgtggagggagtgagcggcggcagctgggtggacattgtgctggagcatggaagctgcgtgaccacgatgatgaaaaacaagcccaccctggacttcgagctcatcaagacagaggctaaacagcccgccaccctcaggaagtactgcatcgaggccaagctgaccaacacaacaaccgagtccagatgccctacacagggcgaacccagcctcaacgaagagcaggacaagaggttcgtgtgcaaacacagcatggtggacaggggctggggcaatggatgcggactcttcggaaaaggcggcatcgtgacctgcgccatgttcaggtgtaaaaagaacatggaaggcaaggtggtgcagcccgaaaatctggagtataccatcgtgattaccccccacagcggagaggagcacgccgtgggcaatgacaccggcaagcacggcaaagagattaagatcaccccccagtcctccattaccgaagctgaactgacaggctacggcaccgtgacaatggagtgtagccccaggaccggactggatttcaacgagatggtcctgctacagatggagaacaaggcctggctcgtgcacaggcaatggtttctggatctgcctctgccttggctgcctggcgccgatacacagggctccaactggatacagaaagagaccctcgtcaccttcaagaatccccatgctaagaagcaggacgtggtggtgctgggcagccaagaaggcgccatgcacacagccctgaccggagctaccgagatccagatgagctccggcaacctgctgttcaccggccatctgaaatgtaggctgaggtgggataagctgcaactcaaaggcatgtcctactccatgtgcaccggaaagttcaaggtggtgaaagaaatcgccgaaacacagcacggcaccatcgtgatcagggtgcagtatgagggcgacggctccccctgtaagatccccttcgaaatcatggacctggaaaagaggcacgtgctgggcaggctcatcaccgtgaaccccattgtcacagagaaagactcccccgtgaacatcgaggccgagcctccctttggcgactcctacatcatcattggcgtggagcccggacagctcaagctgaactggttcaagaag

SEQ ID NO: 48 - protein, 394 aa, synthetic construct
  REGION 1..394: note = DENV2 PM3
MRCIGMSNRDFVEGVSGGSWVDIVLEHGSCVTTMMKNKPTLDFELIKTEAKQPATLRKYCIEAKLTNTTTESRCPTQGEPSLNEEQDKRFVCKHSMVDRGWGNGCGLFGKGGIVTCAMFRCKKNMEGKVVQPENLEYTIVITPHSGEEHAVGNDTGKHGKEIKITPQSSITEAELTGYGTVTMECSPRTGLDFNEMVLLQMENKAWLVHRQWFLDLPLPWLPGADTQGSNWIQKETLVTFKNPHAKKQDVVVLGSQEGAMHTALTGATEIQMSSGNLLFTGHLKCRLRWDKLQLKGMSYSMCTGKFKVVKEIAETQHGTIVIRVQYEGDGSPCKIPFEIMDLEKRHVLGRLITVNPIVTEKDSPVNIEAEPPFGDSYIIIGVEPGQLKLNWFKK

SEQ ID NO: 49 - DNA, 1182 bp, synthetic construct
  misc_feature 1..1182: note = DENV2 PM4
  source 1..1182: mol_type = other DNA
atgaggtgtatcggcatgtccaacagggactttgtggagggagtgagcggcggcagctgggtggacattgtgctggagcatggaaagtgcgtgaccgtgatgatgaaaaacaagcccaccctggacttcgagctcatcaagacagaggctaaacagcccgccaccctcaggaagtactgcatcgaggccaagctgaccaacacaacaaccgagtccagatgccctacacagggcgaacccagcctcaacgaagagcaggacaagaggttcgtgtgcaaacacagcatggtggacaggggctggggcaatggatgcggactcttcggaaaaggcggcatcgtgacctgcgccatgttcaggtgtaaaaagaacatggaaggcaaggtggtgcagcccgaaaatctggagtataccatcgtgattaccccccacagcggagaggagcacgccgtgggcaatgacaccggcaagcacggcaaagagattaagatcaccccccagtcctccattaccgaagctgaactgacaggctacggcaccgtgacaatggagtgtagccccaggaccggactggatttcaacgagatggtcctgctacagatggagaacaaggcctggctcgtgcacaggcaatggtttctggatctgcctctgccttggctgcctggcgccgatacacagggctccaactggatacagaaagagaccctcgtcaccttcaagaatccccatgctaagaagcaggacgtggtggtgctgggcagccaagaaggcgccatgcacacagccctgaccggagctaccgagatccagatgagctccggcaacctgctgttcaccggccatctgaaatgtaggctgaggatggataagctgcaactcaaaggcatgtcctactccatgtgcaccggaaagttcaaggtggtgaaagaaatcgccgaaacacagcacggcaccatcgtgatcagggtgcagtatgagggcgacggctccccctgtaagatccccttcgaaatcatggacctggaaaagaggcacgtgctgggcaggctcatcaccgtgaaccccattgtcacagagaaagactcccccgtgaacatcgaggccgagcctccctttggcgactcctacatcatcattggcgtggagcccggacagctcaagctgaactggttcaagaag

SEQ ID NO: 50 - protein, 394 aa, synthetic construct
  REGION 1..394: note = DENV2 PM4
MRCIGMSNRDFVEGVSGGSWVDIVLEHGKCVTVMMKNKPTLDFELIKTEAKQPATLRKYCIEAKLTNTTTESRCPTQGEPSLNEEQDKRFVCKHSMVDRGWGNGCGLFGKGGIVTCAMFRCKKNMEGKVVQPENLEYTIVITPHSGEEHAVGNDTGKHGKEIKITPQSSITEAELTGYGTVTMECSPRTGLDFNEMVLLQMENKAWLVHRQWFLDLPLPWLPGADTQGSNWIQKETLVTFKNPHAKKQDVVVLGSQEGAMHTALTGATEIQMSSGNLLFTGHLKCRLRMDKLQLKGMSYSMCTGKFKVVKEIAETQHGTIVIRVQYEGDGSPCKIPFEIMDLEKRHVLGRLITVNPIVTEKDSPVNIEAEPPFGDSYIIIGVEPGQLKLNWFKK

SEQ ID NO: 51 - DNA, 1182 bp, synthetic construct
  misc_feature 1..1182: note = DENV2 PM4.1
  source 1..1182: mol_type = other DNA
atgaggtgtatcggcatgtccaacagggactttgtggagggagtgagcggcggcagctgggtggacattgtgctggagcatggaagctgcgtgaccacgatgatgaaaaacaagcccaccctggacttcgagctcatcaagacagaggctaaacagcccgccaccctcaggaagtactgcatcgaggccaagctgaccaacacaacaaccgagtccagatgccctacacagggcgaacccagcctcaacgaagagcaggacaagaggttcgtgtgcaaacacagcatggtggacaggggctggggcaatggatgcggactcttcggaaaaggcggcatcgtgacctgcgccatgttcaggtgtaaaaagaacatggaaggcaaggtggtgcagcccgaaaatctggagtataccatcgtgattaccccccacagcggagaggagcacgccgtgggcaatgacaccggcaagcacggcaaagagattaagatcaccccccagtcctccattaccgaagctgaactgacaggctacggcaccgtgacaatggagtgtagccccaggaccggactggatttcaacgagatggtcctgctacagatggagaacaaggcctggctcgtgcacaggcaatggtttctggatctgcctctgccttggctgcctggcgccgatacacagggctccaactggatacagaaagagaccctcgtcaccttcaagaatccccatgctaagaagcaggacgtggtggtgctgggcagccaagaaggcgccatgcacacagccctgaccggagctaccgagatccagatgagctccggcaacctgctgttcaccggccatctgaaatgtaggctgaggatggataagctgcaactcaaaggcatgtcctactccatgtgcaccggaaagttcaaggtggtgaaagaaatcgccgaaacacagcacggcaccatcgtgatcagggtgcagtatgagggcgacggctccccctgtaagatccccttcgaaatcatggacctggaaaagaggcacgtgctgggcaggctcatcaccgtgaaccccattgtcacagagaaagactcccccgtgaacatcgaggccgagcctccctttggcgactcctacatcatcattggcgtggagcccggacagctcaagctgaactggttcaagaag

SEQ ID NO: 52 - protein, 394 aa, synthetic construct
  REGION 1..394: note = DENV2 PM4.1
MRCIGMSNRDFVEGVSGGSWVDIVLEHGSCVTTMMKNKPTLDFELIKTEAKQPATLRKYCIEAKLTNTTTESRCPTQGEPSLNEEQDKRFVCKHSMVDRGWGNGCGLFGKGGIVTCAMFRCKKNMEGKVVQPENLEYTIVITPHSGEEHAVGNDTGKHGKEIKITPQSSITEAELTGYGTVTMECSPRTGLDFNEMVLLQMENKAWLVHRQWFLDLPLPWLPGADTQGSNWIQKETLVTFKNPHAKKQDVVVLGSQEGAMHTALTGATEIQMSSGNLLFTGHLKCRLRMDKLQLKGMSYSMCTGKFKVVKEIAETQHGTIVIRVQYEGDGSPCKIPFEIMDLEKRHVLGRLITVNPIVTEKDSPVNIEAEPPFGDSYIIIGVEPGQLKLNWFKK

SEQ ID NO: 53 - DNA, 1182 bp, synthetic construct
  misc_feature 1..1182: note = DENV2 PM4.2
  source 1..1182: mol_type = other DNA
atgaggtgtatcggcatgtccaacagggactttgtggagggagtgagcggcggcagctgggtggacattgtgctggagcatggaagctgcgtgaccgtgatgatgaaaaacaagcccaccctggacttcgagctcatcaagacagaggctaaacagcccgccaccctcaggaagtactgcatcgaggccaagctgaccaacacaacaaccgagtccagatgccctacacagggcgaacccagcctcaacgaagagcaggacaagaggttcgtgtgcaaacacagcatggtggacaggggctggggcaatggatgcggactcttcggaaaaggcggcatcgtgacctgcgccatgttcaggtgtaaaaagaacatggaaggcaaggtggtgcagcccgaaaatctggagtataccatcgtgattaccccccacagcggagaggagcacgccgtgggcaatgacaccggcaagcacggcaaagagattaagatcaccccccagtcctccattaccgaagctgaactgacaggctacggcaccgtgacaatggagtgtagccccaggaccggactggatttcaacgagatggtcctgctacagatggagaacaaggcctggctcgtgcacaggcaatggtttctggatctgcctctgccttggctgcctggcgccgatacacagggctccaactggatacagaaagagaccctcgtcaccttcaagaatccccatgctaagaagcaggacgtggtggtgctgggcagccaagaaggcgccatgcacacagccctgaccggagctaccgagatccagatgagctccggcaacctgctgttcaccggccatctgaaatgtaggctgaggatggataagctgcaactcaaaggcatgtcctactccatgtgcaccggaaagttcaaggtggtgaaagaaatcgccgaaacacagcacggcaccatcgtgatcagggtgcagtatgagggcgacggctccccctgtaagatccccttcgaaatcatggacctggaaaagaggcacgtgctgggcaggctcatcaccgtgaaccccattgtcacagagaaagactcccccgtgaacatcgaggccgagcctccctttggcgactcctacatcatcattggcgtggagcccggacagctcaagctgaactggttcaagaag

SEQ ID NO: 54 - protein, 394 aa, synthetic construct
  REGION 1..394: note = DENV2 PM4.2
MRCIGMSNRDFVEGVSGGSWVDIVLEHGSCVTVMMKNKPTLDFELIKTEAKQPATLRKYCIEAKLTNTTTESRCPTQGEPSLNEEQDKRFVCKHSMVDRGWGNGCGLFGKGGIVTCAMFRCKKNMEGKVVQPENLEYTIVITPHSGEEHAVGNDTGKHGKEIKITPQSSITEAELTGYGTVTMECSPRTGLDFNEMVLLQMENKAWLVHRQWFLDLPLPWLPGADTQGSNWIQKETLVTFKNPHAKKQDVVVLGSQEGAMHTALTGATEIQMSSGNLLFTGHLKCRLRMDKLQLKGMSYSMCTGKFKVVKEIAETQHGTIVIRVQYEGDGSPCKIPFEIMDLEKRHVLGRLITVNPIVTEKDSPVNIEAEPPFGDSYIIIGVEPGQLKLNWFKK

SEQ ID NO: 55 - DNA, 1182 bp, synthetic construct
  misc_feature 1..1182: note = DENV2 PM4.3
  source 1..1182: mol_type = other DNA
atgaggtgtatcggcatgtccaacagggactttgtggagggagtgagcggcggcagctgggtggacattgtgctggagcatggaaagtgcgtgaccacgatggcgaaaaacaagcccaccctggacttcgagctcatcaagacagaggctaaacagcccgccaccctcaggaagtactgcatcgaggccaagctgaccaacacaacaaccgagtccagatgccctacacagggcgaacccagcctcaacgaagagcaggacaagaggttcgtgtgcaaacacagcatggtggacaggggctggggcaatggatgcggactcttcggaaaaggcggcatcgtgacctgcgccatgttcaggtgtaaaaagaacatggaaggcaaggtggtgcagcccgaaaatctggagtataccatcgtgattaccccccacagcggagaggagcacgccgtgggcaatgacaccggcaagcacggcaaagagattaagatcaccccccagtcctccattaccgaagctgaactgacaggctacggcaccgtgacaatggagtgtagccccaggaccggactggatttcaacgagatggtcctgctacagatggagaacaaggcctggctcgtgcacaggcaatggtttctggatctgcctctgccttggctgcctggcgccgatacacagggctccaactggatacagaaagagaccctcgtcaccttcaagaatccccatgctaagaagcaggacgtggtggtgctgggcagccaagaaggcgccatgcacacagccctgaccggagctaccgagatccagatgagctccggcaacctgctgttcaccggccatctgaaatgtaggctgaggatggataagctgcaactcaaaggcatgtcctactccatgtgcaccggaaagttcaaggtggtgaaagaaatcgccgaaacacagcacggcaccatcgtgatcagggtgcagtatgagggcgacggctccccctgtaagatccccttcgaaatcatggacctggaaaagaggcacgtgctgggcaggctcatcaccgtgaaccccattgtcacagagaaagactcccccgtgaacatcgaggccgagcctccctttggcgactcctacatcatcattggcgtggagcccggacagctcaagctgaactggttcaagaag

SEQ ID NO: 56 - protein, 394 aa, synthetic construct
  REGION 1..394: note = DENV2 PM4.3
MRCIGMSNRDFVEGVSGGSWVDIVLEHGKCVTTMAKNKPTLDFELIKTEAKQPATLRKYCIEAKLTNTTTESRCPTQGEPSLNEEQDKRFVCKHSMVDRGWGNGCGLFGKGGIVTCAMFRCKKNMEGKVVQPENLEYTIVITPHSGEEHAVGNDTGKHGKEIKITPQSSITEAELTGYGTVTMECSPRTGLDFNEMVLLQMENKAWLVHRQWFLDLPLPWLPGADTQGSNWIQKETLVTFKNPHAKKQDVVVLGSQEGAMHTALTGATEIQMSSGNLLFTGHLKCRLRMDKLQLKGMSYSMCTGKFKVVKEIAETQHGTIVIRVQYEGDGSPCKIPFEIMDLEKRHVLGRLITVNPIVTEKDSPVNIEAEPPFGDSYIIIGVEPGQLKLNWFKK

SEQ ID NO: 57 - DNA, 1182 bp, synthetic construct
  misc_feature 1..1182: note = DENV2 PM5
  source 1..1182: mol_type = other DNA
atgaggtgtatcggcatgtccaacagggactttgtggagggagtgagcggcggcagctgggtggacattgtgctggagcatggaagctgcgtgaccacgatggcgaaaaacaagcccaccctggacttcgagctcatcaagacagaggctaaacagcccgccaccctcaggaagtactgcatcgaggccaagctgaccaacacaacaaccgagtccagatgccctacacagggcgaacccagcctcaacgaagagcaggacaagaggttcgtgtgcaaacacagcatggtggacaggggctggggcaatggatgcggactcttcggaaaaggcggcatcgtgacctgcgccatgttcaggtgtaaaaagaacatggaaggcaaggtggtgcagcccgaaaatctggagtataccatcgtgattaccccccacagcggagaggagcacgccgtgggcaatgacaccggcaagcacggcaaagagattaagatcaccccccagtcctccattaccgaagctgaactgacaggctacggcaccgtgacaatggagtgtagccccaggaccggactggatttcaacgagatggtcctgctacagatggagaacaaggcctggctcgtggacaggcaatggtttctggatctgcctctgccttggctgcctggcgccgatacacagggctccaactggatacagaaagagaccctcgtcaccttcaagaatccccatgctaagaagcaggacgtggtggtgctgggcagccaagaaggcgccatgcacacagccctgacctgggctaccgagatccagatgagctccggcaacctgctgttcaccggccatctgaaatgtaggctgaggatggataagctgcaactcaaaggcatgtcctactccatgtgcaccggaaagttcaaggtggtgaaagaaatcgccgaaacacagcacggcaccatcgtgatcagggtgcagtatgagggcgacggctccccctgtaagatccccttcgaaatcatggacctggaaaagaggcacgtgctgggcaggctcatcaccgtgaaccccattgtcacagagaaagactcccccgtgaacatcgaggccgagcctccctttggcgactcctacatcatcattggcgtggagcccggacagctcaagctgaactggttcaagaag

SEQ ID NO: 58 - protein, 394 aa, synthetic construct
  REGION 1..394: note = DENV2 PM5
MRCIGMSNRDFVEGVSGGSWVDIVLEHGSCVTTMAKNKPTLDFELIKTEAKQPATLRKYCIEAKLTNTTTESRCPTQGEPSLNEEQDKRFVCKHSMVDRGWGNGCGLFGKGGIVTCAMFRCKKNMEGKVVQPENLEYTIVITPHSGEEHAVGNDTGKHGKEIKITPQSSITEAELTGYGTVTMECSPRTGLDFNEMVLLQMENKAWLVDRQWFLDLPLPWLPGADTQGSNWIQKETLVTFKNPHAKKQDVVVLGSQEGAMHTALTWATEIQMSSGNLLFTGHLKCRLRMDKLQLKGMSYSMCTGKFKVVKEIAETQHGTIVIRVQYEGDGSPCKIPFEIMDLEKRHVLGRLITVNPIVTEKDSPVNIEAEPPFGDSYIIIGVEPGQLKLNWFKK

SEQ ID NO: 59 - DNA, 1182 bp, synthetic construct
  misc_feature 1..1182: note = DENV2 PM6
  source 1..1182: mol_type = other DNA
atgaggtgtatcggcatgtccaacagggactttgtggagggagtgagcggcggcagctgggtggacattgtgctggagcatggaagctgcgtgaccacgatggcgaaaaacaagcccaccctggacttcgagctcatcaagacagaggctaaacagcccgccaccctcaggaagtactgcatcgaggccaagctgaccaacacaacaaccgagtccagatgccctacacagggcgaacccagcctcaacgaagagcaggacaagaggttcgtgtgcaaacacagcatggtggacaggggctggggcaatggatgcggactcttcggaaaaggcggcatcgtgacctgcgccatgttcaggtgtaaaaagaacatggaaggcaaggtggtgcagcccgaaaatctggagtataccatcgtgattaccccccacagcggagaggagcacgccgtgggcaatgacaccggcaagcacggcaaagagattaagatcaccccccagtcctccattaccgaagctgaactgacaggctacggcaccgtgacaatggagtgtagccccaggaccggactggatttcaacgagatggtcctgctacagatggagaacaaggcctggctcgtgcacaggcaatggtttctggatctgcctctgccttggctgcctggcgccgatacacagggctccaactggatacagaaagagaccctcgtcaccttcaagaatccccatgctaagaagcaggacgtggtggtgctgggcagccaagaaggcgccatgcacacagccctgaccggagctaccgagatccagatgagctccggcaacctgctgttcaccggccatctgaaatgtaggctgaggatggataagctgcaactcaaaggcatgtcctactccatgtgcaccggaaagttcaaggtggtgaaagaaatcgccgaaacacagcacggcaccatcgtgatcagggtgcagtatgagggcgacggctccccctgtaagatccccttcgaaatcatggacctggaaaagaggcacgtgctgggcaggctcatcaccgtgaaccccattgtcacagagaaagactcccccgtgaacatcgaggccgagcctccctttggcctgtcctacatcatcattggcgtggagcccggacagctcaagctgcagtggttcaagaag

SEQ ID NO: 60 - protein, 394 aa, synthetic construct
  REGION 1..394: note = DENV2 PM6
MRCIGMSNRDFVEGVSGGSWVDIVLEHGSCVTTMAKNKPTLDFELIKTEAKQPATLRKYCIEAKLTNTTTESRCPTQGEPSLNEEQDKRFVCKHSMVDRGWGNGCGLFGKGGIVTCAMFRCKKNMEGKVVQPENLEYTIVITPHSGEEHAVGNDTGKHGKEIKITPQSSITEAELTGYGTVTMECSPRTGLDFNEMVLLQMENKAWLVHRQWFLDLPLPWLPGADTQGSNWIQKETLVTFKNPHAKKQDVVVLGSQEGAMHTALTGATEIQMSSGNLLFTGHLKCRLRMDKLQLKGMSYSMCTGKFKVVKEIAETQHGTIVIRVQYEGDGSPCKIPFEIMDLEKRHVLGRLITVNPIVTEKDSPVNIEAEPPFGLSYIIIGVEPGQLKLQWFKK

SEQ ID NO: 61 - DNA, 1182 bp, synthetic construct
  misc_feature 1..1182: note = DENV2 PM7
  source 1..1182: mol_type = other DNA
atgaggtgtatcggcatgtccaacagggactttgtggagggagtgagcggcggcagctgggtggacattgtgctggagcatggaagctgcgtgaccacgatggcgaaaaacaagcccaccctggacttcgagctcatcaagacagaggctaaacagcccgccaccctcaggaagtactgcatcgaggccaagctgaccaacacaacaaccgagtccagatgccctacacagggcgaacccagcctcaacgaagagcaggacaagaggttcgtgtgcaaacacagcatggtggacaggggctggggcaatggatgcggactcttcggaaaaggcggcatcgtgacctgcgccatgttcaggtgtaaaaagaacatggaaggcaaggtggtgcagcccgaaaatctggagtataccatcgtgattaccccccacagcggagaggagcacgccgtgggcaatgacaccggcaagcacggcaaagagattaagatcaccccccagtcctccattaccgaagctgaactgacaggctacggcaccgtgacaatggagtgtagccccaggaccggactggatttcaacgagatggtcctgctacagatggagaacaaggcctggctcgtgcacaggcaatggtttctggatctgcctctgccttggctgcctggcgccgatacacagggctccaactggatacagaaagagaccctcgtcaccttcaagaatccccatgctaagaagcaggacgtggtggtgctgggcagccaagaaggcgccatgcacacagccctgaccggagctaccgagatccagatgagctccggcaacctgctgttcaccggccatctgaaatgtaggctgaggatggataagctgcaactcaaaggcatgtcctactccatgtgcaccggaaagttcaaggtggtgaaagaaatcgccgaaacacagcacggcaccatcgtgatcagggtgcagtatgagggcgacgcctccccctgtaagatccccttcgaaatcatggacctggaaaagaggcacgtgctgggcaggctcatcaccgtgaaccccattgtcacagagaaagactcccccgtgaacatcgaggccgagcctccctttggcgactcctacatcatcattggcgtggagcccggacagctcaagctgaactggttcaagaag

SEQ ID NO: 62 - protein, 394 aa, synthetic construct
  REGION 1..394: note = DENV2 PM7
MRCIGMSNRDFVEGVSGGSWVDIVLEHGSCVTTMAKNKPTLDFELIKTEAKQPATLRKYCIEAKLTNTTTESRCPTQGEPSLNEEQDKRFVCKHSMVDRGWGNGCGLFGKGGIVTCAMFRCKKNMEGKVVQPENLEYTIVITPHSGEEHAVGNDTGKHGKEIKITPQSSITEAELTGYGTVTMECSPRTGLDFNEMVLLQMENKAWLVHRQWFLDLPLPWLPGADTQGSNWIQKETLVTFKNPHAKKQDVVVLGSQEGAMHTALTGATEIQMSSGNLLFTGHLKCRLRMDKLQLKGMSYSMCTGKFKVVKEIAETQHGTIVIRVQYEGDASPCKIPFEIMDLEKRHVLGRLITVNPIVTEKDSPVNIEAEPPFGDSYIIIGVEPGQLKLNWFKK

SEQ ID NO: 63 - DNA, 1182 bp, synthetic construct
  misc_feature 1..1182: note = DENV2 PM8
  source 1..1182: mol_type = other DNA
atgaggtgtatcggcatgtccaacagggactttgtggagggagtgagcggcggcagctgggtggacattgtgctggagcatggaagctgcgtgaccacgatggcgaaaaacaagcccaccctggacttcgagctcatcaagacagaggctaaacagcccgccaccctcaggaagtactgcatcgaggccaagctgaccaacacaacaaccgagtccagatgccctacacagggcgaacccagcctcaacgaagagcaggacaagaggttcgtgtgcaaacacagcatggtggacaggggctggggcaatggatgcggactcttcggaaaaggcggcatcgtgacctgcgccatgttcaggtgtaaaaagaacatggaaggcaaggtggtgcagcccgaaaatctggagtataccatcgtgattaccccccacagcggagaggagcacgccgtgggcaatgacaccggcaagcacggcaaagagattaagatcaccccccagtcctccattaccgaagctgaactgacaggctacggcaccgtgacaatggagtgtagccccaggaccggactggatttcaacgagatggtcctgctacagatggagaacaaggcctggctcgtgcacaggcaatggtttctggatctgcctctgccttggctgcctggcgccgatacacagggctccaactggatacagaaagagaccctcgtcaccttcaagaatccccatgctaagaagcaggacgtggtggtgctgggcagccaagaaggcgccatgcacacagccctgaccggagctaccgagatccagatgagctccggcaacctgctgttcaccggccatctgaaatgtaggctgaggatggataagctgcaactcaaaggcatgtcctactccatgtgcaccggaaagttcaaggtggtgaaagaaatcgccgaaacacagcacggcaccatcgtgatcagggtgcagtatgagggcgacggctccccctgtaagatccccttcgaaatcatggacctggaaaagaggcacgtgctgggcaggctcatcaccgtgaaccccattgtcacagagaaagactcccccgtgaacatcgaggccgagcctccctttggcgactccgtgatcatcattggcgtggagcccggacagctcaagctgaactggttccggaag

SEQ ID NO: 64 - protein, 394 aa, synthetic construct
  REGION 1..394: note = DENV2 PM8
MRCIGMSNRDFVEGVSGGSWVDIVLEHGSCVTTMAKNKPTLDFELIKTEAKQPATLRKYCIEAKLTNTTTESRCPTQGEPSLNEEQDKRFVCKHSMVDRGWGNGCGLFGKGGIVTCAMFRCKKNMEGKVVQPENLEYTIVITPHSGEEHAVGNDTGKHGKEIKITPQSSITEAELTGYGTVTMECSPRTGLDFNEMVLLQMENKAWLVHRQWFLDLPLPWLPGADTQGSNWIQKETLVTFKNPHAKKQDVVVLGSQEGAMHTALTGATEIQMSSGNLLFTGHLKCRLRMDKLQLKGMSYSMCTGKFKVVKEIAETQHGTIVIRVQYEGDGSPCKIPFEIMDLEKRHVLGRLITVNPIVTEKDSPVNIEAEPPFGDSVIIIGVEPGQLKLNWFRK

SEQ ID NO: 65 - DNA, 1182 bp, synthetic construct
  misc_feature 1..1182: note = DENV2 SHP1
  source 1..1182: mol_type = other DNA
atgaggtgtatcggcatgtccaacagggactttgtggagggagagagcggcggcagctgggtggacattgtgctggagcatggaagctgcgtgaccacgatggcgaaaaacaagcccaccctggacttcgagctcatcaagacagaggctaaacagcccgccaccctcaggaagtactgcatcgaggccaagctgaccaacacaacaaccgagtccagatgccctacacagggcgaacccagcctcaacgaagagcaggacaagaggttcgtgtgcaaacacagcatggtggacaggggctggggcaatggatgcggactcttcggaaaaggcggcatcgtgacctgcgccatgttcaggtgtaaaaagaacatggaaggcaaggtggtgcagcccgaaaatctggagtataccatcgtgattaccccccacagcggagaggagcacgccgtgggcaatgacaccggcaagcacggcaaagagattaagatcaccccccagtcctccattaccgaagctgaactgacaggctacggcaccgtgacaatggagtgtagccccaggaccggactggatttcaacgagatggtcctgctacagatggagaacaaggcctggctcgtgcacaggcaatggtttctggatctgcctctgccttggctgcctggcgccgatacacagggctccaactggatacagaaagagaccctcgtcaccttcaagaatccccatgctaagaagcaggacgtggtggtgctgggcagccaagaaggcgccatgcacacagccctgaccggagctaccgagatccagatgagctccggcaacctgctgttcaccggccatctgaaatgtaggctgaggatggataagctgcaactcaaaggcatgtcctactccatgtgcaccggaaagttcaaggtggtgaaagaaatcgccgaaacacagcacggcaccatcgtgatcagggtgcagtatgagggcgacggctccccctgtaagatccccttcgaaatcatggacctggaaaagaggcacgtgctgggcaggctcatcaccgtgaaccccattgtcacagagaaagactcccccgtgaacatcgaggccgagcctcccgacggcgactcctacatcatcattggcgtggagcccggacagctcaagctgaactggagaaagaag

SEQ ID NO: 66 - protein, 394 aa, synthetic construct
  REGION 1..394: note = DENV2 SHP1
MRCIGMSNRDFVEGESGGSWVDIVLEHGSCVTTMAKNKPTLDFELIKTEAKQPATLRKYCIEAKLTNTTTESRCPTQGEPSLNEEQDKRFVCKHSMVDRGWGNGCGLFGKGGIVTCAMFRCKKNMEGKVVQPENLEYTIVITPHSGEEHAVGNDTGKHGKEIKITPQSSITEAELTGYGTVTMECSPRTGLDFNEMVLLQMENKAWLVHRQWFLDLPLPWLPGADTQGSNWIQKETLVTFKNPHAKKQDVVVLGSQEGAMHTALTGATEIQMSSGNLLFTGHLKCRLRMDKLQLKGMSYSMCTGKFKVVKEIAETQHGTIVIRVQYEGDGSPCKIPFEIMDLEKRHVLGRLITVNPIVTEKDSPVNIEAEPPDGDSYIIIGVEPGQLKLNWRKK

SEQ ID NO: 67 - DNA, 1182 bp, synthetic construct
  misc_feature 1..1182: note = DENV2 SHP2
  source 1..1182: mol_type = other DNA
atgaggtgtatcggcatgtccaacagggactttgtggagggagagagcggcggcagccacgtggacattgtgctggagcatggaagctgcgtgaccacgatggcgaaaaacaagcccaccctggacttcgagctcatcaagacagaggctaaacagcccgccaccctcaggaagtactgcatcgaggccaagctgaccaacacaacaaccgagtccagatgccctacacagggcgaacccagcctcaacgaagagcaggacaagaggttcgtgtgcaaacacagcatggtggacaggggctggggcaatggatgcggactcttcggaaaaggcggcatcgtgacctgcgccatgttcaggtgtaaaaagaacatggaaggcaaggtggtgcagcccgaaaatctggagtataccatcgtgattaccccccacagcggagaggagcacgccgtgggcaatgacaccggcaagcacggcaaagagattaagatcaccccccagtcctccattaccgaagctgaactgacaggctacggcaccgtgacaatggagtgtagccccaggaccggactggatttcaacgagatggtcctgctacagatggagaacaaggcctggctcgtgcacaggcaatggtttctggatctgcctctgccttggctgcctggcgccgatacacagggctccaactggatacagaaagagaccctcgtcaccttcaagaatccccatgctaagaagcaggacgtggtggtgctgggcagccaagaaggcgccatgcacacagccctgaccggagctaccgagatccagatgagctccggcaacctgctgttcaccggccatctgaaatgtaggctgaggatggataagctgcaactcaaaggcatgtcctactccatgtgcaccggaaagttcaaggtggtgaaagaaatcgccgaaacacagcacggcaccatcgtgatcagggtgcagtatgagggcgacggctccccctgtaagatccccttcgaaatcatggacctggaaaagaggcacgtgctgggcaggctcatcaccgtgaaccccattgtcacagagaaagactcccccgtgaacatcgaggccgagcctcccgacggcgactcctacatcatcattggcgtggagcccggacagctcaagctgaactggcggaagaag

SEQ ID NO: 68 - protein, 394 aa, synthetic construct
  REGION 1..394: note = DENV2 SHP2
MRCIGMSNRDFVEGESGGSHVDIVLEHGSCVTTMAKNKPTLDFELIKTEAKQPATLRKYCIEAKLTNTTTESRCPTQGEPSLNEEQDKRFVCKHSMVDRGWGNGCGLFGKGGIVTCAMFRCKKNMEGKVVQPENLEYTIVITPHSGEEHAVGNDTGKHGKEIKITPQSSITEAELTGYGTVTMECSPRTGLDFNEMVLLQMENKAWLVHRQWFLDLPLPWLPGADTQGSNWIQKETLVTFKNPHAKKQDVVVLGSQEGAMHTALTGATEIQMSSGNLLFTGHLKCRLRMDKLQLKGMSYSMCTGKFKVVKEIAETQHGTIVIRVQYEGDGSPCKIPFEIMDLEKRHVLGRLITVNPIVTEKDSPVNIEAEPPDGDSYIIIGVEPGQLKLNWRKK

SEQ ID NO: 69 - DNA, 1182 bp, synthetic construct
  misc_feature 1..1182: note = DENV2 UndPk1
  source 1..1182: mol_type = other DNA
atgaggtgtatcggcatgtccaacagggactttgtggagggagtgagcggcggcagctgggtggacattgtgctggagcatggaagctgcgtgaccacgatggcgaaaaacaagcccaccctggacttcgagctcatcaagacagaggctaaacagcccgccaccctcaggaagtactgcatcgaggccaagctgaccaacacaacaaccgagtccagatgccctacacagggcgaacccagcctcaacgaagagcaggacaagaggttcgtgtgcaaacacagcatggtggacaggggctggggcaatggatgcggactcttcggaaaaggcggcatcgtgacctgcgccatgttcaggtgtaaaaagaacatggaaggcaaggtggtgcagcccgaaaatctggagtataccatcgtgattaccccccacagcggagaggagcacgccgtgggcaatgacaccggcaagcacggcaaagagattaagatcaccccccagtcctccattaccgaagctgaactgacaggctacggcaccgtgacaatggagtgtagccccaggaccggactggatttcaacgagatggtcctgctacagatggagaacaaggcctggctcgtgcacaggcaatggtttctggatctgcctctgccttggctgcctggcgccgatacacagggctccaactggatacagaaagagaccctcgtcaccttcaagaatccccatgctaagaagcaggacgtggtggtgctgggcagccaagaaggcgccatgcacacagccctgaccggagctaccgaggtgcagatgagctccggcaacctgctgttcgccggccatctgaaatgtaggctgaggatggataagctgcaactcaaaggcatgtcctactccatgtgcaccggaaagttcaaggtggtgaaagaaatcgccgaaacacagcacggcaccatcgtgatcagggtgcagtatgagggcgacggctccccctgtaagatccccttcgaaatcatggacctggaaaagaggcacgtgctgggcaggctcatcaccgtgaaccccattgtcacagagaaagactcccccgtgaacatcgaggccgagcctccctttggcgactcctacatcatcattggcgtggagcccggacagctcaagctgaactggttcaagaag

SEQ ID NO: 70 - protein, 394 aa, synthetic construct
  REGION 1..394: note = DENV2 UndPk1
MRCIGMSNRDFVEGVSGGSWVDIVLEHGSCVTTMAKNKPTLDFELIKTEAKQPATLRKYCIEAKLTNTTTESRCPTQGEPSLNEEQDKRFVCKHSMVDRGWGNGCGLFGKGGIVTCAMFRCKKNMEGKVVQPENLEYTIVITPHSGEEHAVGNDTGKHGKEIKITPQSSITEAELTGYGTVTMECSPRTGLDFNEMVLLQMENKAWLVHRQWFLDLPLPWLPGADTQGSNWIQKETLVTFKNPHAKKQDVVVLGSQEGAMHTALTGATEVQMSSGNLLFAGHLKCRLRMDKLQLKGMSYSMCTGKFKVVKEIAETQHGTIVIRVQYEGDGSPCKIPFEIMDLEKRHVLGRLITVNPIVTEKDSPVNIEAEPPFGDSYIIIGVEPGQLKLNWFKK

SEQ ID NO: 71 - DNA, 1182 bp, synthetic construct
  misc_feature 1..1182: note = DENV2 UndPk2
  source 1..1182: mol_type = other DNA
atgaggtgtatcggcatgtccaacagggactttgtggagggagtgagcggcggcagctgggtggacattgtgctggagcatggaagctgcgtgaccacgatggcgaaaaacaagcccaccctggacttcgagctcatcaagacagaggctaaacagcccgccaccctcaggaagtactgcatcgaggccaagctgaccaacacaacaaccgagtccagatgccctacacagggcgaacccagcctcaacgaagagcaggacaagaggttcgtgtgcaaacacagcatggtggacaggggctggggcaatggatgcggactcttcggaaaaggcggcatcgtgacctgcgccatgttcaggtgtaaaaagaacatggaaggcaaggtggtgcagcccgaaaatctggagtataccatcgtgattaccccccacagcggagaggagcacgccgtgggcaatgacaccggcaagcacggcaaagagattaagatcaccccccagtcctccattaccgaagctgaactgacaggctacggcaccgtgacaatggagtgtagccccaggaccggactggatttcaacgagatggtctggctacagatggagaacaaggcctggctcgtgcacaggcaatggtttctggatctgcctctgccttggctgcctggcgccgatacacagggctccaactggatacagaaagagaccctcgtcaccttcaagaatccccatgctaagaagcaggacgtggtggtgctgggcagccaagaaggcgccatgcacacagccctgaccggagctaccgagatccagatgagctccggcaacctgctgttcaccggccatctgaaatgtaggctgaggatggataagctgcaactcaaaggcatgtcctactccatgtgcaccggaaagttcaaggtggtgaaagaaatcgccgaaacacagcacggcaccatcgtgatcagggtgcagtatgagggcgacggctccccctgtaagatccccttcgaaatcatggacctggaaaagaggcacgtgctgggcaggctcatcaccgtgaaccccattgtcacagagaaagactcccccgtgaacatcgaggccgagcctccctttggcgactcctacatcatcattggcgtggagcccggacagctcaagctgaactggttcaagaag

SEQ ID NO: 72 - protein, 394 aa, synthetic construct
  REGION 1..394: note = DENV2 UndPk2
MRCIGMSNRDFVEGVSGGSWVDIVLEHGSCVTTMAKNKPTLDFELIKTEAKQPATLRKYCIEAKLTNTTTESRCPTQGEPSLNEEQDKRFVCKHSMVDRGWGNGCGLFGKGGIVTCAMFRCKKNMEGKVVQPENLEYTIVITPHSGEEHAVGNDTGKHGKEIKITPQSSITEAELTGYGTVTMECSPRTGLDFNEMVWLQMENKAWLVHRQWFLDLPLPWLPGADTQGSNWIQKETLVTFKNPHAKKQDVVVLGSQEGAMHTALTGATEIQMSSGNLLFTGHLKCRLRMDKLQLKGMSYSMCTGKFKVVKEIAETQHGTIVIRVQYEGDGSPCKIPFEIMDLEKRHVLGRLITVNPIVTEKDSPVNIEAEPPFGDSYIIIGVEPGQLKLNWFKK

SEQ ID NO: 73 - DNA, 1182 bp, synthetic construct
  misc_feature 1..1182: note = DENV2 UndPk3
  source 1..1182: mol_type = other DNA
atgaggtgtatcggcatgtccaacagggactttgtggagggagtgagcggcggcagctgggtggacattgtgctggagcatggaagctgcgtgaccacgatggcgaaaaacaagcccaccctggacttcgagctcatcaagacagaggctaaacagcccgccaccctcaggaagtactgcatcgaggccaagctgaccaacacaacaaccgagtccagatgccctacacagggcgaacccagcctcaacgaagagcaggacaagaggttcgtgtgcaaacacagcatggtggacaggggctggggcaatggatgcggactcttcggaaaaggcggcatcgtgacctgcgccatgttcaggtgtaaaaagaacatggaaggcaaggtggtgcagcccgaaaatctggagtataccatcgtgattaccccccacagcggagaggagcacgccgtgggcaatgacaccggcaagcacggcaaagagattaagatcaccccccagtcctccattaccgaagctgaactgacaggctacggcaccgtgacaatggagtgtagccccaggaccggatacgatttcaacgagatggtcctgctacagatggagaacaaggcctggctcgtggacaggcaatggtttctggatctgcctctgccttggctgcctggcgccgatacacagggctccaactggatacagaaagagaccctcgtcaccttcaagaatccccatgctaagaagcaggacgtggtggtgctgggcagccaagaaggcgccatgcacacagccctgaccggagctaccgagatccagatgagctccggcaacctgctgttcaccggccatctgaaatgtaggctgaggatggataagctgcaactcaaaggcatgtcctactccatgtgcaccggaaagttcaaggtggtgaaagaaatcgccgaaacacagcacggcaccatcgtgatcagggtgcagtatgagggcgacggctccccctgtaagatccccttcgaaatcatggacctggaaaagaggcacgtgctgggcaggctcatcaccgtgaaccccattgtcacagagaaagactcccccgtgaacatcgaggccgagcctccctttggcgactcctacatcatcattggcgtggagcccggacagctcaagctgaactggttcaagaag

SEQ ID NO: 74 - protein, 394 aa, synthetic construct
  REGION 1..394: note = DENV2 UndPk3
MRCIGMSNRDFVEGVSGGSWVDIVLEHGSCVTTMAKNKPTLDFELIKTEAKQPATLRKYCIEAKLTNTTTESRCPTQGEPSLNEEQDKRFVCKHSMVDRGWGNGCGLFGKGGIVTCAMFRCKKNMEGKVVQPENLEYTIVITPHSGEEHAVGNDTGKHGKEIKITPQSSITEAELTGYGTVTMECSPRTGYDFNEMVLLQMENKAWLVDRQWFLDLPLPWLPGADTQGSNWIQKETLVTFKNPHAKKQDVVVLGSQEGAMHTALTGATEIQMSSGNLLFTGHLKCRLRMDKLQLKGMSYSMCTGKFKVVKEIAETQHGTIVIRVQYEGDGSPCKIPFEIMDLEKRHVLGRLITVNPIVTEKDSPVNIEAEPPFGDSYIIIGVEPGQLKLNWFKK

SEQ ID NO: 75 - DNA, 1182 bp, synthetic construct
  misc_feature 1..1182: note = DENV2 UndPk4
  source 1..1182: mol_type = other DNA
atgaggtgtatcggcatgtccaacagggactttgtgttcgccgtgagcggcggcagctgggtggacattgtgctggagcatggaagctgcgtgaccacgctggcgaaaaacaagcccaccctggacttcgagctcatcaagacagaggctaaacagcccgccaccctcaggaagtactgcatcgaggccaagctgaccaacacaacaaccgagtccagatgccctacacagggcgaacccagcctcaacgaagagcaggacaagaggttcgtgtgcaaacacagcatggtggacaggggctggggcaatggatgcggactcttcggaaaaggcggcatcgtgacctgcgccatgttcaggtgtaaaaagaacatggaaggcaaggtggtgcagcccgaaaatctggagtataccatcgtgattaccccccacagcggagaggagcacgccgtgggcaatgacaccggcaagcacggcaaagagattaagatcaccccccagtcctccattaccgaagctgaactgacaggctacggcaccgtgacaatggagtgtagccccaggaccggactggatttcaacgagatggtcctgctacagatggagaacaaggcctggctcgtgcacaggcaatggtttctggatctgcctctgccttggctgcctggcgccgatacacagggctccaactggatacagaaagagaccctcgtcaccttcaagaatccccatgctaagaagcaggacgtggtggtgctgggcagccaagaaggcgccatgcacacagccctgaccggagctaccgagatccagatgagctccggcaacctgctgttcaccggccatctgaaatgtaggctgaggatggataagctgcaactcaaaggcatgtcctactccatgtgcaccggaaagttcaaggtggtgaaagaaatcgccgaaacacagcacggcaccatcgtgatcagggtgcagtatgagggcgacggctccccctgtaagatccccttcgaaatcatggacctggaaaagaggcacgtgctgggcaggctcatcaccgtgaaccccattgtcacagagaaagactcccccgtgaacatcgaggccgagcctccctttggcgactcctacatcatcattggcgtggagcccggacagctcaagctgaactggttcaagaag

SEQ ID NO: 76 - protein, 394 aa, synthetic construct
  REGION 1..394: note = DENV2 UndPk4
MRCIGMSNRDFVFAVSGGSWVDIVLEHGSCVTTLAKNKPTLDFELIKTEAKQPATLRKYCIEAKLTNTTTESRCPTQGEPSLNEEQDKRFVCKHSMVDRGWGNGCGLFGKGGIVTCAMFRCKKNMEGKVVQPENLEYTIVITPHSGEEHAVGNDTGKHGKEIKITPQSSITEAELTGYGTVTMECSPRTGLDFNEMVLLQMENKAWLVHRQWFLDLPLPWLPGADTQGSNWIQKETLVTFKNPHAKKQDVVVLGSQEGAMHTALTGATEIQMSSGNLLFTGHLKCRLRMDKLQLKGMSYSMCTGKFKVVKEIAETQHGTIVIRVQYEGDGSPCKIPFEIMDLEKRHVLGRLITVNPIVTEKDSPVNIEAEPPFGDSYIIIGVEPGQLKLNWFKK

SEQ ID NO: 77 - DNA, 1182 bp, synthetic construct
  misc_feature 1..1182: note = DENV2 UndPk5
  source 1..1182: mol_type = other DNA
atgaggtgtatcggcatgtccaacagggactttgtggagggagtgagcggcggcagctgggtggacattgtgctggagcatggaagctgcgtgaccacgatggcgaaaaacaagcccaccctggacttcgagctcatcaagacagaggctaaacagcccgccaccctcaggaagtactgcatcgaggccaagctgaccaacacaacaaccgagtccagatgccctacacagggcgaacccagcctcaacgaagagcaggacaagaggttcgtgtgcaaacacagcatggtggacaggggctggggcaatggatgcggactcttcggaaaaggcggcatcgtgacctgcgccatgttcaggtgtaaaaagaacatggaaggcaaggtggtgcagcccgaaaatctggagtataccatcgtgattaccccccacagcggagaggagcacgccgtgggcaatgacaccggcaagcacggcaaagagattaagatcaccccccagtcctccattaccgaagctgaactgacaggctacggcaccgtgacaatggagtgtagccccaggaccggactggatttcaacgagatggtcctgctacagatggagaacaaggcctggctcgtgcacaggcaatggtttctggatctgcctctgccttggctgcctggcgccgatacacagggctccaactggatacagaaagagaccctcgtcaccttcaagaatccccatgctaagaagcaggacgtggtggtgctgggcagccaagaaggcgccatgcacacagccctgaccggagctaccgagatccagatgagctccggcaacctgctgttcaccggccatctgaaatgtaggctgaggatggataagctgcaactcaaaggcatgtcctactccatgtgcaccggaaagttcaaggtggtgaaagaaatcgccgaaacacagcacggcaccatcgtgatcagggtgcagtatgagggcgacggctccccctgtaagatccccttcgaaatcatggacctggaaaagaggcacgtgctgggcaggctcatcaccgtgaaccccattgtctacgagaaagactcccccgtgaacatcgaggccgagcctccctttggcgactcctacatcatcattggcgtggagcccggacagctcaagctgaactggttcaagaag

SEQ ID NO: 78 - protein, 394 aa, synthetic construct
  REGION 1..394: note = DENV2 UndPk5
MRCIGMSNRDFVEGVSGGSWVDIVLEHGSCVTTMAKNKPTLDFELIKTEAKQPATLRKYCIEAKLTNTTTESRCPTQGEPSLNEEQDKRFVCKHSMVDRGWGNGCGLFGKGGIVTCAMFRCKKNMEGKVVQPENLEYTIVITPHSGEEHAVGNDTGKHGKEIKITPQSSITEAELTGYGTVTMECSPRTGLDFNEMVLLQMENKAWLVHRQWFLDLPLPWLPGADTQGSNWIQKETLVTFKNPHAKKQDVVVLGSQEGAMHTALTGATEIQMSSGNLLFTGHLKCRLRMDKLQLKGMSYSMCTGKFKVVKEIAETQHGTIVIRVQYEGDGSPCKIPFEIMDLEKRHVLGRLITVNPIVYEKDSPVNIEAEPPFGDSYIIIGVEPGQLKLNWFKK

SEQ ID NO: 79 - DNA, 1182 bp, synthetic construct
  misc_feature 1..1182: note = DENV2 UndPk6
  source 1..1182: mol_type = other DNA
atgaggtgtatcggcatgtccaacagggactttgtggagggagtgagcggcggcagctgggtggacattgtgctggagcatggaagctgcgtgaccacgatggcgaaaaacaagcccaccctggacttcgagctcatcaagacagaggctaaacagcccgccaccctcaggaagtactgcatcgaggccaagctgaccaacacaacaaccgagtccagatgccctacacagggcgaacccagcctcaacgaagagcaggacaagaggttcgtgtgcaaacacagcatggtggacaggggctggggcaatggatgcggactcttcggaaaaggcggcatcgtgacctgcgccatgttcaggtgtaaaaagaacatggaaggcaaggtggtgcagcccgaaaatctggagtataccatcgtgattaccccccacagcggagaggagcacgccgtgggcaatgacaccggcaagcacggcaaagagattaagatcaccccccagtcctccattaccgaagctgaactgacaggctacggcaccgtgacaatggagtgtagccccaggaccggactggatttcaacgagatggtcctgctacagatggagaacaaggcctggctcgtgcacaggcaatggtttctggatctgcctctgccttggctgcctggcgccgatacacagggctccaactggatacagaaagagaccctcgtcaccttcaagaatccccatgctaagaagcaggacgtggtggtgctgggcagccaagaaggcgccatgcacacagccctgaccggagctaccgagatccagatgagctccggcaacctgctgtggcccggccatctgaaatgtaggctgaggatggataagctgcaactcaaaggcatgtcctactccatgtgcaccggaaagttcaaggtggtgaaagaaatcgccgaaacacagcacggcaccatcgtgatcagggtgcagtatgagggcgacggctccccctgtaagatccccttcgaaatcatggacctggaaaagaggcacgtgctgggcaggctcatcaccgtgaaccccattgtcacagagaaagactcccccgtgaacatcgaggccgagcctccctttggcgactcctacatcatcattggcgtggagcccggacagctcaagctgaactggttcaagaag

SEQ ID NO: 80 - protein, 394 aa, synthetic construct
  REGION 1..394: note = DENV2 UndPk6
MRCIGMSNRDFVEGVSGGSWVDIVLEHGSCVTTMAKNKPTLDFELIKTEAKQPATLRKYCIEAKLTNTTTESRCPTQGEPSLNEEQDKRFVCKHSMVDRGWGNGCGLFGKGGIVTCAMFRCKKNMEGKVVQPENLEYTIVITPHSGEEHAVGNDTGKHGKEIKITPQSSITEAELTGYGTVTMECSPRTGLDFNEMVLLQMENKAWLVHRQWFLDLPLPWLPGADTQGSNWIQKETLVTFKNPHAKKQDVVVLGSQEGAMHTALTGATEIQMSSGNLLWPGHLKCRLRMDKLQLKGMSYSMCTGKFKVVKEIAETQHGTIVIRVQYEGDGSPCKIPFEIMDLEKRHVLGRLITVNPIVTEKDSPVNIEAEPPFGDSYIIIGVEPGQLKLNWFKK

SEQ ID NO: 81 - DNA, 1182 bp, synthetic construct
  misc_feature 1..1182: note = DENV2 UndPk6.1
  source 1..1182: mol_type = other DNA
atgaggtgtatcggcatgtccaacagggactttgtggagggagtgagcggcggcagctgggtggacattgtgctggagcatggaagctgcgtgaccacgatggcgaaaaacaagcccaccctggacttcgagctcatcaagacagaggctaaacagcccgccaccctcaggaagtactgcatcgaggccaagctgaccaacacaacaaccgagtccagatgccctacacagggcgaacccagcctcaacgaagagcaggacaagaggttcgtgtgcaaacacagcatggtggacaggggctggggcaatggatgcggactcttcggaaaaggcggcatcgtgacctgcgccatgttcaggtgtaaaaagaacatggaaggcaaggtggtgcagcccgaaaatctggagtataccatcgtgattaccccccacagcggagaggagcacgccgtgggcaatgacaccggcaagcacggcaaagagattaagatcaccccccagtcctccattaccgaagctgaactgacaggctacggcaccgtgacaatggagtgtagccccaggaccggactggatttcaacgagatggtcctgctacagatggagaacaaggcctggctcgtgcacaggcaatggtttctggatctgcctctgccttggctgcctggcgccgatacacagggctccaactggatacagaaagagaccctcgtcaccttcaagaatccccatgctaagaagcaggacgtggtggtgctgggcagccaagaaggcgccatgcacacagccctgaccggagctaccgagatccagatgagctccggcaacctgctgttccccggccatctgaaatgtaggctgaggatggataagctgcaactcaaaggcatgtcctactccatgtgcaccggaaagttcaaggtggtgaaagaaatcgccgaaacacagcacggcaccatcgtgatcagggtgcagtatgagggcgacggctccccctgtaagatccccttcgaaatcatggacctggaaaagaggcacgtgctgggcaggctcatcaccgtgaaccccattgtcacagagaaagactcccccgtgaacatcgaggccgagcctccctttggcgactcctacatcatcattggcgtggagcccggacagctcaagctgaactggttcaagaag

SEQ ID NO: 82 - protein, 395 aa, synthetic construct
  REGION 1..395: note = DENV2 UndPk6.1
SMRCIGMSNRDFVEGVSGGSWVDIVLEHGSCVTTMAKNKPTLDFELIKTEAKQPATLRKYCIEAKLTNTTTESRCPTQGEPSLNEEQDKRFVCKHSMVDRGWGNGCGLFGKGGIVTCAMFRCKKNMEGKVVQPENLEYTIVITPHSGEEHAVGNDTGKHGKEIKITPQSSITEAELTGYGTVTMECSPRTGLDFNEMVLLQMENKAWLVHRQWFLDLPLPWLPGADTQGSNWIQKETLVTFKNPHAKKQDVVVLGSQEGAMHTALTGATEIQMSSGNLLFPGHLKCRLRMDKLQLKGMSYSMCTGKFKVVKEIAETQHGTIVIRVQYEGDGSPCKIPFEIMDLEKRHVLGRLITVNPIVTEKDSPVNIEAEPPFGDSYIIIGVEPGQLKLNWFKK

SEQ ID NO: 83 - DNA, 1182 bp, synthetic construct
  misc_feature 1..1182: note = DENV2 UndPk7
  source 1..1182: mol_type = other DNA
atgaggtgtatcggcatgtccaacagggactttgtggagggagtgagcggcggcagctgggtggacattgtgctggagcatggaagctgcgtgaccacgatggcgaaaaacaagcccaccctggacttcgagctcatcaagatcgaggctaaacagcccgccaccctcaggaagtactgcatcgaggccaagctgaccaacacaacaaccgagtccagatgccctacacagggcgaacccagcctcaacgaagagcaggacaagaggttcgtgtgcaaacacagcatggtggacaggggctggggcaatggatgcggactcttcggaaaaggcggcatcgtgacctgcgccatgttcaggtgtaaaaagaacatggaaggcaaggtggtgcagcccgaaaatctggagtataccatcgtgattaccccccacagcggagaggagcacgccgtgggcaatgacaccggcaagcacggcaaagagattaagatcaccccccagtcctccattaccgaagctgaactgacaggctacggcaccgtgacaatggagtgtagccccaggaccggactggatttcaacgagatggtcctgctacagatggagaacaaggcctggctcgtgcacaggcaatggtttctggatctgcctctgccttggctgcctggcgccgatacacagggctccaactggatacagaaagagaccctcgtcaccttcaagaatccccatgctaagaagcaggacgtggtggtgctgggcagccaagaaggcgccatgcacacagccctgaccggagctaccgagatccagatgagctccggcaacatgctgttcaccggccatctgaaatgtaggctgaggatggataagctgcaactcaaaggcatgtcctactccatgtgcaccggaaagttcaaggtggtgaaagaaatcgccgaaacacagcacggcaccatcgtgatcagggtgcagtatgagggcgacggctccccctgtaagatccccttcgaaatcatggacctggaaaagaggcacgtgctgggcaggctcatcaccgtgaaccccattgtcacagagaaagactcccccgtgaacatcgaggccgagcctccctttggcgactcctacatcatcattggcgtggagcccggacagctcaagctgaactggttcaagaag

SEQ ID NO: 84 - protein, 394 aa, synthetic construct
  REGION 1..394: note = DENV2 UndPk7
MRCIGMSNRDFVEGVSGGSWVDIVLEHGSCVTTMAKNKPTLDFELIKIEAKQPATLRKYCIEAKLTNTTTESRCPTQGEPSLNEEQDKRFVCKHSMVDRGWGNGCGLFGKGGIVTCAMFRCKKNMEGKVVQPENLEYTIVITPHSGEEHAVGNDTGKHGKEIKITPQSSITEAELTGYGTVTMECSPRTGLDFNEMVLLQMENKAWLVHRQWFLDLPLPWLPGADTQGSNWIQKETLVTFKNPHAKKQDVVVLGSQEGAMHTALTGATEIQMSSGNMLFTGHLKCRLRMDKLQLKGMSYSMCTGKFKVVKEIAETQHGTIVIRVQYEGDGSPCKIPFEIMDLEKRHVLGRLITVNPIVTEKDSPVNIEAEPPFGDSYIIIGVEPGQLKLNWFKK

SEQ ID NO: 85 - DNA, 1182 bp, synthetic construct
  misc_feature 1..1182: note = DENV2 UndPk8
  source 1..1182: mol_type = other DNA
atgaggtgtatcggcatgtccaacagggactttgtggagggagtgagcggcggcagctgggtggacattgtgctggagcatggaagctgcgtgaccacgatggcgaaaaacaagcccaccctggacttcgagctcatcaagacagaggctaaacagcccgccaccctcaggaagtactgcatcgaggccaagctgaccaacacaacaaccgagtccagatgccctacacagggcgaacccagcctcaacgaagagcaggacaagaggttcgtgtgcaaacacagcatggtggacaggggctggggcaatggatgcggactcttcggaaaaggcggcatcgtgacctgcgccatgttcaggtgtaaaaagaacatggaaggcaaggtggtgcagcccgaaaatctggagtataccatcgtgattaccccccacagcggagaggagcacgccgtgggcaatgacaccggcaagcacggcaaagagattaagatcaccccccagtcctccattaccgaagctgaactgacaggctacggcaccgtgacaatggagtgtagccccaggaccggactggatttcaacgagatggtcctgctacagatggagaacaaggcctggctcgtgcacaggcaatggtttctggatctgcctctgccttggctgcctggcgccgatacacagggctccaactggatacagaaagagaccctcgtcaccttcaagaatccccatgctaagaagcaggacgtggtggtgctgggcagctacgaagcctggctgcacacagccctgaccggagctaccgagatccagatgagctccggcaacctgctgttcaccggccatctgaaatgtaggctgaggatggataagctgcaactcaaaggcatgtcctactccatgtgcaccggaaagttcaaggtggtgaaagaaatcgccgaaacacagcacggcaccatcgtgatcagggtgcagtatgagggcgacggctccccctgtaagatccccttcgaaatcatggacctggaaaagaggcacgtgctgggcaggctcatcaccgtgaaccccattgtcacagagaaagactcccccgtgaacatcgaggccgagcctccctttggcgactcctacatcatcattggcgtggagcccggacagctcaagctgaactggttcaagaag

SEQ ID NO: 86 - protein, 394 aa, synthetic construct
  REGION 1..394: note = DENV2 UndPk8
MRCIGMSNRDFVEGVSGGSWVDIVLEHGSCVTTMAKNKPTLDFELIKTEAKQPATLRKYCIEAKLTNTTTESRCPTQGEPSLNEEQDKRFVCKHSMVDRGWGNGCGLFGKGGIVTCAMFRCKKNMEGKVVQPENLEYTIVITPHSGEEHAVGNDTGKHGKEIKITPQSSITEAELTGYGTVTMECSPRTGLDFNEMVLLQMENKAWLVHRQWFLDLPLPWLPGADTQGSNWIQKETLVTFKNPHAKKQDVVVLGSYEAWLHTALTGATEIQMSSGNLLFTGHLKCRLRMDKLQLKGMSYSMCTGKFKVVKEIAETQHGTIVIRVQYEGDGSPCKIPFEIMDLEKRHVLGRLITVNPIVTEKDSPVNIEAEPPFGDSYIIIGVEPGQLKLNWFKK

SEQ ID NO: 87 - DNA, 1182 bp, synthetic construct
  misc_feature 1..1182: note = DENV2 Cm1
  source 1..1182: mol_type = other DNA
atgaggtgtatcggcatgtccaacagggactttgtggagggagtgagcggcggcagctgggtggacattgtgctggagcatggaagctgcgtgaccacgatggcgaaaaacaagcccaccctggacttcgagctcatcaagacagaggctaaacagcccgccaccctcaggaagtactgcatcgaggccaagctgaccaacacaacaaccgagtccagatgccctacacagggcgaacccagcctcaacgaagagcaggacaagaggttcgtgtgcaaacacagcatggtggacaggggctggggcaatggatgcggactcttcggaaaaggcggcatcgtgacctgcgccatgttcaggtgtaaaaagaacatggaaggcaaggtggtgcagcccgaaaatctggagtataccatcgtgattaccccccacagcggagaggagcacgccgtgggcaatgacaccggcaagcacggcaaagagattaagatcaccccccagtcctccattaccgaagctgaactgacaggctacggcaccgtgacaatggagtgtagccccaggaccggactggatttcaacgagatggtcctgctacagatggagaacaaggcctggctcgtgcacaggcaatggtttctggatctgcctctgccttggctgcctggcgccgatacacagggctccaactggatacagaaagagaccctcgtcaccttcaagaatccccatgctaagaagcaggacgtggtggtgctgggcagccaagaaggctgtatgcacacagccctgaccggagctaccgagatccagatgagctccggcaacctgctgttcaccggccatctgaaatgtaggctgaggatggataagctgcaactcaaaggcatgtcctactccatgtgcaccggaaagttcaaggtggtgaaagaaatcgccgaaacacagcacggcaccatcgtgatcagggtgcagtatgagggcgacggctccccctgtaagatccccttcgaaatcatggacctggaaaagaggcacgtgctgggcaggctcatcaccgtgaaccccattgtcacagagaaagactcccccgtgaacatcgaggccgagcctccctttggcgactcctacatcatcattggcgtggagcccggacagctcaagctgaactggttcaagaag

SEQ ID NO: 88 - protein, 394 aa, synthetic construct
  REGION 1..394: note = DENV2 Cm1
MRCIGMSNRDFVEGVSGGSWVDIVLEHGSCVTTMAKNKPTLDFELIKTEAKQPATLRKYCIEAKLTNTTTESRCPTQGEPSLNEEQDKRFVCKHSMVDRGWGNGCGLFGKGGIVTCAMFRCKKNMEGKVVQPENLEYTIVITPHSGEEHAVGNDTGKHGKEIKITPQSSITEAELTGYGTVTMECSPRTGLDFNEMVLLQMENKAWLVHRQWFLDLPLPWLPGADTQGSNWIQKETLVTFKNPHAKKQDVVVLGSQEGCMHTALTGATEIQMSSGNLLFTGHLKCRLRMDKLQLKGMSYSMCTGKFKVVKEIAETQHGTIVIRVQYEGDGSPCKIPFEIMDLEKRHVLGRLITVNPIVTEKDSPVNIEAEPPFGDSYIIIGVEPGQLKLNWFKK

SEQ ID NO: 89 - DNA, 1182 bp, synthetic construct
  misc_feature 1..1182: note = DENV2 Cm2
  source 1..1182: mol_type = other DNA
atgaggtgtatcggcatgtccaacagggactttgtggagggagtgagcggcggcagctgggtggacattgtgctggagcatggaagctgcgtgaccacgatggcgaaaaacaagcccaccctggacttcgagctcatcaagacagaggctaaacagcccgccaccctcaggaagtactgcatcgaggccaagctgaccaacacaacaaccgagtccagatgccctacacagggcgaacccagcctcaacgaagagcaggacaagaggttcgtgtgcaaacacagcatggtggacaggggctggggcaatggatgcggatgtttcggaaaaggcggcatcgtgacctgcgccatgttcaggtgtaaaaagaacatggaaggcaaggtggtgcagcccgaaaatctggagtataccatcgtgattaccccccacagcggagaggagcacgccgtgggcaatgacaccggcaagcacggcaaagagattaagatcaccccccagtcctccattaccgaagctgaactgacaggctacggcaccgtgacaatggagtgtagccccaggaccggactggatttcaacgagatggtcctgctacagatggagaacaaggcctggctcgtgcacaggcaatggtttctggatctgcctctgccttggctgcctggcgccgatacacagggctccaactggatacagaaagagaccctcgtcaccttcaagaatccccatgctaagaagcaggacgtggtggtgctgggcagccaagaaggcgccatgcacacagccctgaccggagctaccgagatccagatgagctccggcaacctgctgttcaccggccatctgaaatgtaggctgaggatggataagctgcaactcaaaggcatgtcctactccatgtgcaccggaaagttcaaggtggtgaaagaaatctgtgaaacacagcacggcaccatcgtgatcagggtgcagtatgagggcgacggctccccctgtaagatccccttcgaaatcatggacctggaaaagaggcacgtgctgggcaggctcatcaccgtgaaccccattgtcacagagaaagactcccccgtgaacatcgaggccgagcctccctttggcgactcctacatcatcattggcgtggagcccggacagctcaagctgaactggttcaagaag

SEQ ID NO: 90 - protein, 394 aa, synthetic construct
  REGION 1..394: note = DENV2 Cm2
MRCIGMSNRDFVEGVSGGSWVDIVLEHGSCVTTMAKNKPTLDFELIKTEAKQPATLRKYCIEAKLTNTTTESRCPTQGEPSLNEEQDKRFVCKHSMVDRGWGNGCGCFGKGGIVTCAMFRCKKNMEGKVVQPENLEYTIVITPHSGEEHAVGNDTGKHGKEIKITPQSSITEAELTGYGTVTMECSPRTGLDFNEMVLLQMENKAWLVHRQWFLDLPLPWLPGADTQGSNWIQKETLVTFKNPHAKKQDVVVLGSQEGAMHTALTGATEIQMSSGNLLFTGHLKCRLRMDKLQLKGMSYSMCTGKFKVVKEICETQHGTIVIRVQYEGDGSPCKIPFEIMDLEKRHVLGRLITVNPIVTEKDSPVNIEAEPPFGDSYIIIGVEPGQLKLNWFKK

SEQ ID NO: 91 - DNA, 1182 bp, synthetic construct
  misc_feature 1..1182: note = DENV2 SC.1 (I2-I8-P4)
  source 1..1182: mol_type = other DNA
atgaggtgtatcggcatgtccaacagggactttgtggagggagtgagcggcggcagctgggtggacattgtgctggagcatggaaagtgcgtgaccgtgatgatgaaaaacaagcccaccctggacttcgagctcatcaagacagaggctaaacagcccgccaccctcaggaagtactgcatcgaggccaagctgaccaacacaacaaccgagtccagatgccctacacagggcgaacccagcctcaacgaagagcaggacaagaggttcgtgtgcaaacacagcatggtggacaggggctggggcaatggatgcgacctcttcggaaaaggcggcatcgtgacctgcgccatgttcaggtgtaaaaagaacatggaaggcaaggtggtgcagcccgaaaatctggagtataccatcgtgattaccccccacagcggagaggagcacgccgtgggcaatgacaccggcaagcacggcaaagagattaagatcaccccccagtcctccattaccgaagctgaactgacaggctacggcaccgtgacaatggagtgtagccccaggaccggactggatttcaacgagatggtcctgctacagatggagaacaaggcctggctcgtgcacaggcaatggtttctggatctgcctctgccttggctgcctggcgccgatacacagggctccaactggatacagaaagagaccctcgtcaccttcaagaatccccatgctaagaagcaggacgtggtggtgctgggcagccaagaaggctggatgcaccgggccctgaccggagctaccgagatccagatgagctccggcaacctgctgttcaccggccatctgaaatgtaggctgaggatggataagctgcaactcaaaggcatgtcctactccatgtgcaccggaaagttcaaggtggtgaaagaaatcgccgaaacacagcacggcaccatcgtgatcagggtgcagtatgagggcgacggctccccctgtaagatccccttcgaaatcatggacctggaaaagaggcacgtgctgggcaggctcatcaccgtgaaccccattgtcacagagaaagactcccccgtgaacatcgaggccgagcctccctttggcgactcctacatcatcattggcgtggagcccggacagctcaagctgaactggttcaagaag

SEQ ID NO: 92 - protein, 394 aa, synthetic construct
  REGION 1..394: note = DENV2 SC.1 (I2-I8-P4)
MRCIGMSNRDFVEGVSGGSWVDIVLEHGKCVTVMMKNKPTLDFELIKTEAKQPATLRKYCIEAKLTNTTTESRCPTQGEPSLNEEQDKRFVCKHSMVDRGWGNGCDLFGKGGIVTCAMFRCKKNMEGKVVQPENLEYTIVITPHSGEEHAVGNDTGKHGKEIKITPQSSITEAELTGYGTVTMECSPRTGLDFNEMVLLQMENKAWLVHRQWFLDLPLPWLPGADTQGSNWIQKETLVTFKNPHAKKQDVVVLGSQEGWMHRALTGATEIQMSSGNLLFTGHLKCRLRMDKLQLKGMSYSMCTGKFKVVKEIAETQHGTIVIRVQYEGDGSPCKIPFEIMDLEKRHVLGRLITVNPIVTEKDSPVNIEAEPPFGDSYIIIGVEPGQLKLNWFKK

SEQ ID NO: 93 - DNA, 1182 bp, synthetic construct
  misc_feature 1..1182: note = DENV2 SC.2 (I2-I8-P4-H3)
  source 1..1182: mol_type = other DNA
atgaggtgtatcggcatgtccaacagggactttgtggagggagtgagcggcggcagctgggtggacattgtgctggagcccggaaagtgcgtgaccgtgatgatgaaaaacaagcccaccctggacttcgagctcatcaagatcgaggctaaacagcccgccaccctcaggaagtactgcatcgaggccaagctgaccaacacaacaaccgagtccagatgccctacacagggcgaacccagcctcaacgaagagcaggacaagaggttcgtgtgcaaacacagcatggtggacaggggctggggcaatggatgcgacctcttcggaaaaggcggcatcgtgacctgcgccatgttcaggtgtaaaaagaacatggaaggcaaggtggtgcagcccgaaaatctggagtataccatcgtgattaccccccacagcggagaggagcacgccgtgggcaatgacaccggcaagcacggcaaagagattaagatcaccccccagtcctccattaccgaagctgaactgacaggctacggcaccgtgacaatggagtgtagccccaggaccggactggatttcaacgagatggtcctgctacagatggagaacaaggcctggctcgtgcacaggcaatggtttctggatctgcctctgccttggctgcctggcgccgatacacagggctccaactggatacagaaagagaccctcgtcaccttcaagaatccccatgctaagaagcaggacgtggtggtgctgggcagccaagaaggctggatgcaccgggccctgaccggagctaccgagatccagatgagctccggcaacctgctgttcaccggccatctgaaatgtaggctgaggatggataagctgcaactcaaaggcatgtcctactccatgtgcaccggaaagttcaaggtggtgaaagaaatcgccgaaacacagcacggcaccatcgtgatcagggtgcagtatgagggcgacggctccccctgtaagatccccttcgaaatcatggacctggaaaagaggcacgtgctgggcaggctcatcaccgtgaaccccattgtcacagagaaagactcccccgtgaacatcgaggccgagcctccctttggcgactcctacatcatcattggcgtggagcccggacagctcaagctgaactggttcaagaag

SEQ ID NO: 94 - protein, 394 aa, synthetic construct
  REGION 1..394: note = DENV2 SC.2 (I2-I8-P4-H3)
MRCIGMSNRDFVEGVSGGSWVDIVLEPGKCVTVMMKNKPTLDFELIKIEAKQPATLRKYCIEAKLTNTTTESRCPTQGEPSLNEEQDKRFVCKHSMVDRGWGNGCDLFGKGGIVTCAMFRCKKNMEGKVVQPENLEYTIVITPHSGEEHAVGNDTGKHGKEIKITPQSSITEAELTGYGTVTMECSPRTGLDFNEMVLLQMENKAWLVHRQWFLDLPLPWLPGADTQGSNWIQKETLVTFKNPHAKKQDVVVLGSQEGWMHRALTGATEIQMSSGNLLFTGHLKCRLRMDKLQLKGMSYSMCTGKFKVVKEIAETQHGTIVIRVQYEGDGSPCKIPFEIMDLEKRHVLGRLITVNPIVTEKDSPVNIEAEPPFGDSYIIIGVEPGQLKLNWFKK

SEQ ID NO: 95 - DNA, 1182 bp, synthetic construct
  misc_feature 1..1182: note = DENV2 SC.3 (I2-I8-U4-U5-U6-P5)
  source 1..1182: mol_type = other DNA
atgaggtgtatcggcatgtccaacagggactttgtgttcgccgtgagcggcggcagctgggtggacattgtgctggagcatggaagctgcgtgaccacgctggcgaaaaacaagcccaccctggacttcgagctcatcaagacagaggctaaacagcccgccaccctcaggaagtactgcatcgaggccaagctgaccaacacaacaaccgagtccagatgccctacacagggcgaacccagcctcaacgaagagcaggacaagaggttcgtgtgcaaacacagcatggtggacaggggctggggcaatggatgcgacctcttcggaaaaggcggcatcgtgacctgcgccatgttcaggtgtaaaaagaacatggaaggcaaggtggtgcagcccgaaaatctggagtataccatcgtgattaccccccacagcggagaggagcacgccgtgggcaatgacaccggcaagcacggcaaagagattaagatcaccccccagtcctccattaccgaagctgaactgacaggctacggcaccgtgacaatggagtgtagccccaggaccggactggatttcaacgagatggtcctgctacagatggagaacaaggcctggctcgtggacaggcaatggtttctggatctgcctctgccttggctgcctggcgccgatacacagggctccaactggatacagaaagagaccctcgtcaccttcaagaatccccatgctaagaagcaggacgtggtggtgctgggcagccaagaaggctggatgcaccgggccctgacctgggctaccgagatccagatgagctccggcaacctgctgtggcccggccatctgaaatgtaggctgaggatggataagctgcaactcaaaggcatgtcctactccatgtgcaccggaaagttcaaggtggtgaaagaaatcgccgaaacacagcacggcaccatcgtgatcagggtgcagtatgagggcgacggctccccctgtaagatccccttcgaaatcatggacctggaaaagaggcacgtgctgggcaggctcatcaccgtgaaccccattgtctacgagaaagactcccccgtgaacatcgaggccgagcctccctttggcgactcctacatcatcattggcgtggagcccggacagctcaagctgaactggttcaagaag

SEQ ID NO: 96 - protein, 394 aa, synthetic construct
  REGION 1..394: note = DENV2 SC.3 (I2-I8-U4-U5-U6-P5)
MRCIGMSNRDFVFAVSGGSWVDIVLEHGSCVTTLAKNKPTLDFELIKTEAKQPATLRKYCIEAKLTNTTTESRCPTQGEPSLNEEQDKRFVCKHSMVDRGWGNGCDLFGKGGIVTCAMFRCKKNMEGKVVQPENLEYTIVITPHSGEEHAVGNDTGKHGKEIKITPQSSITEAELTGYGTVTMECSPRTGLDFNEMVLLQMENKAWLVDRQWFLDLPLPWLPGADTQGSNWIQKETLVTFKNPHAKKQDVVVLGSQEGWMHRALTWATEIQMSSGNLLWPGHLKCRLRMDKLQLKGMSYSMCTGKFKVVKEIAETQHGTIVIRVQYEGDGSPCKIPFEIMDLEKRHVLGRLITVNPIVYEKDSPVNIEAEPPFGDSYIIIGVEPGQLKLNWFKK

SEQ ID NO: 97 - DNA, 1182 bp, synthetic construct
  misc_feature 1..1182: note = DENV2 SC.4 (I2-I8-U4-U5-U6-P4-P5-H3)
  source 1..1182: mol_type = other DNA
atgaggtgtatcggcatgtccaacagggactttgtgttcgccgtgagcggcggcagctgggtggacattgtgctggagcccggaaagtgcgtgaccgtgctgatgaaaaacaagcccaccctggacttcgagctcatcaagatcgaggctaaacagcccgccaccctcaggaagtactgcatcgaggccaagctgaccaacacaacaaccgagtccagatgccctacacagggcgaacccagcctcaacgaagagcaggacaagaggttcgtgtgcaaacacagcatggtggacaggggctggggcaatggatgcgacctcttcggaaaaggcggcatcgtgacctgcgccatgttcaggtgtaaaaagaacatggaaggcaaggtggtgcagcccgaaaatctggagtataccatcgtgattaccccccacagcggagaggagcacgccgtgggcaatgacaccggcaagcacggcaaagagattaagatcaccccccagtcctccattaccgaagctgaactgacaggctacggcaccgtgacaatggagtgtagccccaggaccggactggatttcaacgagatggtcctgctacagatggagaacaaggcctggctcgtggacaggcaatggtttctggatctgcctctgccttggctgcctggcgccgatacacagggctccaactggatacagaaagagaccctcgtcaccttcaagaatccccatgctaagaagcaggacgtggtggtgctgggcagccaagaaggctggatgcaccgggccctgacctgggctaccgagatccagatgagctccggcaacctgctgtggcccggccatctgaaatgtaggctgaggatggataagctgcaactcaaaggcatgtcctactccatgtgcaccggaaagttcaaggtggtgaaagaaatcgccgaaacacagcacggcaccatcgtgatcagggtgcagtatgagggcgacggctccccctgtaagatccccttcgaaatcatggacctggaaaagaggcacgtgctgggcaggctcatcaccgtgaaccccattgtctacgagaaagactcccccgtgaacatcgaggccgagcctccctttggcgactcctacatcatcattggcgtggagcccggacagctcaagctgaactggttcaagaag

SEQ ID NO: 98 - protein, 394 aa, synthetic construct
  REGION 1..394: note = DENV2 SC.4 (I2-I8-U4-U5-U6-P4-P5-H3)
MRCIGMSNRDFVFAVSGGSWVDIVLEPGKCVTVLMKNKPTLDFELIKIEAKQPATLRKYCIEAKLTNTTTESRCPTQGEPSLNEEQDKRFVCKHSMVDRGWGNGCDLFGKGGIVTCAMFRCKKNMEGKVVQPENLEYTIVITPHSGEEHAVGNDTGKHGKEIKITPQSSITEAELTGYGTVTMECSPRTGLDFNEMVLLQMENKAWLVDRQWFLDLPLPWLPGADTQGSNWIQKETLVTFKNPHAKKQDVVVLGSQEGWMHRALTWATEIQMSSGNLLWPGHLKCRLRMDKLQLKGMSYSMCTGKFKVVKEIAETQHGTIVIRVQYEGDGSPCKIPFEIMDLEKRHVLGRLITVNPIVYEKDSPVNIEAEPPFGDSYIIIGVEPGQLKLNWFKK

SEQ ID NO: 99 - DNA, 1182 bp, synthetic construct
  misc_feature 1..1182: note = DENV2 SC.5 (I2-I8-U4-U6)
  source 1..1182: mol_type = other DNA
atgaggtgtatcggcatgtccaacagggactttgtgttcgccgtgagcggcggcagctgggtggacattgtgctggagcatggaagctgcgtgaccacgctggcgaaaaacaagcccaccctggacttcgagctcatcaagacagaggctaaacagcccgccaccctcaggaagtactgcatcgaggccaagctgaccaacacaacaaccgagtccagatgccctacacagggcgaacccagcctcaacgaagagcaggacaagaggttcgtgtgcaaacacagcatggtggacaggggctggggcaatggatgcgacctcttcggaaaaggcggcatcgtgacctgcgccatgttcaggtgtaaaaagaacatggaaggcaaggtggtgcagcccgaaaatctggagtataccatcgtgattaccccccacagcggagaggagcacgccgtgggcaatgacaccggcaagcacggcaaagagattaagatcaccccccagtcctccattaccgaagctgaactgacaggctacggcaccgtgacaatggagtgtagccccaggaccggactggatttcaacgagatggtcctgctacagatggagaacaaggcctggctcgtgcacaggcaatggtttctggatctgcctctgccttggctgcctggcgccgatacacagggctccaactggatacagaaagagaccctcgtcaccttcaagaatccccatgctaagaagcaggacgtggtggtgctgggcagccaagaaggctggatgcaccgggccctgaccggagctaccgagatccagatgagctccggcaacctgctgtggcccggccatctgaaatgtaggctgaggatggataagctgcaactcaaaggcatgtcctactccatgtgcaccggaaagttcaaggtggtgaaagaaatcgccgaaacacagcacggcaccatcgtgatcagggtgcagtatgagggcgacggctccccctgtaagatccccttcgaaatcatggacctggaaaagaggcacgtgctgggcaggctcatcaccgtgaaccccattgtcacagagaaagactcccccgtgaacatcgaggccgagcctccctttggcgactcctacatcatcattggcgtggagcccggacagctcaagctgaactggttcaagaag

SEQ ID NO: 100 - protein, 394 aa, synthetic construct
  REGION 1..394: note = DENV2 SC.5 (I2-I8-U4-U6)
MRCIGMSNRDFVFAVSGGSWVDIVLEHGSCVTTLAKNKPTLDFELIKTEAKQPATLRKYCIEAKLTNTTTESRCPTQGEPSLNEEQDKRFVCKHSMVDRGWGNGCDLFGKGGIVTCAMFRCKKNMEGKVVQPENLEYTIVITPHSGEEHAVGNDTGKHGKEIKITPQSSITEAELTGYGTVTMECSPRTGLDFNEMVLLQMENKAWLVHRQWFLDLPLPWLPGADTQGSNWIQKETLVTFKNPHAKKQDVVVLGSQEGWMHRALTGATEIQMSSGNLLWPGHLKCRLRMDKLQLKGMSYSMCTGKFKVVKEIAETQHGTIVIRVQYEGDGSPCKIPFEIMDLEKRHVLGRLITVNPIVTEKDSPVNIEAEPPFGDSYIIIGVEPGQLKLNWFKK

SEQ ID NO: 101 - DNA, 1182 bp, synthetic construct
  misc_feature 1..1182: note = DENV2 SC.6 (I2-I8-U5-P4)
  source 1..1182: mol_type = other DNA
atgaggtgtatcggcatgtccaacagggactttgtggagggagtgagcggcggcagctgggtggacattgtgctggagcatggaaagtgcgtgaccgtgatgatgaaaaacaagcccaccctggacttcgagctcatcaagacagaggctaaacagcccgccaccctcaggaagtactgcatcgaggccaagctgaccaacacaacaaccgagtccagatgccctacacagggcgaacccagcctcaacgaagagcaggacaagaggttcgtgtgcaaacacagcatggtggacaggggctggggcaatggatgcgacctcttcggaaaaggcggcatcgtgacctgcgccatgttcaggtgtaaaaagaacatggaaggcaaggtggtgcagcccgaaaatctggagtataccatcgtgattaccccccacagcggagaggagcacgccgtgggcaatgacaccggcaagcacggcaaagagattaagatcaccccccagtcctccattaccgaagctgaactgacaggctacggcaccgtgacaatggagtgtagccccaggaccggactggatttcaacgagatggtcctgctacagatggagaacaaggcctggctcgtgcacaggcaatggtttctggatctgcctctgccttggctgcctggcgccgatacacagggctccaactggatacagaaagagaccctcgtcaccttcaagaatccccatgctaagaagcaggacgtggtggtgctgggcagccaagaaggctggatgcaccgggccctgaccggagctaccgagatccagatgagctccggcaacctgctgttcaccggccatctgaaatgtaggctgaggatggataagctgcaactcaaaggcatgtcctactccatgtgcaccggaaagttcaaggtggtgaaagaaatcgccgaaacacagcacggcaccatcgtgatcagggtgcagtatgagggcgacggctccccctgtaagatccccttcgaaatcatggacctggaaaagaggcacgtgctgggcaggctcatcaccgtgaaccccattgtctacgagaaagactcccccgtgaacatcgaggccgagcctccctttggcgactcctacatcatcattggcgtggagcccggacagctcaagctgaactggttcaagaag

SEQ ID NO: 102 - protein, 394 aa, synthetic construct
  REGION 1..394: note = DENV2 SC.6 (I2-I8-U5-P4)
MRCIGMSNRDFVEGVSGGSWVDIVLEHGKCVTVMMKNKPTLDFELIKTEAKQPATLRKYCIEAKLTNTTTESRCPTQGEPSLNEEQDKRFVCKHSMVDRGWGNGCDLFGKGGIVTCAMFRCKKNMEGKVVQPENLEYTIVITPHSGEEHAVGNDTGKHGKEIKITPQSSITEAELTGYGTVTMECSPRTGLDFNEMVLLQMENKAWLVHRQWFLDLPLPWLPGADTQGSNWIQKETLVTFKNPHAKKQDVVVLGSQEGWMHRALTGATEIQMSSGNLLFTGHLKCRLRMDKLQLKGMSYSMCTGKFKVVKEIAETQHGTIVIRVQYEGDGSPCKIPFEIMDLEKRHVLGRLITVNPIVYEKDSPVNIEAEPPFGDSYIIIGVEPGQLKLNWFKK

SEQ ID NO: 103 - DNA, 1182 bp, synthetic construct
  misc_feature 1..1182: note = DENV2 SC.7 (I2-I8-U5-U6)
  source 1..1182: mol_type = other DNA
atgaggtgtatcggcatgtccaacagggactttgtggagggagtgagcggcggcagctgggtggacattgtgctggagcatggaagctgcgtgaccacgatggcgaaaaacaagcccaccctggacttcgagctcatcaagacagaggctaaacagcccgccaccctcaggaagtactgcatcgaggccaagctgaccaacacaacaaccgagtccagatgccctacacagggcgaacccagcctcaacgaagagcaggacaagaggttcgtgtgcaaacacagcatggtggacaggggctggggcaatggatgcgacctcttcggaaaaggcggcatcgtgacctgcgccatgttcaggtgtaaaaagaacatggaaggcaaggtggtgcagcccgaaaatctggagtataccatcgtgattaccccccacagcggagaggagcacgccgtgggcaatgacaccggcaagcacggcaaagagattaagatcaccccccagtcctccattaccgaagctgaactgacaggctacggcaccgtgacaatggagtgtagccccaggaccggactggatttcaacgagatggtcctgctacagatggagaacaaggcctggctcgtgcacaggcaatggtttctggatctgcctctgccttggctgcctggcgccgatacacagggctccaactggatacagaaagagaccctcgtcaccttcaagaatccccatgctaagaagcaggacgtggtggtgctgggcagccaagaaggctggatgcaccgggccctgaccggagctaccgagatccagatgagctccggcaacctgctgtggcccggccatctgaaatgtaggctgaggatggataagctgcaactcaaaggcatgtcctactccatgtgcaccggaaagttcaaggtggtgaaagaaatcgccgaaacacagcacggcaccatcgtgatcagggtgcagtatgagggcgacggctccccctgtaagatccccttcgaaatcatggacctggaaaagaggcacgtgctgggcaggctcatcaccgtgaaccccattgtctacgagaaagactcccccgtgaacatcgaggccgagcctccctttggcgactcctacatcatcattggcgtggagcccggacagctcaagctgaactggttcaagaag

SEQ ID NO: 104 - protein, 394 aa, synthetic construct
  REGION 1..394: note = DENV2 SC.7 (I2-I8-U5-U6)
MRCIGMSNRDFVEGVSGGSWVDIVLEHGSCVTTMAKNKPTLDFELIKTEAKQPATLRKYCIEAKLTNTTTESRCPTQGEPSLNEEQDKRFVCKHSMVDRGWGNGCDLFGKGGIVTCAMFRCKKNMEGKVVQPENLEYTIVITPHSGEEHAVGNDTGKHGKEIKITPQSSITEAELTGYGTVTMECSPRTGLDFNEMVLLQMENKAWLVHRQWFLDLPLPWLPGADTQGSNWIQKETLVTFKNPHAKKQDVVVLGSQEGWMHRALTGATEIQMSSGNLLWPGHLKCRLRMDKLQLKGMSYSMCTGKFKVVKEIAETQHGTIVIRVQYEGDGSPCKIPFEIMDLEKRHVLGRLITVNPIVYEKDSPVNIEAEPPFGDSYIIIGVEPGQLKLNWFKK

SEQ ID NO: 105 - DNA, 1182 bp, synthetic construct
  misc_feature 1..1182: note = DENV2 SC.8 (I2-I8-U5-U6-P4)
  source 1..1182: mol_type = other DNA
atgaggtgtatcggcatgtccaacagggactttgtggagggagtgagcggcggcagctgggtggacattgtgctggagcatggaaagtgcgtgaccgtgatgatgaaaaacaagcccaccctggacttcgagctcatcaagacagaggctaaacagcccgccaccctcaggaagtactgcatcgaggccaagctgaccaacacaacaaccgagtccagatgccctacacagggcgaacccagcctcaacgaagagcaggacaagaggttcgtgtgcaaacacagcatggtggacaggggctggggcaatggatgcgacctcttcggaaaaggcggcatcgtgacctgcgccatgttcaggtgtaaaaagaacatggaaggcaaggtggtgcagcccgaaaatctggagtataccatcgtgattaccccccacagcggagaggagcacgccgtgggcaatgacaccggcaagcacggcaaagagattaagatcaccccccagtcctccattaccgaagctgaactgacaggctacggcaccgtgacaatggagtgtagccccaggaccggactggatttcaacgagatggtcctgctacagatggagaacaaggcctggctcgtgcacaggcaatggtttctggatctgcctctgccttggctgcctggcgccgatacacagggctccaactggatacagaaagagaccctcgtcaccttcaagaatccccatgctaagaagcaggacgtggtggtgctgggcagccaagaaggctggatgcaccgggccctgaccggagctaccgagatccagatgagctccggcaacctgctgtggcccggccatctgaaatgtaggctgaggatggataagctgcaactcaaaggcatgtcctactccatgtgcaccggaaagttcaaggtggtgaaagaaatcgccgaaacacagcacggcaccatcgtgatcagggtgcagtatgagggcgacggctccccctgtaagatccccttcgaaatcatggacctggaaaagaggcacgtgctgggcaggctcatcaccgtgaaccccattgtctacgagaaagactcccccgtgaacatcgaggccgagcctccctttggcgactcctacatcatcattggcgtggagcccggacagctcaagctgaactggttcaagaag

SEQ ID NO: 106 - protein, 394 aa, synthetic construct
  REGION 1..394: note = DENV2 SC.8 (I2-I8-U5-U6-P4)
MRCIGMSNRDFVEGVSGGSWVDIVLEHGKCVTVMMKNKPTLDFELIKTEAKQPATLRKYCIEAKLTNTTTESRCPTQGEPSLNEEQDKRFVCKHSMVDRGWGNGCDLFGKGGIVTCAMFRCKKNMEGKVVQPENLEYTIVITPHSGEEHAVGNDTGKHGKEIKITPQSSITEAELTGYGTVTMECSPRTGLDFNEMVLLQMENKAWLVHRQWFLDLPLPWLPGADTQGSNWIQKETLVTFKNPHAKKQDVVVLGSQEGWMHRALTGATEIQMSSGNLLWPGHLKCRLRMDKLQLKGMSYSMCTGKFKVVKEIAETQHGTIVIRVQYEGDGSPCKIPFEIMDLEKRHVLGRLITVNPIVYEKDSPVNIEAEPPFGDSYIIIGVEPGQLKLNWFKK

SEQ ID NO: 107 - DNA, 1182 bp, synthetic construct
  misc_feature 1..1182: note = DENV2 SC.9 (I2-I8-U5-U6-P4-S1)
  source 1..1182: mol_type = other DNA
atgaggtgtatcggcatgtccaacagggactttgtggagggagagagcggcggcagctgggtggacattgtgctggagcatggaaagtgcgtgaccgtgatgatgaaaaacaagcccaccctggacttcgagctcatcaagacagaggctaaacagcccgccaccctcaggaagtactgcatcgaggccaagctgaccaacacaacaaccgagtccagatgccctacacagggcgaacccagcctcaacgaagagcaggacaagaggttcgtgtgcaaacacagcatggtggacaggggctggggcaatggatgcgacctcttcggaaaaggcggcatcgtgacctgcgccatgttcaggtgtaaaaagaacatggaaggcaaggtggtgcagcccgaaaatctggagtataccatcgtgattaccccccacagcggagaggagcacgccgtgggcaatgacaccggcaagcacggcaaagagattaagatcaccccccagtcctccattaccgaagctgaactgacaggctacggcaccgtgacaatggagtgtagccccaggaccggactggatttcaacgagatggtcctgctacagatggagaacaaggcctggctcgtgcacaggcaatggtttctggatctgcctctgccttggctgcctggcgccgatacacagggctccaactggatacagaaagagaccctcgtcaccttcaagaatccccatgctaagaagcaggacgtggtggtgctgggcagccaagaaggctggatgcaccgggccctgaccggagctaccgagatccagatgagctccggcaacctgctgtggcccggccatctgaaatgtaggctgaggatggataagctgcaactcaaaggcatgtcctactccatgtgcaccggaaagttcaaggtggtgaaagaaatcgccgaaacacagcacggcaccatcgtgatcagggtgcagtatgagggcgacggctccccctgtaagatccccttcgaaatcatggacctggaaaagaggcacgtgctgggcaggctcatcaccgtgaaccccattgtctacgagaaagactcccccgtgaacatcgaggccgagcctcccgacggcgactcctacatcatcattggcgtggagcccggacagctcaagctgaactggagaaagaag

SEQ ID NO: 108 - protein, 394 aa, synthetic construct
  REGION 1..394: note = DENV2 SC.9 (I2-I8-U5-U6-P4-S1)
MRCIGMSNRDFVEGESGGSWVDIVLEHGKCVTVMMKNKPTLDFELIKTEAKQPATLRKYCIEAKLTNTTTESRCPTQGEPSLNEEQDKRFVCKHSMVDRGWGNGCDLFGKGGIVTCAMFRCKKNMEGKVVQPENLEYTIVITPHSGEEHAVGNDTGKHGKEIKITPQSSITEAELTGYGTVTMECSPRTGLDFNEMVLLQMENKAWLVHRQWFLDLPLPWLPGADTQGSNWIQKETLVTFKNPHAKKQDVVVLGSQEGWMHRALTGATEIQMSSGNLLWPGHLKCRLRMDKLQLKGMSYSMCTGKFKVVKEIAETQHGTIVIRVQYEGDGSPCKIPFEIMDLEKRHVLGRLITVNPIVYEKDSPVNIEAEPPDGDSYIIIGVEPGQLKLNWRKK

SEQ ID NO: 109 - DNA, 1182 bp, synthetic construct
  misc_feature 1..1182: note = DENV2 SC.10 (I2-I8-U6)
  source 1..1182: mol_type = other DNA
atgaggtgtatcggcatgtccaacagggactttgtggagggagtgagcggcggcagctgggtggacattgtgctggagcatggaagctgcgtgaccacgatggcgaaaaacaagcccaccctggacttcgagctcatcaagacagaggctaaacagcccgccaccctcaggaagtactgcatcgaggccaagctgaccaacacaacaaccgagtccagatgccctacacagggcgaacccagcctcaacgaagagcaggacaagaggttcgtgtgcaaacacagcatggtggacaggggctggggcaatggatgcgacctcttcggaaaaggcggcatcgtgacctgcgccatgttcaggtgtaaaaagaacatggaaggcaaggtggtgcagcccgaaaatctggagtataccatcgtgattaccccccacagcggagaggagcacgccgtgggcaatgacaccggcaagcacggcaaagagattaagatcaccccccagtcctccattaccgaagctgaactgacaggctacggcaccgtgacaatggagtgtagccccaggaccggactggatttcaacgagatggtcctgctacagatggagaacaaggcctggctcgtgcacaggcaatggtttctggatctgcctctgccttggctgcctggcgccgatacacagggctccaactggatacagaaagagaccctcgtcaccttcaagaatccccatgctaagaagcaggacgtggtggtgctgggcagccaagaaggctggatgcaccgggccctgaccggagctaccgagatccagatgagctccggcaacctgctgtggcccggccatctgaaatgtaggctgaggatggataagctgcaactcaaaggcatgtcctactccatgtgcaccggaaagttcaaggtggtgaaagaaatcgccgaaacacagcacggcaccatcgtgatcagggtgcagtatgagggcgacggctccccctgtaagatccccttcgaaatcatggacctggaaaagaggcacgtgctgggcaggctcatcaccgtgaaccccattgtcacagagaaagactcccccgtgaacatcgaggccgagcctccctttggcgactcctacatcatcattggcgtggagcccggacagctcaagctgaactggttcaagaag

SEQ ID NO: 110 - protein, 394 aa, synthetic construct
  REGION 1..394: note = DENV2 SC.10 (I2-I8-U6)
MRCIGMSNRDFVEGVSGGSWVDIVLEHGSCVTTMAKNKPTLDFELIKTEAKQPATLRKYCIEAKLTNTTTESRCPTQGEPSLNEEQDKRFVCKHSMVDRGWGNGCDLFGKGGIVTCAMFRCKKNMEGKVVQPENLEYTIVITPHSGEEHAVGNDTGKHGKEIKITPQSSITEAELTGYGTVTMECSPRTGLDFNEMVLLQMENKAWLVHRQWFLDLPLPWLPGADTQGSNWIQKETLVTFKNPHAKKQDVVVLGSQEGWMHRALTGATEIQMSSGNLLWPGHLKCRLRMDKLQLKGMSYSMCTGKFKVVKEIAETQHGTIVIRVQYEGDGSPCKIPFEIMDLEKRHVLGRLITVNPIVTEKDSPVNIEAEPPFGDSYIIIGVEPGQLKLNWFKK

SEQ ID NO: 111 - DNA, 1182 bp, synthetic construct
  misc_feature 1..1182: note = DENV2 SC.11 (I2-I8-U6-H3)
  source 1..1182: mol_type = other DNA
atgaggtgtatcggcatgtccaacagggactttgtggagggagtgagcggcggcagctgggtggacattgtgctggagcccggaagctgcgtgaccacgatggcgaaaaacaagcccaccctggacttcgagctcatcaagatcgaggctaaacagcccgccaccctcaggaagtactgcatcgaggccaagctgaccaacacaacaaccgagtccagatgccctacacagggcgaacccagcctcaacgaagagcaggacaagaggttcgtgtgcaaacacagcatggtggacaggggctggggcaatggatgcgacctcttcggaaaaggcggcatcgtgacctgcgccatgttcaggtgtaaaaagaacatggaaggcaaggtggtgcagcccgaaaatctggagtataccatcgtgattaccccccacagcggagaggagcacgccgtgggcaatgacaccggcaagcacggcaaagagattaagatcaccccccagtcctccattaccgaagctgaactgacaggctacggcaccgtgacaatggagtgtagccccaggaccggactggatttcaacgagatggtcctgctacagatggagaacaaggcctggctcgtgcacaggcaatggtttctggatctgcctctgccttggctgcctggcgccgatacacagggctccaactggatacagaaagagaccctcgtcaccttcaagaatccccatgctaagaagcaggacgtggtggtgctgggcagccaagaaggctggatgcaccgggccctgaccggagctaccgagatccagatgagctccggcaacctgctgtggcccggccatctgaaatgtaggctgaggatggataagctgcaactcaaaggcatgtcctactccatgtgcaccggaaagttcaaggtggtgaaagaaatcgccgaaacacagcacggcaccatcgtgatcagggtgcagtatgagggcgacggctccccctgtaagatccccttcgaaatcatggacctggaaaagaggcacgtgctgggcaggctcatcaccgtgaaccccattgtcacagagaaagactcccccgtgaacatcgaggccgagcctccctttggcgactcctacatcatcattggcgtggagcccggacagctcaagctgaactggttcaagaag

SEQ ID NO: 112 - protein, 394 aa, synthetic construct
  REGION 1..394: note = DENV2 SC.11 (I2-I8-U6-H3)
MRCIGMSNRDFVEGVSGGSWVDIVLEPGSCVTTMAKNKPTLDFELIKIEAKQPATLRKYCIEAKLTNTTTESRCPTQGEPSLNEEQDKRFVCKHSMVDRGWGNGCDLFGKGGIVTCAMFRCKKNMEGKVVQPENLEYTIVITPHSGEEHAVGNDTGKHGKEIKITPQSSITEAELTGYGTVTMECSPRTGLDFNEMVLLQMENKAWLVHRQWFLDLPLPWLPGADTQGSNWIQKETLVTFKNPHAKKQDVVVLGSQEGWMHRALTGATEIQMSSGNLLWPGHLKCRLRMDKLQLKGMSYSMCTGKFKVVKEIAETQHGTIVIRVQYEGDGSPCKIPFEIMDLEKRHVLGRLITVNPIVTEKDSPVNIEAEPPFGDSYIIIGVEPGQLKLNWFKK

SEQ ID NO: 113 - DNA, 1182 bp, synthetic construct
  misc_feature 1..1182: note = DENV2 SC.12 (I2-I8-U6-P4)
  source 1..1182: mol_type = other DNA
atgaggtgtatcggcatgtccaacagggactttgtggagggagtgagcggcggcagctgggtggacattgtgctggagcatggaaagtgcgtgaccgtgatgatgaaaaacaagcccaccctggacttcgagctcatcaagacagaggctaaacagcccgccaccctcaggaagtactgcatcgaggccaagctgaccaacacaacaaccgagtccagatgccctacacagggcgaacccagcctcaacgaagagcaggacaagaggttcgtgtgcaaacacagcatggtggacaggggctggggcaatggatgcgacctcttcggaaaaggcggcatcgtgacctgcgccatgttcaggtgtaaaaagaacatggaaggcaaggtggtgcagcccgaaaatctggagtataccatcgtgattaccccccacagcggagaggagcacgccgtgggcaatgacaccggcaagcacggcaaagagattaagatcaccccccagtcctccattaccgaagctgaactgacaggctacggcaccgtgacaatggagtgtagccccaggaccggactggatttcaacgagatggtcctgctacagatggagaacaaggcctggctcgtgcacaggcaatggtttctggatctgcctctgccttggctgcctggcgccgatacacagggctccaactggatacagaaagagaccctcgtcaccttcaagaatccccatgctaagaagcaggacgtggtggtgctgggcagccaagaaggctggatgcaccgggccctgaccggagctaccgagatccagatgagctccggcaacctgctgtggcccggccatctgaaatgtaggctgaggatggataagctgcaactcaaaggcatgtcctactccatgtgcaccggaaagttcaaggtggtgaaagaaatcgccgaaacacagcacggcaccatcgtgatcagggtgcagtatgagggcgacggctccccctgtaagatccccttcgaaatcatggacctggaaaagaggcacgtgctgggcaggctcatcaccgtgaaccccattgtcacagagaaagactcccccgtgaacatcgaggccgagcctccctttggcgactcctacatcatcattggcgtggagcccggacagctcaagctgaactggttcaagaag

SEQ ID NO: 114 - protein, 394 aa, synthetic construct
  REGION 1..394: note = DENV2 SC.12 (I2-I8-U6-P4)
MRCIGMSNRDFVEGVSGGSWVDIVLEHGKCVTVMMKNKPTLDFELIKTEAKQPATLRKYCIEAKLTNTTTESRCPTQGEPSLNEEQDKRFVCKHSMVDRGWGNGCDLFGKGGIVTCAMFRCKKNMEGKVVQPENLEYTIVITPHSGEEHAVGNDTGKHGKEIKITPQSSITEAELTGYGTVTMECSPRTGLDFNEMVLLQMENKAWLVHRQWFLDLPLPWLPGADTQGSNWIQKETLVTFKNPHAKKQDVVVLGSQEGWMHRALTGATEIQMSSGNLLWPGHLKCRLRMDKLQLKGMSYSMCTGKFKVVKEIAETQHGTIVIRVQYEGDGSPCKIPFEIMDLEKRHVLGRLITVNPIVTEKDSPVNIEAEPPFGDSYIIIGVEPGQLKLNWFKK

SEQ ID NO: 115 - DNA, 1182 bp, synthetic construct
  misc_feature 1..1182: note = DENV2 SC.13 (I2-U5-U6-P4)
  source 1..1182: mol_type = other DNA
atgaggtgtatcggcatgtccaacagggactttgtggagggagtgagcggcggcagctgggtggacattgtgctggagcatggaaagtgcgtgaccgtgatgatgaaaaacaagcccaccctggacttcgagctcatcaagacagaggctaaacagcccgccaccctcaggaagtactgcatcgaggccaagctgaccaacacaacaaccgagtccagatgccctacacagggcgaacccagcctcaacgaagagcaggacaagaggttcgtgtgcaaacacagcatggtggacaggggctggggcaatggatgcggactcttcggaaaaggcggcatcgtgacctgcgccatgttcaggtgtaaaaagaacatggaaggcaaggtggtgcagcccgaaaatctggagtataccatcgtgattaccccccacagcggagaggagcacgccgtgggcaatgacaccggcaagcacggcaaagagattaagatcaccccccagtcctccattaccgaagctgaactgacaggctacggcaccgtgacaatggagtgtagccccaggaccggactggatttcaacgagatggtcctgctacagatggagaacaaggcctggctcgtgcacaggcaatggtttctggatctgcctctgccttggctgcctggcgccgatacacagggctccaactggatacagaaagagaccctcgtcaccttcaagaatccccatgctaagaagcaggacgtggtggtgctgggcagccaagaaggctggatgcaccgggccctgaccggagctaccgagatccagatgagctccggcaacctgctgtggcccggccatctgaaatgtaggctgaggatggataagctgcaactcaaaggcatgtcctactccatgtgcaccggaaagttcaaggtggtgaaagaaatcgccgaaacacagcacggcaccatcgtgatcagggtgcagtatgagggcgacggctccccctgtaagatccccttcgaaatcatggacctggaaaagaggcacgtgctgggcaggctcatcaccgtgaaccccattgtctacgagaaagactcccccgtgaacatcgaggccgagcctccctttggcgactcctacatcatcattggcgtggagcccggacagctcaagctgaactggttcaagaag

SEQ ID NO: 116 - protein, 394 aa, synthetic construct
  REGION 1..394: note = DENV2 SC.13 (I2-U5-U6-P4)
MRCIGMSNRDFVEGVSGGSWVDIVLEHGKCVTVMMKNKPTLDFELIKTEAKQPATLRKYCIEAKLTNTTTESRCPTQGEPSLNEEQDKRFVCKHSMVDRGWGNGCGLFGKGGIVTCAMFRCKKNMEGKVVQPENLEYTIVITPHSGEEHAVGNDTGKHGKEIKITPQSSITEAELTGYGTVTMECSPRTGLDFNEMVLLQMENKAWLVHRQWFLDLPLPWLPGADTQGSNWIQKETLVTFKNPHAKKQDVVVLGSQEGWMHRALTGATEIQMSSGNLLWPGHLKCRLRMDKLQLKGMSYSMCTGKFKVVKEIAETQHGTIVIRVQYEGDGSPCKIPFEIMDLEKRHVLGRLITVNPIVYEKDSPVNIEAEPPFGDSYIIIGVEPGQLKLNWFKK

SEQ ID NO: 117 - DNA, 1182 bp, synthetic construct
  misc_feature 1..1182: note = DENV2 SC.14 (I2-U6)
  source 1..1182: mol_type = other DNA
atgaggtgtatcggcatgtccaacagggactttgtggagggagtgagcggcggcagctgggtggacattgtgctggagcatggaagctgcgtgaccacgatggcgaaaaacaagcccaccctggacttcgagctcatcaagacagaggctaaacagcccgccaccctcaggaagtactgcatcgaggccaagctgaccaacacaacaaccgagtccagatgccctacacagggcgaacccagcctcaacgaagagcaggacaagaggttcgtgtgcaaacacagcatggtggacaggggctggggcaatggatgcggactcttcggaaaaggcggcatcgtgacctgcgccatgttcaggtgtaaaaagaacatggaaggcaaggtggtgcagcccgaaaatctggagtataccatcgtgattaccccccacagcggagaggagcacgccgtgggcaatgacaccggcaagcacggcaaagagattaagatcaccccccagtcctccattaccgaagctgaactgacaggctacggcaccgtgacaatggagtgtagccccaggaccggactggatttcaacgagatggtcctgctacagatggagaacaaggcctggctcgtgcacaggcaatggtttctggatctgcctctgccttggctgcctggcgccgatacacagggctccaactggatacagaaagagaccctcgtcaccttcaagaatccccatgctaagaagcaggacgtggtggtgctgggcagccaagaaggctggatgcaccgggccctgaccggagctaccgagatccagatgagctccggcaacctgctgtggcccggccatctgaaatgtaggctgaggatggataagctgcaactcaaaggcatgtcctactccatgtgcaccggaaagttcaaggtggtgaaagaaatcgccgaaacacagcacggcaccatcgtgatcagggtgcagtatgagggcgacggctccccctgtaagatccccttcgaaatcatggacctggaaaagaggcacgtgctgggcaggctcatcaccgtgaaccccattgtcacagagaaagactcccccgtgaacatcgaggccgagcctccctttggcgactcctacatcatcattggcgtggagcccggacagctcaagctgaactggttcaagaag

SEQ ID NO: 118 - protein, 394 aa, synthetic construct
  REGION 1..394: note = DENV2 SC.14 (I2-U6)
MRCIGMSNRDFVEGVSGGSWVDIVLEHGSCVTTMAKNKPTLDFELIKTEAKQPATLRKYCIEAKLTNTTTESRCPTQGEPSLNEEQDKRFVCKHSMVDRGWGNGCGLFGKGGIVTCAMFRCKKNMEGKVVQPENLEYTIVITPHSGEEHAVGNDTGKHGKEIKITPQSSITEAELTGYGTVTMECSPRTGLDFNEMVLLQMENKAWLVHRQWFLDLPLPWLPGADTQGSNWIQKETLVTFKNPHAKKQDVVVLGSQEGWMHRALTGATEIQMSSGNLLWPGHLKCRLRMDKLQLKGMSYSMCTGKFKVVKEIAETQHGTIVIRVQYEGDGSPCKIPFEIMDLEKRHVLGRLITVNPIVTEKDSPVNIEAEPPFGDSYIIIGVEPGQLKLNWFKK

SEQ ID NO: 119 - DNA, 1182 bp, synthetic construct
  misc_feature 1..1182: note = DENV2 SC.15 (I8-U6)
  source 1..1182: mol_type = other DNA
atgaggtgtatcggcatgtccaacagggactttgtggagggagtgagcggcggcagctgggtggacattgtgctggagcatggaagctgcgtgaccacgatggcgaaaaacaagcccaccctggacttcgagctcatcaagacagaggctaaacagcccgccaccctcaggaagtactgcatcgaggccaagctgaccaacacaacaaccgagtccagatgccctacacagggcgaacccagcctcaacgaagagcaggacaagaggttcgtgtgcaaacacagcatggtggacaggggctggggcaatggatgcgacctcttcggaaaaggcggcatcgtgacctgcgccatgttcaggtgtaaaaagaacatggaaggcaaggtggtgcagcccgaaaatctggagtataccatcgtgattaccccccacagcggagaggagcacgccgtgggcaatgacaccggcaagcacggcaaagagattaagatcaccccccagtcctccattaccgaagctgaactgacaggctacggcaccgtgacaatggagtgtagccccaggaccggactggatttcaacgagatggtcctgctacagatggagaacaaggcctggctcgtgcacaggcaatggtttctggatctgcctctgccttggctgcctggcgccgatacacagggctccaactggatacagaaagagaccctcgtcaccttcaagaatccccatgctaagaagcaggacgtggtggtgctgggcagccaagaaggcgccatgcacacagccctgaccggagctaccgagatccagatgagctccggcaacctgctgtggcccggccatctgaaatgtaggctgaggatggataagctgcaactcaaaggcatgtcctactccatgtgcaccggaaagttcaaggtggtgaaagaaatcgccgaaacacagcacggcaccatcgtgatcagggtgcagtatgagggcgacggctccccctgtaagatccccttcgaaatcatggacctggaaaagaggcacgtgctgggcaggctcatcaccgtgaaccccattgtcacagagaaagactcccccgtgaacatcgaggccgagcctccctttggcgactcctacatcatcattggcgtggagcccggacagctcaagctgaactggttcaagaag

SEQ ID NO: 120 - protein, 394 aa, synthetic construct
  REGION 1..394: note = DENV2 SC.15 (I8-U6)
MRCIGMSNRDFVEGVSGGSWVDIVLEHGSCVTTMAKNKPTLDFELIKTEAKQPATLRKYCIEAKLTNTTTESRCPTQGEPSLNEEQDKRFVCKHSMVDRGWGNGCDLFGKGGIVTCAMFRCKKNMEGKVVQPENLEYTIVITPHSGEEHAVGNDTGKHGKEIKITPQSSITEAELTGYGTVTMECSPRTGLDFNEMVLLQMENKAWLVHRQWFLDLPLPWLPGADTQGSNWIQKETLVTFKNPHAKKQDVVVLGSQEGAMHTALTGATEIQMSSGNLLWPGHLKCRLRMDKLQLKGMSYSMCTGKFKVVKEIAETQHGTIVIRVQYEGDGSPCKIPFEIMDLEKRHVLGRLITVNPIVTEKDSPVNIEAEPPFGDSYIIIGVEPGQLKLNWFKK

SEQ ID NO: 121 - DNA, 1182 bp, synthetic construct
  misc_feature 1..1182: note = DENV2 SC.16 (I2-U6-H3)
  source 1..1182: mol_type = other DNA
atgaggtgtatcggcatgtccaacagggactttgtggagggagtgagcggcggcagctgggtggacattgtgctggagcccggaagctgcgtgaccacgatggcgaaaaacaagcccaccctggacttcgagctcatcaagatcgaggctaaacagcccgccaccctcaggaagtactgcatcgaggccaagctgaccaacacaacaaccgagtccagatgccctacacagggcgaacccagcctcaacgaagagcaggacaagaggttcgtgtgcaaacacagcatggtggacaggggctggggcaatggatgcggactcttcggaaaaggcggcatcgtgacctgcgccatgttcaggtgtaaaaagaacatggaaggcaaggtggtgcagcccgaaaatctggagtataccatcgtgattaccccccacagcggagaggagcacgccgtgggcaatgacaccggcaagcacggcaaagagattaagatcaccccccagtcctccattaccgaagctgaactgacaggctacggcaccgtgacaatggagtgtagccccaggaccggactggatttcaacgagatggtcctgctacagatggagaacaaggcctggctcgtgcacaggcaatggtttctggatctgcctctgccttggctgcctggcgccgatacacagggctccaactggatacagaaagagaccctcgtcaccttcaagaatccccatgctaagaagcaggacgtggtggtgctgggcagccaagaaggctggatgcaccgggccctgaccggagctaccgagatccagatgagctccggcaacctgctgtggcccggccatctgaaatgtaggctgaggatggataagctgcaactcaaaggcatgtcctactccatgtgcaccggaaagttcaaggtggtgaaagaaatcgccgaaacacagcacggcaccatcgtgatcagggtgcagtatgagggcgacggctccccctgtaagatccccttcgaaatcatggacctggaaaagaggcacgtgctgggcaggctcatcaccgtgaaccccattgtcacagagaaagactcccccgtgaacatcgaggccgagcctccctttggcgactcctacatcatcattggcgtggagcccggacagctcaagctgaactggttcaagaag

SEQ ID NO: 122 - protein, 394 aa, synthetic construct
  REGION 1..394: note = DENV2 SC.16 (I2-U6-H3)
MRCIGMSNRDFVEGVSGGSWVDIVLEPGSCVTTMAKNKPTLDFELIKIEAKQPATLRKYCIEAKLTNTTTESRCPTQGEPSLNEEQDKRFVCKHSMVDRGWGNGCGLFGKGGIVTCAMFRCKKNMEGKVVQPENLEYTIVITPHSGEEHAVGNDTGKHGKEIKITPQSSITEAELTGYGTVTMECSPRTGLDFNEMVLLQMENKAWLVHRQWFLDLPLPWLPGADTQGSNWIQKETLVTFKNPHAKKQDVVVLGSQEGWMHRALTGATEIQMSSGNLLWPGHLKCRLRMDKLQLKGMSYSMCTGKFKVVKEIAETQHGTIVIRVQYEGDGSPCKIPFEIMDLEKRHVLGRLITVNPIVTEKDSPVNIEAEPPFGDSYIIIGVEPGQLKLNWFKK

SEQ ID NO: 123 - DNA, 1182 bp, synthetic construct
  misc_feature 1..1182: note = DENV2 SC.17 (I2-U6-P4)
  source 1..1182: mol_type = other DNA
atgaggtgtatcggcatgtccaacagggactttgtggagggagtgagcggcggcagctgggtggacattgtgctggagcatggaaagtgcgtgaccgtgatgatgaaaaacaagcccaccctggacttcgagctcatcaagacagaggctaaacagcccgccaccctcaggaagtactgcatcgaggccaagctgaccaacacaacaaccgagtccagatgccctacacagggcgaacccagcctcaacgaagagcaggacaagaggttcgtgtgcaaacacagcatggtggacaggggctggggcaatggatgcggactcttcggaaaaggcggcatcgtgacctgcgccatgttcaggtgtaaaaagaacatggaaggcaaggtggtgcagcccgaaaatctggagtataccatcgtgattaccccccacagcggagaggagcacgccgtgggcaatgacaccggcaagcacggcaaagagattaagatcaccccccagtcctccattaccgaagctgaactgacaggctacggcaccgtgacaatggagtgtagccccaggaccggactggatttcaacgagatggtcctgctacagatggagaacaaggcctggctcgtgcacaggcaatggtttctggatctgcctctgccttggctgcctggcgccgatacacagggctccaactggatacagaaagagaccctcgtcaccttcaagaatccccatgctaagaagcaggacgtggtggtgctgggcagccaagaaggctggatgcaccgggccctgaccggagctaccgagatccagatgagctccggcaacctgctgtggcccggccatctgaaatgtaggctgaggatggataagctgcaactcaaaggcatgtcctactccatgtgcaccggaaagttcaaggtggtgaaagaaatcgccgaaacacagcacggcaccatcgtgatcagggtgcagtatgagggcgacggctccccctgtaagatccccttcgaaatcatggacctggaaaagaggcacgtgctgggcaggctcatcaccgtgaaccccattgtcacagagaaagactcccccgtgaacatcgaggccgagcctccctttggcgactcctacatcatcattggcgtggagcccggacagctcaagctgaactggttcaagaag

SEQ ID NO: 124 - protein, 394 aa, synthetic construct
  REGION 1..394: note = DENV2 SC.17 (I2-U6-P4)
MRCIGMSNRDFVEGVSGGSWVDIVLEHGKCVTVMMKNKPTLDFELIKTEAKQPATLRKYCIEAKLTNTTTESRCPTQGEPSLNEEQDKRFVCKHSMVDRGWGNGCGLFGKGGIVTCAMFRCKKNMEGKVVQPENLEYTIVITPHSGEEHAVGNDTGKHGKEIKITPQSSITEAELTGYGTVTMECSPRTGLDFNEMVLLQMENKAWLVHRQWFLDLPLPWLPGADTQGSNWIQKETLVTFKNPHAKKQDVVVLGSQEGWMHRALTGATEIQMSSGNLLWPGHLKCRLRMDKLQLKGMSYSMCTGKFKVVKEIAETQHGTIVIRVQYEGDGSPCKIPFEIMDLEKRHVLGRLITVNPIVTEKDSPVNIEAEPPFGDSYIIIGVEPGQLKLNWFKK

SEQ ID NO: 125 - DNA, 1182 bp, synthetic construct
  misc_feature 1..1182: note = DENV2 SC.18 (I2-I8-U4-U6-P4)
  source 1..1182: mol_type = other DNA
atgaggtgtatcggcatgtccaacagggactttgtgttcgccgtgagcggcggcagctgggtggacattgtgctggagcatggaaagtgcgtgaccgtgctgatgaaaaacaagcccaccctggacttcgagctcatcaagacagaggctaaacagcccgccaccctcaggaagtactgcatcgaggccaagctgaccaacacaacaaccgagtccagatgccctacacagggcgaacccagcctcaacgaagagcaggacaagaggttcgtgtgcaaacacagcatggtggacaggggctggggcaatggatgcgacctcttcggaaaaggcggcatcgtgacctgcgccatgttcaggtgtaaaaagaacatggaaggcaaggtggtgcagcccgaaaatctggagtataccatcgtgattaccccccacagcggagaggagcacgccgtgggcaatgacaccggcaagcacggcaaagagattaagatcaccccccagtcctccattaccgaagctgaactgacaggctacggcaccgtgacaatggagtgtagccccaggaccggactggatttcaacgagatggtcctgctacagatggagaacaaggcctggctcgtgcacaggcaatggtttctggatctgcctctgccttggctgcctggcgccgatacacagggctccaactggatacagaaagagaccctcgtcaccttcaagaatccccatgctaagaagcaggacgtggtggtgctgggcagccaagaaggctggatgcaccgggccctgaccggagctaccgagatccagatgagctccggcaacctgctgtggcccggccatctgaaatgtaggctgaggatggataagctgcaactcaaaggcatgtcctactccatgtgcaccggaaagttcaaggtggtgaaagaaatcgccgaaacacagcacggcaccatcgtgatcagggtgcagtatgagggcgacggctccccctgtaagatccccttcgaaatcatggacctggaaaagaggcacgtgctgggcaggctcatcaccgtgaaccccattgtcacagagaaagactcccccgtgaacatcgaggccgagcctccctttggcgactcctacatcatcattggcgtggagcccggacagctcaagctgaactggttcaagaag

SEQ ID NO: 126 - protein, 394 aa, synthetic construct
  REGION 1..394: note = DENV2 SC.18 (I2-I8-U4-U6-P4)
MRCIGMSNRDFVFAVSGGSWVDIVLEHGKCVTVLMKNKPTLDFELIKTEAKQPATLRKYCIEAKLTNTTTESRCPTQGEPSLNEEQDKRFVCKHSMVDRGWGNGCDLFGKGGIVTCAMFRCKKNMEGKVVQPENLEYTIVITPHSGEEHAVGNDTGKHGKEIKITPQSSITEAELTGYGTVTMECSPRTGLDFNEMVLLQMENKAWLVHRQWFLDLPLPWLPGADTQGSNWIQKETLVTFKNPHAKKQDVVVLGSQEGWMHRALTGATEIQMSSGNLLWPGHLKCRLRMDKLQLKGMSYSMCTGKFKVVKEIAETQHGTIVIRVQYEGDGSPCKIPFEIMDLEKRHVLGRLITVNPIVTEKDSPVNIEAEPPFGDSYIIIGVEPGQLKLNWFKK

SEQ ID NO: 127 - DNA, 1182 bp, synthetic construct
  misc_feature 1..1182: note = DENV2 SC.19 (I8-U5-U6-P4)
  source 1..1182: mol_type = other DNA
atgaggtgtatcggcatgtccaacagggactttgtggagggagtgagcggcggcagctgggtggacattgtgctggagcatggaaagtgcgtgaccgtgatgatgaaaaacaagcccaccctggacttcgagctcatcaagacagaggctaaacagcccgccaccctcaggaagtactgcatcgaggccaagctgaccaacacaacaaccgagtccagatgccctacacagggcgaacccagcctcaacgaagagcaggacaagaggttcgtgtgcaaacacagcatggtggacaggggctggggcaatggatgcgacctcttcggaaaaggcggcatcgtgacctgcgccatgttcaggtgtaaaaagaacatggaaggcaaggtggtgcagcccgaaaatctggagtataccatcgtgattaccccccacagcggagaggagcacgccgtgggcaatgacaccggcaagcacggcaaagagattaagatcaccccccagtcctccattaccgaagctgaactgacaggctacggcaccgtgacaatggagtgtagccccaggaccggactggatttcaacgagatggtcctgctacagatggagaacaaggcctggctcgtgcacaggcaatggtttctggatctgcctctgccttggctgcctggcgccgatacacagggctccaactggatacagaaagagaccctcgtcaccttcaagaatccccatgctaagaagcaggacgtggtggtgctgggcagccaagaaggcgccatgcacacagccctgaccggagctaccgagatccagatgagctccggcaacctgctgtggcccggccatctgaaatgtaggctgaggatggataagctgcaactcaaaggcatgtcctactccatgtgcaccggaaagttcaaggtggtgaaagaaatcgccgaaacacagcacggcaccatcgtgatcagggtgcagtatgagggcgacggctccccctgtaagatccccttcgaaatcatggacctggaaaagaggcacgtgctgggcaggctcatcaccgtgaaccccattgtctacgagaaagactcccccgtgaacatcgaggccgagcctccctttggcgactcctacatcatcattggcgtggagcccggacagctcaagctgaactggttcaagaag

SEQ ID NO: 128 - protein, 394 aa, synthetic construct
  REGION 1..394: note = DENV2 SC.19 (I8-U5-U6-P4)
MRCIGMSNRDFVEGVSGGSWVDIVLEHGKCVTVMMKNKPTLDFELIKTEAKQPATLRKYCIEAKLTNTTTESRCPTQGEPSLNEEQDKRFVCKHSMVDRGWGNGCDLFGKGGIVTCAMFRCKKNMEGKVVQPENLEYTIVITPHSGEEHAVGNDTGKHGKEIKITPQSSITEAELTGYGTVTMECSPRTGLDFNEMVLLQMENKAWLVHRQWFLDLPLPWLPGADTQGSNWIQKETLVTFKNPHAKKQDVVVLGSQEGAMHTALTGATEIQMSSGNLLWPGHLKCRLRMDKLQLKGMSYSMCTGKFKVVKEIAETQHGTIVIRVQYEGDGSPCKIPFEIMDLEKRHVLGRLITVNPIVYEKDSPVNIEAEPPFGDSYIIIGVEPGQLKLNWFKK

SEQ ID NO: 129 - DNA, 1182 bp, synthetic construct
  misc_feature 1..1182: note = DENV2 SC.20 (P4-U4)
  source 1..1182: mol_type = other DNA
atgaggtgtatcggcatgtccaacagggactttgtgttcgccgtgagcggcggcagctgggtggacattgtgctggagcatggaaagtgcgtgaccgtgctgatgaaaaacaagcccaccctggacttcgagctcatcaagacagaggctaaacagcccgccaccctcaggaagtactgcatcgaggccaagctgaccaacacaacaaccgagtccagatgccctacacagggcgaacccagcctcaacgaagagcaggacaagaggttcgtgtgcaaacacagcatggtggacaggggctggggcaatggatgcggactcttcggaaaaggcggcatcgtgacctgcgccatgttcaggtgtaaaaagaacatggaaggcaaggtggtgcagcccgaaaatctggagtataccatcgtgattaccccccacagcggagaggagcacgccgtgggcaatgacaccggcaagcacggcaaagagattaagatcaccccccagtcctccattaccgaagctgaactgacaggctacggcaccgtgacaatggagtgtagccccaggaccggactggatttcaacgagatggtcctgctacagatggagaacaaggcctggctcgtgcacaggcaatggtttctggatctgcctctgccttggctgcctggcgccgatacacagggctccaactggatacagaaagagaccctcgtcaccttcaagaatccccatgctaagaagcaggacgtggtggtgctgggcagccaagaaggcgccatgcacacagccctgaccggagctaccgagatccagatgagctccggcaacctgctgttcaccggccatctgaaatgtaggctgaggatggataagctgcaactcaaaggcatgtcctactccatgtgcaccggaaagttcaaggtggtgaaagaaatcgccgaaacacagcacggcaccatcgtgatcagggtgcagtatgagggcgacggctccccctgtaagatccccttcgaaatcatggacctggaaaagaggcacgtgctgggcaggctcatcaccgtgaaccccattgtcacagagaaagactcccccgtgaacatcgaggccgagcctccctttggcgactcctacatcatcattggcgtggagcccggacagctcaagctgaactggttcaagaag

SEQ ID NO: 130 - protein, 394 aa, synthetic construct
  REGION 1..394: note = DENV2 SC.20 (P4-U4)
MRCIGMSNRDFVFAVSGGSWVDIVLEHGKCVTVLMKNKPTLDFELIKTEAKQPATLRKYCIEAKLTNTTTESRCPTQGEPSLNEEQDKRFVCKHSMVDRGWGNGCGLFGKGGIVTCAMFRCKKNMEGKVVQPENLEYTIVITPHSGEEHAVGNDTGKHGKEIKITPQSSITEAELTGYGTVTMECSPRTGLDFNEMVLLQMENKAWLVHRQWFLDLPLPWLPGADTQGSNWIQKETLVTFKNPHAKKQDVVVLGSQEGAMHTALTGATEIQMSSGNLLFTGHLKCRLRMDKLQLKGMSYSMCTGKFKVVKEIAETQHGTIVIRVQYEGDGSPCKIPFEIMDLEKRHVLGRLITVNPIVTEKDSPVNIEAEPPFGDSYIIIGVEPGQLKLNWFKK

SEQ ID NO: 131 - DNA, 1182 bp, synthetic construct
  misc_feature 1..1182: note = DENV2 SC.21 (U4-U5-U6)
  source 1..1182: mol_type = other DNA
atgaggtgtatcggcatgtccaacagggactttgtgttcgccgtgagcggcggcagctgggtggacattgtgctggagcatggaagctgcgtgaccacgctggcgaaaaacaagcccaccctggacttcgagctcatcaagacagaggctaaacagcccgccaccctcaggaagtactgcatcgaggccaagctgaccaacacaacaaccgagtccagatgccctacacagggcgaacccagcctcaacgaagagcaggacaagaggttcgtgtgcaaacacagcatggtggacaggggctggggcaatggatgcggactcttcggaaaaggcggcatcgtgacctgcgccatgttcaggtgtaaaaagaacatggaaggcaaggtggtgcagcccgaaaatctggagtataccatcgtgattaccccccacagcggagaggagcacgccgtgggcaatgacaccggcaagcacggcaaagagattaagatcaccccccagtcctccattaccgaagctgaactgacaggctacggcaccgtgacaatggagtgtagccccaggaccggactggatttcaacgagatggtcctgctacagatggagaacaaggcctggctcgtgcacaggcaatggtttctggatctgcctctgccttggctgcctggcgccgatacacagggctccaactggatacagaaagagaccctcgtcaccttcaagaatccccatgctaagaagcaggacgtggtggtgctgggcagccaagaaggcgccatgcacacagccctgaccggagctaccgagatccagatgagctccggcaacctgctgtggcccggccatctgaaatgtaggctgaggatggataagctgcaactcaaaggcatgtcctactccatgtgcaccggaaagttcaaggtggtgaaagaaatcgccgaaacacagcacggcaccatcgtgatcagggtgcagtatgagggcgacggctccccctgtaagatccccttcgaaatcatggacctggaaaagaggcacgtgctgggcaggctcatcaccgtgaaccccattgtctacgagaaagactcccccgtgaacatcgaggccgagcctccctttggcgactcctacatcatcattggcgtggagcccggacagctcaagctgaactggttcaagaag

SEQ ID NO: 132 - protein, 394 aa, synthetic construct
  REGION 1..394: note = DENV2 SC.21 (U4-U5-U6)
MRCIGMSNRDFVFAVSGGSWVDIVLEHGSCVTTLAKNKPTLDFELIKTEAKQPATLRKYCIEAKLTNTTTESRCPTQGEPSLNEEQDKRFVCKHSMVDRGWGNGCGLFGKGGIVTCAMFRCKKNMEGKVVQPENLEYTIVITPHSGEEHAVGNDTGKHGKEIKITPQSSITEAELTGYGTVTMECSPRTGLDFNEMVLLQMENKAWLVHRQWFLDLPLPWLPGADTQGSNWIQKETLVTFKNPHAKKQDVVVLGSQEGAMHTALTGATEIQMSSGNLLWPGHLKCRLRMDKLQLKGMSYSMCTGKFKVVKEIAETQHGTIVIRVQYEGDGSPCKIPFEIMDLEKRHVLGRLITVNPIVYEKDSPVNIEAEPPFGDSYIIIGVEPGQLKLNWFKK

SEQ ID NO: 133 - DNA, 1182 bp, synthetic construct
  misc_feature 1..1182: note = DENV2 SC.22 (U4-U5-U6-P5)
  source 1..1182: mol_type = other DNA
atgaggtgtatcggcatgtccaacagggactttgtgttcgccgtgagcggcggcagctgggtggacattgtgctggagcatggaagctgcgtgaccacgctggcgaaaaacaagcccaccctggacttcgagctcatcaagacagaggctaaacagcccgccaccctcaggaagtactgcatcgaggccaagctgaccaacacaacaaccgagtccagatgccctacacagggcgaacccagcctcaacgaagagcaggacaagaggttcgtgtgcaaacacagcatggtggacaggggctggggcaatggatgcggactcttcggaaaaggcggcatcgtgacctgcgccatgttcaggtgtaaaaagaacatggaaggcaaggtggtgcagcccgaaaatctggagtataccatcgtgattaccccccacagcggagaggagcacgccgtgggcaatgacaccggcaagcacggcaaagagattaagatcaccccccagtcctccattaccgaagctgaactgacaggctacggcaccgtgacaatggagtgtagccccaggaccggactggatttcaacgagatggtcctgctacagatggagaacaaggcctggctcgtggacaggcaatggtttctggatctgcctctgccttggctgcctggcgccgatacacagggctccaactggatacagaaagagaccctcgtcaccttcaagaatccccatgctaagaagcaggacgtggtggtgctgggcagccaagaaggcgccatgcacacagccctgacctgggctaccgagatccagatgagctccggcaacctgctgtggcccggccatctgaaatgtaggctgaggatggataagctgcaactcaaaggcatgtcctactccatgtgcaccggaaagttcaaggtggtgaaagaaatcgccgaaacacagcacggcaccatcgtgatcagggtgcagtatgagggcgacggctccccctgtaagatccccttcgaaatcatggacctggaaaagaggcacgtgctgggcaggctcatcaccgtgaaccccattgtctacgagaaagactcccccgtgaacatcgaggccgagcctccctttggcgactcctacatcatcattggcgtggagcccggacagctcaagctgaactggttcaagaag

SEQ ID NO: 134 - protein, 394 aa, synthetic construct
  REGION 1..394: note = DENV2 SC.22 (U4-U5-U6-P5)
MRCIGMSNRDFVFAVSGGSWVDIVLEHGSCVTTLAKNKPTLDFELIKTEAKQPATLRKYCIEAKLTNTTTESRCPTQGEPSLNEEQDKRFVCKHSMVDRGWGNGCGLFGKGGIVTCAMFRCKKNMEGKVVQPENLEYTIVITPHSGEEHAVGNDTGKHGKEIKITPQSSITEAELTGYGTVTMECSPRTGLDFNEMVLLQMENKAWLVDRQWFLDLPLPWLPGADTQGSNWIQKETLVTFKNPHAKKQDVVVLGSQEGAMHTALTWATEIQMSSGNLLWPGHLKCRLRMDKLQLKGMSYSMCTGKFKVVKEIAETQHGTIVIRVQYEGDGSPCKIPFEIMDLEKRHVLGRLITVNPIVYEKDSPVNIEAEPPFGDSYIIIGVEPGQLKLNWFKK

SEQ ID NO: 135 - DNA, 1182 bp, synthetic construct
  misc_feature 1..1182: note = DENV2 SC.23 (I2-I8)
  source 1..1182: mol_type = other DNA
atgaggtgtatcggcatgtccaacagggactttgtggagggagtgagcggcggcagctgggtggacattgtgctggagcatggaagctgcgtgaccacgatggcgaaaaacaagcccaccctggacttcgagctcatcaagacagaggctaaacagcccgccaccctcaggaagtactgcatcgaggccaagctgaccaacacaacaaccgagtccagatgccctacacagggcgaacccagcctcaacgaagagcaggacaagaggttcgtgtgcaaacacagcatggtggacaggggctggggcaatggatgcgacctcttcggaaaaggcggcatcgtgacctgcgccatgttcaggtgtaaaaagaacatggaaggcaaggtggtgcagcccgaaaatctggagtataccatcgtgattaccccccacagcggagaggagcacgccgtgggcaatgacaccggcaagcacggcaaagagattaagatcaccccccagtcctccattaccgaagctgaactgacaggctacggcaccgtgacaatggagtgtagccccaggaccggactggatttcaacgagatggtcctgctacagatggagaacaaggcctggctcgtgcacaggcaatggtttctggatctgcctctgccttggctgcctggcgccgatacacagggctccaactggatacagaaagagaccctcgtcaccttcaagaatccccatgctaagaagcaggacgtggtggtgctgggcagccaagaaggctggatgcaccgggccctgaccggagctaccgagatccagatgagctccggcaacctgctgttcaccggccatctgaaatgtaggctgaggatggataagctgcaactcaaaggcatgtcctactccatgtgcaccggaaagttcaaggtggtgaaagaaatcgccgaaacacagcacggcaccatcgtgatcagggtgcagtatgagggcgacggctccccctgtaagatccccttcgaaatcatggacctggaaaagaggcacgtgctgggcaggctcatcaccgtgaaccccattgtcacagagaaagactcccccgtgaacatcgaggccgagcctccctttggcgactcctacatcatcattggcgtggagcccggacagctcaagctgaactggttcaagaag

SEQ ID NO: 136 - protein, 394 aa, synthetic construct
  REGION 1..394: note = DENV2 SC.23 (I2-I8)
MRCIGMSNRDFVEGVSGGSWVDIVLEHGSCVTTMAKNKPTLDFELIKTEAKQPATLRKYCIEAKLTNTTTESRCPTQGEPSLNEEQDKRFVCKHSMVDRGWGNGCDLFGKGGIVTCAMFRCKKNMEGKVVQPENLEYTIVITPHSGEEHAVGNDTGKHGKEIKITPQSSITEAELTGYGTVTMECSPRTGLDFNEMVLLQMENKAWLVHRQWFLDLPLPWLPGADTQGSNWIQKETLVTFKNPHAKKQDVVVLGSQEGWMHRALTGATEIQMSSGNLLFTGHLKCRLRMDKLQLKGMSYSMCTGKFKVVKEIAETQHGTIVIRVQYEGDGSPCKIPFEIMDLEKRHVLGRLITVNPIVTEKDSPVNIEAEPPFGDSYIIIGVEPGQLKLNWFKK

SEQ ID NO: 137 - DNA, 1182 bp, synthetic construct
  misc_feature 1..1182: note = DENV2 SC.24 (M2-H3)
  source 1..1182: mol_type = other DNA
atgaggtgtatcggcatgtccaacagggactttgtggagggagtgagcggcggcagctgggtggacattgtgctggagcccggaagctgcgtgaccacgatggcgaaaaacaagcccaccctggacttcgagctcatcaagatcgaggctaaacagcccgccaccctcaggaagtactgcatcgaggccaagctgaccaacacaacaaccgagtccagatgccctacacagggcgaacccagcctcaacgaagagcaggacaagaggttcgtgtgcaaacacagcatggtggacaggggctggggcaatggatgcggactcttcggaaaaggcggcatcgtgacctgcgccatgttcaggtgtaaaaagaacatggaaggcaaggtggtgcagcccgaaaatctggagtataccatcgtgattaccccccacagcggagaggagcacgccgtgggcaatgacaccggcaagcacggcaaagagattaagatcaccccccagtcctccattaccgaagctgaactgacaggctacggcaccgtgacaatggagtgtagccccaggaccggactggatttcaacgagatggtcctgctacagatggagaacaaggcctggctcgtgcacaggcaatggtttctggatctgcctctgccttggctgcctggcgccgatacacagggctccaactggatacagaaagagaccctcgtcaccttcaagaatccccatgctaagaagcaggacgtggtggtgctgggcagccaagaagaggccatgcacacagccctgaccggagctaccgagatccagatgagctccggcaacctgctgttcaccggccatctgaaatgtaggctgaggatggataagctgcaactcaaaggcatgtcctactccatgtgcaccggaaagttcaaggtggtgaaagaaatcgccgaaacacagcacggcaccatcgtgatcagggtgcagtatgagggcgacggctccccctgtaagatccccttcgaaatcatggacctggaaaagaggcacgtgctgggcaggctcatcaccgtgaaccccattgtcacagagaaagactcccccgtgaacatcgaggccgagcctccctttggcgactcctacatcatcattggcgtggagcccggacagctcaagctgaactggttcaagaag

SEQ ID NO: 138 - protein, 394 aa, synthetic construct
  REGION 1..394: note = DENV2 SC.24 (M2-H3)
MRCIGMSNRDFVEGVSGGSWVDIVLEPGSCVTTMAKNKPTLDFELIKIEAKQPATLRKYCIEAKLTNTTTESRCPTQGEPSLNEEQDKRFVCKHSMVDRGWGNGCGLFGKGGIVTCAMFRCKKNMEGKVVQPENLEYTIVITPHSGEEHAVGNDTGKHGKEIKITPQSSITEAELTGYGTVTMECSPRTGLDFNEMVLLQMENKAWLVHRQWFLDLPLPWLPGADTQGSNWIQKETLVTFKNPHAKKQDVVVLGSQEEAMHTALTGATEIQMSSGNLLFTGHLKCRLRMDKLQLKGMSYSMCTGKFKVVKEIAETQHGTIVIRVQYEGDGSPCKIPFEIMDLEKRHVLGRLITVNPIVTEKDSPVNIEAEPPFGDSYIIIGVEPGQLKLNWFKK

SEQ ID NO: 139 - DNA, 1183 bp, synthetic construct
  misc_feature 1..1183: note = DENV2 SC.25 (M2-P4)
  source 1..1183: mol_type = other DNA
catgaggtgtatcggcatgtccaacagggactttgtggagggagtgagcggcggcagctgggtggacattgtgctggagcatggaaagtgcgtgaccgtgatgatgaaaaacaagcccaccctggacttcgagctcatcaagacagaggctaaacagcccgccaccctcaggaagtactgcatcgaggccaagctgaccaacacaacaaccgagtccagatgccctacacagggcgaacccagcctcaacgaagagcaggacaagaggttcgtgtgcaaacacagcatggtggacaggggctggggcaatggatgcggactcttcggaaaaggcggcatcgtgacctgcgccatgttcaggtgtaaaaagaacatggaaggcaaggtggtgcagcccgaaaatctggagtataccatcgtgattaccccccacagcggagaggagcacgccgtgggcaatgacaccggcaagcacggcaaagagattaagatcaccccccagtcctccattaccgaagctgaactgacaggctacggcaccgtgacaatggagtgtagccccaggaccggactggatttcaacgagatggtcctgctacagatggagaacaaggcctggctcgtgcacaggcaatggtttctggatctgcctctgccttggctgcctggcgccgatacacagggctccaactggatacagaaagagaccctcgtcaccttcaagaatccccatgctaagaagcaggacgtggtggtgctgggcagccaagaagaggccatgcacacagccctgaccggagctaccgagatccagatgagctccggcaacctgctgttcaccggccatctgaaatgtaggctgaggatggataagctgcaactcaaaggcatgtcctactccatgtgcaccggaaagttcaaggtggtgaaagaaatcgccgaaacacagcacggcaccatcgtgatcagggtgcagtatgagggcgacggctccccctgtaagatccccttcgaaatcatggacctggaaaagaggcacgtgctgggcaggctcatcaccgtgaaccccattgtcacagagaaagactcccccgtgaacatcgaggccgagcctccctttggcgactcctacatcatcattggcgtggagcccggacagctcaagctgaactggttcaagaag

SEQ ID NO: 140 - protein, 394 aa, synthetic construct
  REGION 1..394: note = DENV2 SC.25 (M2-P4)
MRCIGMSNRDFVEGVSGGSWVDIVLEHGKCVTVMMKNKPTLDFELIKTEAKQPATLRKYCIEAKLTNTTTESRCPTQGEPSLNEEQDKRFVCKHSMVDRGWGNGCGLFGKGGIVTCAMFRCKKNMEGKVVQPENLEYTIVITPHSGEEHAVGNDTGKHGKEIKITPQSSITEAELTGYGTVTMECSPRTGLDFNEMVLLQMENKAWLVHRQWFLDLPLPWLPGADTQGSNWIQKETLVTFKNPHAKKQDVVVLGSQEEAMHTALTGATEIQMSSGNLLFTGHLKCRLRMDKLQLKGMSYSMCTGKFKVVKEIAETQHGTIVIRVQYEGDGSPCKIPFEIMDLEKRHVLGRLITVNPIVTEKDSPVNIEAEPPFGDSYIIIGVEPGQLKLNWFKK

SEQ ID NO: 141 - DNA, 1182 bp, synthetic construct
  misc_feature 1..1182: note = DENV2 SC.26 (I3-I8-U6)
  source 1..1182: mol_type = other DNA
atgaggtgtatcggcatgtccaacagggactttgtggagggagtgagcggcggcagctgggtggacattgtgctggagcatggaagctgcgtgaccacgatggcgaaaaacaagcccaccctggacttcgagctcatcaagacagaggctaaacagcccgccaccctcaggaagtactgcatcgaggccaagctgaccaacacaacaaccgagtccagatgccctacacagggcgaacccagcctcaacgaagagcaggacaagaggttcgtgtgcaaacacagcatggtggacaggggctggggcaatggatgcgacctcttcggaaaaggcggcatcgtgacctgcgccatgttcaggtgtaaaaagaacatggaaggcaaggtggtgcagcccgaaaatctggagtataccatcgtgattaccccccacagcggagaggagcacgccgtgggcaatgacaccggcaagcacggcaaagagattaagatcaccccccagtcctccattaccgaagctgaactgacaggctacggcaccgtgacaatggagtgtagccccaggaccggactggatttcaacgagatggtcctgctacagatggagaacaaggcctggctcgtgcacaggcaatggtttctggatctgcctctgccttggctgcctggcgccgatacacagggctccaactggatacagaaagagaccctcgtcaccttcaagaatccccatgctaagaagcaggacgtggtggtgctgggcagccaagaaggcgtgatgcaccggtggctgaccggagctaccgagatccagatgagctccggcaacctgctgtggcccggccatctgaaatgtaggctgaggatggataagctgcaactcaaaggcatgtcctactccatgtgcaccggaaagttcaaggtggtgaaagaaatcgccgaaacacagcacggcaccatcgtgatcagggtgcagtatgagggcgacggctccccctgtaagatccccttcgaaatcatggacctggaaaagaggcacgtgctgggcaggctcatcaccgtgaaccccattgtcacagagaaagactcccccgtgaacatcgaggccgagcctccctttggcgactcctacatcatcattggcgtggagcccggacagctcaagctgaactggttcaagaag

SEQ ID NO: 142 - protein, 394 aa, synthetic construct
  REGION 1..394: note = DENV2 SC.26 (I3-I8-U6)
MRCIGMSNRDFVEGVSGGSWVDIVLEHGSCVTTMAKNKPTLDFELIKTEAKQPATLRKYCIEAKLTNTTTESRCPTQGEPSLNEEQDKRFVCKHSMVDRGWGNGCDLFGKGGIVTCAMFRCKKNMEGKVVQPENLEYTIVITPHSGEEHAVGNDTGKHGKEIKITPQSSITEAELTGYGTVTMECSPRTGLDFNEMVLLQMENKAWLVHRQWFLDLPLPWLPGADTQGSNWIQKETLVTFKNPHAKKQDVVVLGSQEGVMHRWLTGATEIQMSSGNLLWPGHLKCRLRMDKLQLKGMSYSMCTGKFKVVKEIAETQHGTIVIRVQYEGDGSPCKIPFEIMDLEKRHVLGRLITVNPIVTEKDSPVNIEAEPPFGDSYIIIGVEPGQLKLNWFKK

SEQ ID NO: 143 - DNA, 1182 bp, synthetic construct
  misc_feature 1..1182: note = DENV2 SC.27 (I3-I8-U6-P4)
  source 1..1182: mol_type = other DNA
atgaggtgtatcggcatgtccaacagggactttgtggagggagtgagcggcggcagctgggtggacattgtgctggagcatggaaagtgcgtgaccgtgatgatgaaaaacaagcccaccctggacttcgagctcatcaagacagaggctaaacagcccgccaccctcaggaagtactgcatcgaggccaagctgaccaacacaacaaccgagtccagatgccctacacagggcgaacccagcctcaacgaagagcaggacaagaggttcgtgtgcaaacacagcatggtggacaggggctggggcaatggatgcgacctcttcggaaaaggcggcatcgtgacctgcgccatgttcaggtgtaaaaagaacatggaaggcaaggtggtgcagcccgaaaatctggagtataccatcgtgattaccccccacagcggagaggagcacgccgtgggcaatgacaccggcaagcacggcaaagagattaagatcaccccccagtcctccattaccgaagctgaactgacaggctacggcaccgtgacaatggagtgtagccccaggaccggactggatttcaacgagatggtcctgctacagatggagaacaaggcctggctcgtgcacaggcaatggtttctggatctgcctctgccttggctgcctggcgccgatacacagggctccaactggatacagaaagagaccctcgtcaccttcaagaatccccatgctaagaagcaggacgtggtggtgctgggcagccaagaaggcgtgatgcaccggtggctgaccggagctaccgagatccagatgagctccggcaacctgctgtggcccggccatctgaaatgtaggctgaggatggataagctgcaactcaaaggcatgtcctactccatgtgcaccggaaagttcaaggtggtgaaagaaatcgccgaaacacagcacggcaccatcgtgatcagggtgcagtatgagggcgacggctccccctgtaagatccccttcgaaatcatggacctggaaaagaggcacgtgctgggcaggctcatcaccgtgaaccccattgtcacagagaaagactcccccgtgaacatcgaggccgagcctccctttggcgactcctacatcatcattggcgtggagcccggacagctcaagctgaactggttcaagaag

SEQ ID NO: 144 - protein, 394 aa, synthetic construct
  REGION 1..394: note = DENV2 SC.27 (I3-I8-U6-P4)
MRCIGMSNRDFVEGVSGGSWVDIVLEHGKCVTVMMKNKPTLDFELIKTEAKQPATLRKYCIEAKLTNTTTESRCPTQGEPSLNEEQDKRFVCKHSMVDRGWGNGCDLFGKGGIVTCAMFRCKKNMEGKVVQPENLEYTIVITPHSGEEHAVGNDTGKHGKEIKITPQSSITEAELTGYGTVTMECSPRTGLDFNEMVLLQMENKAWLVHRQWFLDLPLPWLPGADTQGSNWIQKETLVTFKNPHAKKQDVVVLGSQEGVMHRWLTGATEIQMSSGNLLWPGHLKCRLRMDKLQLKGMSYSMCTGKFKVVKEIAETQHGTIVIRVQYEGDGSPCKIPFEIMDLEKRHVLGRLITVNPIVTEKDSPVNIEAEPPFGDSYIIIGVEPGQLKLNWFKK

SEQ ID NO: 145 - DNA, 1182 bp, synthetic construct
  misc_feature 1..1182: note = DENV2 SC.28 (P4-Cm2)
  source 1..1182: mol_type = other DNA
atgaggtgtatcggcatgtccaacagggactttgtggagggagtgagcggcggcagctgggtggacattgtgctggagcatggaaagtgcgtgaccgtgatgatgaaaaacaagcccaccctggacttcgagctcatcaagacagaggctaaacagcccgccaccctcaggaagtactgcatcgaggccaagctgaccaacacaacaaccgagtccagatgccctacacagggcgaacccagcctcaacgaagagcaggacaagaggttcgtgtgcaaacacagcatggtggacaggggctggggcaatggatgcggatgtttcggaaaaggcggcatcgtgacctgcgccatgttcaggtgtaaaaagaacatggaaggcaaggtggtgcagcccgaaaatctggagtataccatcgtgattaccccccacagcggagaggagcacgccgtgggcaatgacaccggcaagcacggcaaagagattaagatcaccccccagtcctccattaccgaagctgaactgacaggctacggcaccgtgacaatggagtgtagccccaggaccggactggatttcaacgagatggtcctgctacagatggagaacaaggcctggctcgtgcacaggcaatggtttctggatctgcctctgccttggctgcctggcgccgatacacagggctccaactggatacagaaagagaccctcgtcaccttcaagaatccccatgctaagaagcaggacgtggtggtgctgggcagccaagaaggcgccatgcacacagccctgaccggagctaccgagatccagatgagctccggcaacctgctgttcaccggccatctgaaatgtaggctgaggatggataagctgcaactcaaaggcatgtcctactccatgtgcaccggaaagttcaaggtggtgaaagaaatctgtgaaacacagcacggcaccatcgtgatcagggtgcagtatgagggcgacggctccccctgtaagatccccttcgaaatcatggacctggaaaagaggcacgtgctgggcaggctcatcaccgtgaaccccattgtcacagagaaagactcccccgtgaacatcgaggccgagcctccctttggcgactcctacatcatcattggcgtggagcccggacagctcaagctgaactggttcaagaag

SEQ ID NO: 146 - protein, 394 aa, synthetic construct
  REGION 1..394: note = DENV2 SC.28 (P4-Cm2)
MRCIGMSNRDFVEGVSGGSWVDIVLEHGKCVTVMMKNKPTLDFELIKTEAKQPATLRKYCIEAKLTNTTTESRCPTQGEPSLNEEQDKRFVCKHSMVDRGWGNGCGCFGKGGIVTCAMFRCKKNMEGKVVQPENLEYTIVITPHSGEEHAVGNDTGKHGKEIKITPQSSITEAELTGYGTVTMECSPRTGLDFNEMVLLQMENKAWLVHRQWFLDLPLPWLPGADTQGSNWIQKETLVTFKNPHAKKQDVVVLGSQEGAMHTALTGATEIQMSSGNLLFTGHLKCRLRMDKLQLKGMSYSMCTGKFKVVKEICETQHGTIVIRVQYEGDGSPCKIPFEIMDLEKRHVLGRLITVNPIVTEKDSPVNIEAEPPFGDSYIIIGVEPGQLKLNWFKK

SEQ ID NO: 147 - protein, 394 aa, synthetic construct
  REGION 1..394: note = DENV1 sE WT
MRCVGIGNRDFVEGLSGATWVDVVLEHGSCVTTMAKDKPTLDIELLKTEVTNPAVLRKLCIEAKISNTTTDSRCPTQGEATLVEEQDTNFVCRRTFVDRGWGNGCGLFGKGSLITCAKFKCVTKLEGKIVQYENLKYSVIVTVHTGDQHQVGNETTEHGTTATITPQAPTSEIQLTDYGALTLDCSPRTGLDFNEMVLLTMEKKSWLVHKQWFLDLPLPWTSGASTSQETWNRQDLLVTFKTAHAKKQEVVVLGSQEGAMHTALTGATEIQTSGTTTIFAGHLKCRLKMDKLTLKGMSYVMCTGSFKLEKEVAETQHGTVLVQVKYEGTDAPCKIPFSSQDEKGVTQNGRLITANPIVTDKEKPVNIEAEPPFGESYIVVGAGEKALKLSWFKK

SEQ ID NO: 148 - protein, 394 aa, synthetic construct
  REGION 1..394: note = DENV1 sE PM4
MRCVGIGNRDFVEGLSGATWVDVVLEHGKCVTVMMKDKPTLDIELLKTEVTNPAVLRKLCIEAKISNTTTDSRCPTQGEATLVEEQDTNFVCRRTFVDRGWGNGCGLFGKGSLITCAKFKCVTKLEGKIVQYENLKYSVIVTVHTGDQHQVGNETTEHGTTATITPQAPTSEIQLTDYGALTLDCSPRTGLDFNEMVLLTMEKKSWLVHKQWFLDLPLPWTSGASTSQETWNRQDLLVTFKTAHAKKQEVVVLGSQEGAMHTALTGATEIQTSGTTTIFAGHLKCRLKMDKLTLKGMSYVMCTGSFKLEKEVAETQHGTVLVQVKYEGTDAPCKIPFSSQDEKGVTQNGRLITANPIVTDKEKPVNIEAEPPFGESYIVVGAGEKALKLSWFKK

SEQ ID NO: 149 - protein, 394 aa, synthetic construct
  REGION 1..394: note = DENV1 sE IntFc2
MRCVGIGNRDFVEGLSGATWVDVVLEHGSCVTTMAKDKPTLDIELLKTEVTNPAVLRKLCIEAKISNTTTDSRCPTQGEATLVEEQDTNFVCRRTFVDRGWGNGCGLFGKGSLITCAKFKCVTKLEGKIVQYENLKYSVIVTVHTGDQHQVGNETTEHGTTATITPQAPTSEIQLTDYGALTLDCSPRTGLDFNEMVLLTMEKKSWLVHKQWFLDLPLPWTSGASTSQETWNRQDLLVTFKTAHAKKQEVVVLGSQEGWMHRALTGATEIQTSGTTTIFAGHLKCRLKMDKLTLKGMSYVMCTGSFKLEKEVAETQHGTVLVQVKYEGTDAPCKIPFSSQDEKGVTQNGRLITANPIVTDKEKPVNIEAEPPFGESYIVVGAGEKALKLSWFKK

SEQ ID NO: 150 - protein, 394 aa, synthetic construct
  REGION 1..394: note = DENV1 sE IntFc8
MRCVGIGNRDFVEGLSGATWVDVVLEHGSCVTTMAKDKPTLDIELLKTEVTNPAVLRKLCIEAKISNTTTDSRCPTQGEATLVEEQDTNFVCRRTFVDRGWGNGCDLFGKGSLITCAKFKCVTKLEGKIVQYENLKYSVIVTVHTGDQHQVGNETTEHGTTATITPQAPTSEIQLTDYGALTLDCSPRTGLDFNEMVLLTMEKKSWLVHKQWFLDLPLPWTSGASTSQETWNRQDLLVTFKTAHAKKQEVVVLGSQEGAMHTALTGATEIQTSGTTTIFAGHLKCRLKMDKLTLKGMSYVMCTGSFKLEKEVAETQHGTVLVQVKYEGTDAPCKIPFSSQDEKGVTQNGRLITANPIVTDKEKPVNIEAEPPFGESYIVVGAGEKALKLSWFKK

SEQ ID NO: 151 - protein, 394 aa, synthetic construct
  REGION 1..394: note = DENV1 sE UndPk6
MRCVGIGNRDFVEGLSGATWVDVVLEHGSCVTTMAKDKPTLDIELLKTEVTNPAVLRKLCIEAKISNTTTDSRCPTQGEATLVEEQDTNFVCRRTFVDRGWGNGCGLFGKGSLITCAKFKCVTKLEGKIVQYENLKYSVIVTVHTGDQHQVGNETTEHGTTATITPQAPTSEIQLTDYGALTLDCSPRTGLDFNEMVLLTMEKKSWLVHKQWFLDLPLPWTSGASTSQETWNRQDLLVTFKTAHAKKQEVVVLGSQEGAMHTALTGATEIQTSGTTTIWPGHLKCRLKMDKLTLKGMSYVMCTGSFKLEKEVAETQHGTVLVQVKYEGTDAPCKIPFSSQDEKGVTQNGRLITANPIVTDKEKPVNIEAEPPFGESYIVVGAGEKALKLSWFKK

SEQ ID NO: 152 - protein, 392 aa, synthetic construct
  REGION 1..392: note = DENV3 sE WT
MRCVGVGNRDFVEGLSGATWVDVVLEHGGCVTTMAKNKPTLDIELQKTEATQLATLRKLCIEGKITNITTDSRCPTQGEAILPEEQDQNYVCKHTYVDRGWGNGCGLFGKGSLVTCAKFQCLESIEGKVVQHENLKYTVIITVHTGDQHQVGNETQGVTAEITPQASTVEAILPEYGTLGLECSPRTGLDFNEMILLTMKNKAWMVHRQWFFDLPLPWTSGATTETPTWNRKELLVTFKNAHAKKQEVVVLGSQEGAMHTALTGATEIQNSGGTSIFAGHLKCRLKMDKLELKGMSYAMCLNTFVLKKEVSETQHGTILIKVEYKGEDAPCKIPFSTEDGQGKAHNGRLITANPVVTKKEEPVNIEAEPPFGESNIVIGIGDKALKINWYKK

SEQ ID NO: 153 - protein, 392 aa, synthetic construct
  REGION 1..392: note = DENV3 sE PM4
MRCVGVGNRDFVEGLSGATWVDVVLEHGKCVTVMMKNKPTLDIELQKTEATQLATLRKLCIEGKITNITTDSRCPTQGEAILPEEQDQNYVCKHTYVDRGWGNGCGLFGKGSLVTCAKFQCLESIEGKVVQHENLKYTVIITVHTGDQHQVGNETQGVTAEITPQASTVEAILPEYGTLGLECSPRTGLDFNEMILLTMKNKAWMVHRQWFFDLPLPWTSGATTETPTWNRKELLVTFKNAHAKKQEVVVLGSQEGAMHTALTGATEIQNSGGTSIFAGHLKCRLKMDKLELKGMSYAMCLNTFVLKKEVSETQHGTILIKVEYKGEDAPCKIPFSTEDGQGKAHNGRLITANPVVTKKEEPVNIEAEPPFGESNIVIGIGDKALKINWYKK

SEQ ID NO: 154 - protein, 392 aa, synthetic construct
  REGION 1..392: note = DENV3 sE IntFc2
MRCVGVGNRDFVEGLSGATWVDVVLEHGGCVTTMAKNKPTLDIELQKTEATQLATLRKLCIEGKITNITTDSRCPTQGEAILPEEQDQNYVCKHTYVDRGWGNGCGLFGKGSLVTCAKFQCLESIEGKVVQHENLKYTVIITVHTGDQHQVGNETQGVTAEITPQASTVEAILPEYGTLGLECSPRTGLDFNEMILLTMKNKAWMVHRQWFFDLPLPWTSGATTETPTWNRKELLVTFKNAHAKKQEVVVLGSQEGWMHRALTGATEIQNSGGTSIFAGHLKCRLKMDKLELKGMSYAMCLNTFVLKKEVSETQHGTILIKVEYKGEDAPCKIPFSTEDGQGKAHNGRLITANPVVTKKEEPVNIEAEPPFGESNIVIGIGDKALKINWYKK

SEQ ID NO: 155 - protein, 392 aa, synthetic construct
  REGION 1..392: note = DENV3 sE IntFc8
MRCVGVGNRDFVEGLSGATWVDVVLEHGGCVTTMAKNKPTLDIELQKTEATQLATLRKLCIEGKITNITTDSRCPTQGEAILPEEQDQNYVCKHTYVDRGWGNGCDLFGKGSLVTCAKFQCLESIEGKVVQHENLKYTVIITVHTGDQHQVGNETQGVTAEITPQASTVEAILPEYGTLGLECSPRTGLDFNEMILLTMKNKAWMVHRQWFFDLPLPWTSGATTETPTWNRKELLVTFKNAHAKKQEVVVLGSQEGAMHTALTGATEIQNSGGTSIFAGHLKCRLKMDKLELKGMSYAMCLNTFVLKKEVSETQHGTILIKVEYKGEDAPCKIPFSTEDGQGKAHNGRLITANPVVTKKEEPVNIEAEPPFGESNIVIGIGDKALKINWYKK

SEQ ID NO: 156 - protein, 392 aa, synthetic construct
  REGION 1..392: note = DENV3 sE UndPk6
MRCVGVGNRDFVEGLSGATWVDVVLEHGGCVTTMAKNKPTLDIELQKTEATQLATLRKLCIEGKITNITTDSRCPTQGEAILPEEQDQNYVCKHTYVDRGWGNGCGLFGKGSLVTCAKFQCLESIEGKVVQHENLKYTVIITVHTGDQHQVGNETQGVTAEITPQASTVEAILPEYGTLGLECSPRTGLDFNEMILLTMKNKAWMVHRQWFFDLPLPWTSGATTETPTWNRKELLVTFKNAHAKKQEVVVLGSQEGAMHTALTGATEIQNSGGTSIWPGHLKCRLKMDKLELKGMSYAMCLNTFVLKKEVSETQHGTILIKVEYKGEDAPCKIPFSTEDGQGKAHNGRLITANPVVTKKEEPVNIEAEPPFGESNIVIGIGDKALKINWYKK

SEQ ID NO: 157 - protein, 392 aa, synthetic construct
  REGION 1..392: note = DENV3 sE UndPk6 DV2Hingemut
MRCVGVGNRDFVEGLSGATWVDVVLEHGGCVTTMAKNKPTLDIELQKTEATQLATLRKLCIEGKITNITTDSRCPTQGEAILPEEQDQNYVCKHTYVDRGWGNGCGLFGKGSLVTCAKFQCLESIEGKVVQHENLKYTVIITVHTGDQHQVGNETQGVTAEITPQASTVEAILPEYGTLGLECSPRTGLDFNEMILLTMKNKAWLVHRQWFFDLPLPWTSGATTETPTWNRKELLVTFKNAHAKKQEVVVLGSQEGAMHTALTGATEIQNSGGTLIWPGHLKCRLKMDKLELKGMSYAMCLNTFVLKKEVSETQHGTILIKVEYKGEDAPCKIPFSTEDGQGKAHNGRLITANPVVTKKEEPVNIEAEPPFGESNIVIGIGDKALKINWYKK

SEQ ID NO: 158 - protein, 392 aa, synthetic construct
  REGION 1..392: note = DENV3 sE SC.10 (I2-I8-U6)
MRCVGVGNRDFVEGLSGATWVDVVLEHGGCVTTMAKNKPTLDIELQKTEATQLATLRKLCIEGKITNITTDSRCPTQGEAILPEEQDQNYVCKHTYVDRGWGNGCDLFGKGSLVTCAKFQCLESIEGKVVQHENLKYTVIITVHTGDQHQVGNETQGVTAEITPQASTVEAILPEYGTLGLECSPRTGLDFNEMILLTMKNKAWMVHRQWFFDLPLPWTSGATTETPTWNRKELLVTFKNAHAKKQEVVVLGSQEGWMHRALTGATEIQNSGGTSIWPGHLKCRLKMDKLELKGMSYAMCLNTFVLKKEVSETQHGTILIKVEYKGEDAPCKIPFSTEDGQGKAHNGRLITANPVVTKKEEPVNIEAEPPFGESNIVIGIGDKALKINWYKK

SEQ ID NO: 159 - protein, 392 aa, synthetic construct
  REGION 1..392: note = DENV3 sE SC.14 (I2-U6)
MRCVGVGNRDFVEGLSGATWVDVVLEHGGCVTTMAKNKPTLDIELQKTEATQLATLRKLCIEGKITNITTDSRCPTQGEAILPEEQDQNYVCKHTYVDRGWGNGCGLFGKGSLVTCAKFQCLESIEGKVVQHENLKYTVIITVHTGDQHQVGNETQGVTAEITPQASTVEAILPEYGTLGLECSPRTGLDFNEMILLTMKNKAWMVHRQWFFDLPLPWTSGATTETPTWNRKELLVTFKNAHAKKQEVVVLGSQEGWMHRALTGATEIQNSGGTSIWPGHLKCRLKMDKLELKGMSYAMCLNTFVLKKEVSETQHGTILIKVEYKGEDAPCKIPFSTEDGQGKAHNGRLITANPVVTKKEEPVNIEAEPPFGESNIVIGIGDKALKINWYKK

SEQ ID NO: 160 - protein, 392 aa, synthetic construct
  REGION 1..392: note = DENV3 sE UndPk6.1 (A278P)
MRCVGVGNRDFVEGLSGATWVDVVLEHGGCVTTMAKNKPTLDIELQKTEATQLATLRKLCIEGKITNITTDSRCPTQGEAILPEEQDQNYVCKHTYVDRGWGNGCGLFGKGSLVTCAKFQCLESIEGKVVQHENLKYTVIITVHTGDQHQVGNETQGVTAEITPQASTVEAILPEYGTLGLECSPRTGLDFNEMILLTMKNKAWMVHRQWFFDLPLPWTSGATTETPTWNRKELLVTFKNAHAKKQEVVVLGSQEGAMHTALTGATEIQNSGGTSIFPGHLKCRLKMDKLELKGMSYAMCLNTFVLKKEVSETQHGTILIKVEYKGEDAPCKIPFSTEDGQGKAHNGRLITANPVVTKKEEPVNIEAEPPFGESNIVIGIGDKALKINWYKK

SEQ ID NO: 161 - protein, 392 aa, synthetic construct
  REGION 1..392: note = DENV3 sE HCat3
MRCVGVGNRDFVEGLSGATWVDVVLEPGGCVTTMAKNKPTLDIELQKIEATQLATLRKLCIEGKITNITTDSRCPTQGEAILPEEQDQNYVCKHTYVDRGWGNGCGLFGKGSLVTCAKFQCLESIEGKVVQHENLKYTVIITVHTGDQHQVGNETQGVTAEITPQASTVEAILPEYGTLGLECSPRTGLDFNEMILLTMKNKAWMVHRQWFFDLPLPWTSGATTETPTWNRKELLVTFKNAHAKKQEVVVLGSQEGAMHTALTGATEIQNSGGTSIFAGHLKCRLKMDKLELKGMSYAMCLNTFVLKKEVSETQHGTILIKVEYKGEDAPCKIPFSTEDGQGKAHNGRLITANPVVTKKEEPVNIEAEPPFGESNIVIGIGDKALKINWYKK

SEQ ID NO: 162 - protein, 392 aa, synthetic construct
  REGION 1..392: note = DENV3 sE SC.12 (I2-I8-U6-P4)
MRCVGVGNRDFVEGLSGATWVDVVLEHGKCVTVMMKNKPTLDIELQKTEATQLATLRKLCIEGKITNITTDSRCPTQGEAILPEEQDQNYVCKHTYVDRGWGNGCDLFGKGSLVTCAKFQCLESIEGKVVQHENLKYTVIITVHTGDQHQVGNETQGVTAEITPQASTVEAILPEYGTLGLECSPRTGLDFNEMILLTMKNKAWMVHRQWFFDLPLPWTSGATTETPTWNRKELLVTFKNAHAKKQEVVVLGSQEGWMHRALTGATEIQNSGGTSIWPGHLKCRLKMDKLELKGMSYAMCLNTFVLKKEVSETQHGTILIKVEYKGEDAPCKIPFSTEDGQGKAHNGRLITANPVVTKKEEPVNIEAEPPFGESNIVIGIGDKALKINWYKK

SEQ ID NO: 163 - protein, 392 aa, synthetic construct
  REGION 1..392: note = DENV3 sE SC.29 (I8-U6-P4)
MRCVGVGNRDFVEGLSGATWVDVVLEHGKCVTVMMKNKPTLDIELQKTEATQLATLRKLCIEGKITNITTDSRCPTQGEAILPEEQDQNYVCKHTYVDRGWGNGCDLFGKGSLVTCAKFQCLESIEGKVVQHENLKYTVIITVHTGDQHQVGNETQGVTAEITPQASTVEAILPEYGTLGLECSPRTGLDFNEMILLTMKNKAWMVHRQWFFDLPLPWTSGATTETPTWNRKELLVTFKNAHAKKQEVVVLGSQEGAMHTALTGATEIQNSGGTSIWPGHLKCRLKMDKLELKGMSYAMCLNTFVLKKEVSETQHGTILIKVEYKGEDAPCKIPFSTEDGQGKAHNGRLITANPVVTKKEEPVNIEAEPPFGESNIVIGIGDKALKINWYKK

SEQ ID NO: 164 - protein, 392 aa, synthetic construct
  REGION 1..392: note = DENV3 sE SC.16 (I2-U6-H3)
MRCVGVGNRDFVEGLSGATWVDVVLEPGGCVTTMAKNKPTLDIELQKIEATQLATLRKLCIEGKITNITTDSRCPTQGEAILPEEQDQNYVCKHTYVDRGWGNGCGLFGKGSLVTCAKFQCLESIEGKVVQHENLKYTVIITVHTGDQHQVGNETQGVTAEITPQASTVEAILPEYGTLGLECSPRTGLDFNEMILLTMKNKAWMVHRQWFFDLPLPWTSGATTETPTWNRKELLVTFKNAHAKKQEVVVLGSQEGWMHRALTGATEIQNSGGTSIWPGHLKCRLKMDKLELKGMSYAMCLNTFVLKKEVSETQHGTILIKVEYKGEDAPCKIPFSTEDGQGKAHNGRLITANPVVTKKEEPVNIEAEPPFGESNIVIGIGDKALKINWYKK

SEQ ID NO: 165 - protein, 392 aa, synthetic construct
  REGION 1..392: note = DENV3 sE SC.11 (I2-I8-U6-H3)
MRCVGVGNRDFVEGLSGATWVDVVLEPGGCVTTMAKNKPTLDIELQKIEATQLATLRKLCIEGKITNITTDSRCPTQGEAILPEEQDQNYVCKHTYVDRGWGNGCDLFGKGSLVTCAKFQCLESIEGKVVQHENLKYTVIITVHTGDQHQVGNETQGVTAEITPQASTVEAILPEYGTLGLECSPRTGLDFNEMILLTMKNKAWMVHRQWFFDLPLPWTSGATTETPTWNRKELLVTFKNAHAKKQEVVVLGSQEGWMHRALTGATEIQNSGGTSIWPGHLKCRLKMDKLELKGMSYAMCLNTFVLKKEVSETQHGTILIKVEYKGEDAPCKIPFSTEDGQGKAHNGRLITANPVVTKKEEPVNIEAEPPFGESNIVIGIGDKALKINWYKK

SEQ ID NO: 166 - protein, 392 aa, synthetic construct
  REGION 1..392: note = DENV3 sE SC.15 (I8-U6)
MRCVGVGNRDFVEGLSGATWVDVVLEHGGCVTTMAKNKPTLDIELQKTEATQLATLRKLCIEGKITNITTDSRCPTQGEAILPEEQDQNYVCKHTYVDRGWGNGCDLFGKGSLVTCAKFQCLESIEGKVVQHENLKYTVIITVHTGDQHQVGNETQGVTAEITPQASTVEAILPEYGTLGLECSPRTGLDFNEMILLTMKNKAWMVHRQWFFDLPLPWTSGATTETPTWNRKELLVTFKNAHAKKQEVVVLGSQEGAMHTALTGATEIQNSGGTSIWPGHLKCRLKMDKLELKGMSYAMCLNTFVLKKEVSETQHGTILIKVEYKGEDAPCKIPFSTEDGQGKAHNGRLITANPVVTKKEEPVNIEAEPPFGESNIVIGIGDKALKINWYKK

SEQ ID NO: 167 - protein, 392 aa, synthetic construct
  REGION 1..392: note = DENV3 sE SC.23 (I2-I8)
MRCVGVGNRDFVEGLSGATWVDVVLEHGGCVTTMAKNKPTLDIELQKTEATQLATLRKLCIEGKITNITTDSRCPTQGEAILPEEQDQNYVCKHTYVDRGWGNGCDLFGKGSLVTCAKFQCLESIEGKVVQHENLKYTVIITVHTGDQHQVGNETQGVTAEITPQASTVEAILPEYGTLGLECSPRTGLDFNEMILLTMKNKAWMVHRQWFFDLPLPWTSGATTETPTWNRKELLVTFKNAHAKKQEVVVLGSQEGWMHRALTGATEIQNSGGTSIFAGHLKCRLKMDKLELKGMSYAMCLNTFVLKKEVSETQHGTILIKVEYKGEDAPCKIPFSTEDGQGKAHNGRLITANPVVTKKEEPVNIEAEPPFGESNIVIGIGDKALKINWYKK

SEQ ID NO: 168 - protein, 392 aa, synthetic construct
  REGION 1..392: note = DENV3 sE SC.1 (I2-I8-P4)
MRCVGVGNRDFVEGLSGATWVDVVLEHGKCVTVMMKNKPTLDIELQKTEATQLATLRKLCIEGKITNITTDSRCPTQGEAILPEEQDQNYVCKHTYVDRGWGNGCDLFGKGSLVTCAKFQCLESIEGKVVQHENLKYTVIITVHTGDQHQVGNETQGVTAEITPQASTVEAILPEYGTLGLECSPRTGLDFNEMILLTMKNKAWMVHRQWFFDLPLPWTSGATTETPTWNRKELLVTFKNAHAKKQEVVVLGSQEGWMHRALTGATEIQNSGGTSIFAGHLKCRLKMDKLELKGMSYAMCLNTFVLKKEVSETQHGTILIKVEYKGEDAPCKIPFSTEDGQGKAHNGRLITANPVVTKKEEPVNIEAEPPFGESNIVIGIGDKALKINWYKK

SEQ ID NO: 169 - protein, 394 aa, synthetic construct
  REGION 1..394: note = DENV4 sE WT
MRCVGVGNRDFVEGVSGGAWVDLVLEHGGCVTTMAQGKPTLDFELTKTTAKEVALLRTYCIEASISNITTATRCPTQGEPYLKEEQDQQYICRRDVVDRGWGNGCGLFGKGGVVTCAKFSCSGKITGNLVQIENLEYTVVVTVHNGDTHAVGNDTSNHGVTAMITPRSPSVEVKLPDYGELTLDCEPRSGIDFNEMILMKMKKKTWLVHKQWFLDLPLPWTAGADTSEVHWNYKERMVTFKVPHAKRQDVTVLGSQEGAMHSALAGATEVDSGDGNHMFAGHLKCKVRMEKLRIKGMSYTMCSGKFSIDKEMAETQHGTTVVKVKYEGAGAPCKVPIEIRDVNKEKVVGRIISSTPLAENTNSVTNIELEPPFGDSYIVIGVGNSALTLHWFRK

SEQ ID NO: 170 - protein, 394 aa, synthetic construct
  REGION 1..394: note = DENV4 sE PM4
MRCVGVGNRDFVEGVSGGAWVDLVLEHGKCVTVMMQGKPTLDFELTKTTAKEVALLRTYCIEASISNITTATRCPTQGEPYLKEEQDQQYICRRDVVDRGWGNGCGLFGKGGVVTCAKFSCSGKITGNLVQIENLEYTVVVTVHNGDTHAVGNDTSNHGVTAMITPRSPSVEVKLPDYGELTLDCEPRSGIDFNEMILMKMKKKTWLVHKQWFLDLPLPWTAGADTSEVHWNYKERMVTFKVPHAKRQDVTVLGSQEGAMHSALAGATEVDSGDGNHMFAGHLKCKVRMEKLRIKGMSYTMCSGKFSIDKEMAETQHGTTVVKVKYEGAGAPCKVPIEIRDVNKEKVVGRIISSTPLAENTNSVTNIELEPPFGDSYIVIGVGNSALTLHWFRK

SEQ ID NO: 171 - protein, 394 aa, synthetic construct
  REGION 1..394: note = DENV4 sE IntFc2
MRCVGVGNRDFVEGVSGGAWVDLVLEHGGCVTTMAQGKPTLDFELTKTTAKEVALLRTYCIEASISNITTATRCPTQGEPYLKEEQDQQYICRRDVVDRGWGNGCGLFGKGGVVTCAKFSCSGKITGNLVQIENLEYTVVVTVHNGDTHAVGNDTSNHGVTAMITPRSPSVEVKLPDYGELTLDCEPRSGIDFNEMILMKMKKKTWLVHKQWFLDLPLPWTAGADTSEVHWNYKERMVTFKVPHAKRQDVTVLGSQEGWMHRALAGATEVDSGDGNHMFAGHLKCKVRMEKLRIKGMSYTMCSGKFSIDKEMAETQHGTTVVKVKYEGAGAPCKVPIEIRDVNKEKVVGRIISSTPLAENTNSVTNIELEPPFGDSYIVIGVGNSALTLHWFRK

SEQ ID NO: 172 - protein, 394 aa, synthetic construct
  REGION 1..394: note = DENV4 sE IntFc8
MRCVGVGNRDFVEGVSGGAWVDLVLEHGGCVTTMAQGKPTLDFELTKTTAKEVALLRTYCIEASISNITTATRCPTQGEPYLKEEQDQQYICRRDVVDRGWGNGCDLFGKGGVVTCAKFSCSGKITGNLVQIENLEYTVVVTVHNGDTHAVGNDTSNHGVTAMITPRSPSVEVKLPDYGELTLDCEPRSGIDFNEMILMKMKKKTWLVHKQWFLDLPLPWTAGADTSEVHWNYKERMVTFKVPHAKRQDVTVLGSQEGAMHSALAGATEVDSGDGNHMFAGHLKCKVRMEKLRIKGMSYTMCSGKFSIDKEMAETQHGTTVVKVKYEGAGAPCKVPIEIRDVNKEKVVGRIISSTPLAENTNSVTNIELEPPFGDSYIVIGVGNSALTLHWFRK

SEQ ID NO: 173 - protein, 395 aa, synthetic construct
  REGION 1..395: note = DENV4 sE UndPk6
MRCVGVGNRDFVEGVSGGAWVDLVLEHGGCVTTMAQGKPTLDFELTKTTAKEVALLRTYCIEASISNITTATRCPTQGEPYLKEEQDQQYICRRDVVDRGWGNGCGLFGKGGVVTCAKFSCSGKITGNLVQIENLEYTVVVTVHNGDTHAVGNDTSNHGVTAMITPRSPSVEVKLPDYGELTLDCEPRSGIDFNEMILMKMKKKTWLVHKQWFLDLPLPWTAGADTSEVHWNYKERMVTFKVPHAKRQDVTVLGSQEGAMHSALAGATEVDSGDGNHMWPAGHLKCKVRMEKLRIKGMSYTMCSGKFSIDKEMAETQHGTTVVKVKYEGAGAPCKVPIEIRDVNKEKVVGRIISSTPLAENTNSVTNIELEPPFGDSYIVIGVGNSALTLHWFRK

SEQ ID NO: 174 - protein, 395 aa, synthetic construct
  REGION 1..395: note = DENV4 sE SC.12 (I2-I8-U6-P4)
MRCVGVGNRDFVEGVSGGAWVDLVLEHGKCVTVMMQGKPTLDFELTKTTAKEVALLRTYCIEASISNITTATRCPTQGEPYLKEEQDQQYICRRDVVDRGWGNGCDLFGKGGVVTCAKFSCSGKITGNLVQIENLEYTVVVTVHNGDTHAVGNDTSNHGVTAMITPRSPSVEVKLPDYGELTLDCEPRSGIDFNEMILMKMKKKTWLVHKQWFLDLPLPWTAGADTSEVHWNYKERMVTFKVPHAKRQDVTVLGSQEGWMHRALAGATEVDSGDGNHMWPAGHLKCKVRMEKLRIKGMSYTMCSGKFSIDKEMAETQHGTTVVKVKYEGAGAPCKVPIEIRDVNKEKVVGRIISSTPLAENTNSVTNIELEPPFGDSYIVIGVGNSALTLHWFRK

SEQ ID NO: 175 - protein, 394 aa, synthetic construct
  REGION 1..394: note = DENV4 sE UndPk6.1 (A280P)
MRCVGVGNRDFVEGVSGGAWVDLVLEHGGCVTTMAQGKPTLDFELTKTTAKEVALLRTYCIEASISNITTATRCPTQGEPYLKEEQDQQYICRRDVVDRGWGNGCGLFGKGGVVTCAKFSCSGKITGNLVQIENLEYTVVVTVHNGDTHAVGNDTSNHGVTAMITPRSPSVEVKLPDYGELTLDCEPRSGIDFNEMILMKMKKKTWLVHKQWFLDLPLPWTAGADTSEVHWNYKERMVTFKVPHAKRQDVTVLGSQEGAMHSALAGATEVDSGDGNHMFPGHLKCKVRMEKLRIKGMSYTMCSGKFSIDKEMAETQHGTTVVKVKYEGAGAPCKVPIEIRDVNKEKVVGRIISSTPLAENTNSVTNIELEPPFGDSYIVIGVGNSALTLHWFRK

SEQ ID NO: 176 - protein, 394 aa, synthetic construct
  REGION 1..394: note = DENV4 sE HCat3
MRCVGVGNRDFVEGVSGGAWVDLVLEPGGCVTTMAQGKPTLDFELTKITAKEVALLRTYCIEASISNITTATRCPTQGEPYLKEEQDQQYICRRDVVDRGWGNGCGLFGKGGVVTCAKFSCSGKITGNLVQIENLEYTVVVTVHNGDTHAVGNDTSNHGVTAMITPRSPSVEVKLPDYGELTLDCEPRSGIDFNEMILMKMKKKTWLVHKQWFLDLPLPWTAGADTSEVHWNYKERMVTFKVPHAKRQDVTVLGSQEGAMHSALAGATEVDSGDGNHMFAGHLKCKVRMEKLRIKGMSYTMCSGKFSIDKEMAETQHGTTVVKVKYEGAGAPCKVPIEIRDVNKEKVVGRIISSTPLAENTNSVTNIELEPPFGDSYIVIGVGNSALTLHWFRK

SEQ ID NO: 177 - protein, 394 aa, synthetic construct
  REGION 1..394: note = DENV4 sE SC.1 (I2-I8-P4)
MRCVGVGNRDFVEGVSGGAWVDLVLEHGKCVTVMMQGKPTLDFELTKTTAKEVALLRTYCIEASISNITTATRCPTQGEPYLKEEQDQQYICRRDVVDRGWGNGCDLFGKGGVVTCAKFSCSGKITGNLVQIENLEYTVVVTVHNGDTHAVGNDTSNHGVTAMITPRSPSVEVKLPDYGELTLDCEPRSGIDFNEMILMKMKKKTWLVHKQWFLDLPLPWTAGADTSEVHWNYKERMVTFKVPHAKRQDVTVLGSQEGWMHRALAGATEVDSGDGNHMFAGHLKCKVRMEKLRIKGMSYTMCSGKFSIDKEMAETQHGTTVVKVKYEGAGAPCKVPIEIRDVNKEKVVGRIISSTPLAENTNSVTNIELEPPFGDSYIVIGVGNSALTLHWFRK

SEQ ID NO: 178 - protein, 404 aa, synthetic construct
  REGION 1..404: note = ZIKV sE WT
IRCIGVSNRDFVEGMSGGTWVDIVLEHGGCVTVMAQDKPTVDIELVTTTVSNMAEVRSYCYEASISDMASDSRCPTQGEAYLDKQSDTQYVCKRTLVDRGWGNGCGLFGKGSLVTCAKFACSKKMTGKSIQPENLEYRIMLSVHGSQHSGMIVNDTGHETDENRAKVEITPNSPRAEATLGGFGSLGLDCEPRTGLDFSDLYYLTMNNKHWLVHKEWFHDIPLPWHAGADTGTPHWNNKEALVEFKDAHAKRQTVVVLGSQEGAVHTALAGALEAEMDGAKGRLSSGHLKCRLKMDKLRLKGVSYSLCTAAFTFTKIPAETLHGTVTVEVQYAGTDGPCKVPAQMAVDMQTLTPVGRLITANPVITESTENSKMMLELDPPFGDSYIVIGVGEKKITHHWHRSG

SEQ ID NO: 179 - protein, 404 aa, synthetic construct
  REGION 1..404: note = ZIKV sE PM4
IRCIGVSNRDFVEGMSGGTWVDIVLEHGKCVTVMMQDKPTVDIELVTTTVSNMAEVRSYCYEASISDMASDSRCPTQGEAYLDKQSDTQYVCKRTLVDRGWGNGCGLFGKGSLVTCAKFACSKKMTGKSIQPENLEYRIMLSVHGSQHSGMIVNDTGHETDENRAKVEITPNSPRAEATLGGFGSLGLDCEPRTGLDFSDLYYLTMNNKHWLVHKEWFHDIPLPWHAGADTGTPHWNNKEALVEFKDAHAKRQTVVVLGSQEGAVHTALAGALEAEMDGAKGRLSSGHLKCRLKMDKLRLKGVSYSLCTAAFTFTKIPAETLHGTVTVEVQYAGTDGPCKVPAQMAVDMQTLTPVGRLITANPVITESTENSKMMLELDPPFGDSYIVIGVGEKKITHHWHRSG

SEQ ID NO: 180 - protein, 404 aa, synthetic construct
  REGION 1..404: note = ZIKV sE IntFc2
IRCIGVSNRDFVEGMSGGTWVDIVLEHGGCVTVMAQDKPTVDIELVTTTVSNMAEVRSYCYEASISDMASDSRCPTQGEAYLDKQSDTQYVCKRTLVDRGWGNGCGLFGKGSLVTCAKFACSKKMTGKSIQPENLEYRIMLSVHGSQHSGMIVNDTGHETDENRAKVEITPNSPRAEATLGGFGSLGLDCEPRTGLDFSDLYYLTMNNKHWLVHKEWFHDIPLPWHAGADTGTPHWNNKEALVEFKDAHAKRQTVVVLGSQEGWVHRALAGALEAEMDGAKGRLSSGHLKCRLKMDKLRLKGVSYSLCTAAFTFTKIPAETLHGTVTVEVQYAGTDGPCKVPAQMAVDMQTLTPVGRLITANPVITESTENSKMMLELDPPFGDSYIVIGVGEKKITHHWHRSG

SEQ ID NO: 181 - protein, 404 aa, synthetic construct
  REGION 1..404: note = ZIKV sE IntFc8
IRCIGVSNRDFVEGMSGGTWVDIVLEHGGCVTVMAQDKPTVDIELVTTTVSNMAEVRSYCYEASISDMASDSRCPTQGEAYLDKQSDTQYVCKRTLVDRGWGNGCDLFGKGSLVTCAKFACSKKMTGKSIQPENLEYRIMLSVHGSQHSGMIVNDTGHETDENRAKVEITPNSPRAEATLGGFGSLGLDCEPRTGLDFSDLYYLTMNNKHWLVHKEWFHDIPLPWHAGADTGTPHWNNKEALVEFKDAHAKRQTVVVLGSQEGAVHTALAGALEAEMDGAKGRLSSGHLKCRLKMDKLRLKGVSYSLCTAAFTFTKIPAETLHGTVTVEVQYAGTDGPCKVPAQMAVDMQTLTPVGRLITANPVITESTENSKMMLELDPPFGDSYIVIGVGEKKITHHWHRSG

SEQ ID NO: 182 - protein, 495 aa, Dengue virus type 2
MRCIGMSNRDFVEGVSGGSWVDIVLEHGSCVTTMAKNKPTLDFELIKTEAKQPATLRKYCIEAKLTNTTTESRCPTQGEPSLNEEQDKRFVCKHSMVDRGWGNGCGLFGKGGIVTCAMFRCKKNMEGKVVQPENLEYTIVITPHSGEEHAVGNDTGKHGKEIKITPQSSITEAELTGYGTVTMECSPRTGLDFNEMVLLQMENKAWLVHRQWFLDLPLPWLPGADTQGSNWIQKETLVTFKNPHAKKQDVVVLGSQEGAMHTALTGATEIQMSSGNLLFTGHLKCRLRMDKLQLKGMSYSMCTGKFKVVKEIAETQHGTIVIRVQYEGDGSPCKIPFEIMDLEKRHVLGRLITVNPIVTEKDSPVNIEAEPPFGDSYIIIGVEPGQLKLNWFKKGSSIGQMFETTMRGAKRMAILGDTAWDFGSLGGVFTSIGKALHQVFGAIYGAAFSGVSWTMKILIGVIITWIGMNSRSTSLSVTLVLVGIVTLYLGVMVQA

SEQ ID NO: 183 - protein, 495 aa, Dengue virus type 1
MRCVGIGNRDFVEGLSGATWVDVVLEHGSCVTTMAKDKPTLDIELLKTEVTNPAVLRKLCIEAKISNTTTDSRCPTQGEATLVEEQDTNFVCRRTFVDRGWGNGCGLFGKGSLITCAKFKCVTKLEGKIVQYENLKYSVIVTVHTGDQHQVGNETTEHGTTATITPQAPTSEIQLTDYGALTLDCSPRTGLDFNEMVLLTMEKKSWLVHKQWFLDLPLPWTSGASTSQETWNRQDLLVTFKTAHAKKQEVVVLGSQEGAMHTALTGATEIQTSGTTTIFAGHLKCRLKMDKLTLKGMSYVMCTGSFKLEKEVAETQHGTVLVQVKYEGTDAPCKIPFSSQDEKGVTQNGRLITANPIVTDKEKPVNIEAEPPFGESYIVVGAGEKALKLSWFKKGSSIGKMFEATARGARRMAILGDTAWDFGSIGGVFTSVGKLIHQIFGTAYGVLFSGVSWTMKIGIGILLTWLGLNSRSTSLSMTCIAVGMVTLYLGVMVQA

SEQ ID NO: 184 - protein, 493 aa, Dengue virus type 3
MRCVGVGNRDFVEGLSGATWVDVVLEHGGCVTTMAKNKPTLDIELQKTEATQLATLRKLCIEGKITNITTDSRCPTQGEAILPEEQDQNYVCKHTYVDRGWGNGCGLFGKGSLVTCAKFQCLESIEGKVVQHENLKYTVIITVHTGDQHQVGNETQGVTAEITPQASTVEAILPEYGTLGLECSPRTGLDFNEMILLTMKNKAWMVHRQWFFDLPLPWTSGATTETPTWNRKELLVTFKNAHAKKQEVVVLGSQEGAMHTALTGATEIQNSGGTSIFAGHLKCRLKMDKLELKGMSYAMCLNTFVLKKEVSETQHGTILIKVEYKGEDAPCKIPFSTEDGQGKAHNGRLITANPVVTKKEEPVNIEAEPPFGESNIVIGIGDKALKINWYKKGSSIGKMFEATARGARRMAILGDTAWDFGSVGGVLNSLGKMVHQIFGSAYTALFSGVSWIMKIGIGVLLTWIGLNSKNTSMSFSCIAIGIITLYLGAVVQA

SEQ ID NO: 185 - protein, 558 aa, Dengue virus type 4
MAYMIGQTGIQRTVFFVLMMLVAPSYGMRCVGVGNRDFVEGVSGGAWVDLVLEHGGCVTTMAQGKPTLDFELTKTTAKEVALLRTYCIEASISNITTATRCPTQGEPYLKEEQDQQYICRRDVVDRGWGNGCGLFGKGGVVTCAKFSCSGKITGNLVQIENLEYTVVVTVHNGDTHAVGNDTSNHGVTAMITPRSPSVEVKLPDYGELTLDCEPRSGIDFNEMILMKMKKKTWLVHKQWFLDLPLPWTAGADTSEVHWNYKERMVTFKVPHAKRQDVTVLGSQEGAMHSALAGATEVDSGDGNHMFAGHLKCKVRMEKLRIKGMSYTMCSGKFSIDKEMAETQHGTTVVKVKYEGAGAPCKVPIEIRDVNKEKVVGRIISSTPLAENTNSVTNIELEPPFGDSYIVIGVGNSALTLHWFRKGSSIGKMFESTYRGAKRMAILGETAWDFGSVGGLFTSLGKAVHQVFGSVYTTMFGGVSWMIRILIGFLVLWIGTNSRNTSMAMTCIAVGGITLFLGFTVQADMGCVVSWSGKELKCGSGIFVVDNVHTWTEQYKFQP

SEQ ID NO: 186 - protein, 505 aa, Zika Virus
IRCIGVSNRDFVEGMSGGTWVDVVLEHGGCVTVMAQDKPTVDIELVTTTVSNMAEVRSYCYEASISDMASDSRCPTQGEAYLDKQSDTQYVCKRTLVDRGWGNGCGLFGKGSLVTCAKFACSKKMTGKSIQPENLEYRIMLSVHGSQHSGMIVNDTGHETDENRAKVEITPNSPRAEATLGGFGSLGLDCEPRTGLDFSDLYYLTMNNKHWLVHKEWFHDIPLPWHAGADTGTPHWNNKEALVEFKDAHAKRQTVVVLGSQEGAVHTALAGALEAEMDGAKGRLSSGHLKCRLKMDKLRLKGVSYSLCTAAFTFTKIPAETLHGTVTVEVQYAGTDGPCKVPAQMAVDMQTLTPVGRLITANPVITESTENSKMMLELDPPFGDSYIVIGVGEKKITHHWHRSGSTIGKAFEATVRGAKRMAVLGDTAWDFGSVGGALNSLGKGIHQIFGAAFKSLFGGMSWFSQILIGTLLMWLGLNTKNGSISLMCLALGGVLIFLSTAVSAD

SEQ ID NO: 187 - protein, 500 aa, Yellow fever virus
HGGTWVSATLEQDKCVTVMAPDKPSLDISLETVAIDRPAEVRKVCYNAVLTHVKINDKCPSTGEAHLAEENEGDNACKRTYSDRGWGNGCGLFGKGSIVACAKFTCAKSMSLFEVDQTKIQYVIRAQLHVGAKQENWTTDIKTLKFDALSGSQEVEFIGYGKATLECQVQTAVDFGNSYIAEMETESWIVDRQWAQDLTLPWQSGSGGVWREMHHLVEFEPPHAATIRVLALGNQEGSLKTALTGAMRVTKDTNDNNLYKLHGGHVSCRVKLSALTLKGTSYKICTDKMFFVKNPTDTGHGTVVMQVKVSKGAPCRIPVIVADDLTAAINKGILVTVNPIASTNDDEVLIEVNPPFGDSYIIVGRGDSRLTYQWHKEGSSIGKLFTQTMKGVERLAVMGDTAWDFSSAGGFFTSVGKGIHTVFGSAFQGLFGGLNWITKVIMGAVLIWVGINTRNMTMSMSMILVGVIMMFLSLGVGADQGCAINFGKRELKCGDGIFIF

SEQ ID NO: 188 - protein, 500 aa, Japanese encephalitis virus
FNCLGMGNRDFIEGASGATWVDLVLEGDSCLTIMANNKPTLDVRMINIEASQLAEVRSYCYHASVTDISTVARCPTTGEAHNEKRADSSYVCKQGFTDRGWGNGCGFFGKGSIDTCAKFSCTSKAIGRTIQPENIKYKVGIFVHGTTTSENHGNYSAQVGASQAAKFTVTPNAPSVALKLGDYGEVTLDCEPRSGLNTEAFYVMTVGSKSFLVHREWFHDLALPWTSPSSTAWRNRELLMEFEGAHATKQSVVALGSQEGGLHHALAGAIVVEYSSSVMLTSGHLKCRLKMDKLALKGTTYGMCTEKFSFAKNPVDTGHGTVVIELSYSGSDGPCKIPIVSVASLNDMTPVGRLVTVNPFVATSSANSKVLVEMEPPFGDSYIVVGRGAKQINHHWHKAGSTLGKAFSTTLKGAQRLAALGDTAWDFGSIGGVFNSIGRAVHQVFGGAFRTLFGGMSWITQGLMGALLLWMGVNARDRSIALAFLATGGVLVFLATNVHA

SEQ ID NO: 189 - protein, 501 aa, West Nile virus
FNCLGMSNRDFLEGVSGATWVDLVLEGDSCVTIMSKDKPTIDVKMMNMEAANLAEVRSYCYLATVSDLSTKAACPTMGEAHNDKRADPAFVCRQGVVDRGWGNGCGLFGKGSIDTCAKFACSTKAIGRTILKENIKYEVAIFVHGPTTVESHGNYSTQVGATQAGRLSITPAAPSYTLKLGEYGEVTVDCEPRSGIDTNAYYVMTVGTKTFLVHREWFMDLNLPWSSAGSTVWRNRETLMEFEEPHATKQSVIALGSQEGALHQALAGAIPVEFSSNTVKLTSGHLKCRVKMEKLQLKGTTYGVCSKAFKFLGTPADTGHGTVVLELQYTGTDGPCKVPISSVASLNDLTPVGRLVTVNPFVSVATANAKVLIELEPPFGDSYIVVGRGEQQINHHWHKSGSSIGKAFTTTLKGAQRLAALGDTAWDFGSVGGVFTSVGKAVHQVFGGAFRSLFGGMSWITQGLLGALLLWMGINARDRSIALTFLAVGGVLLFLSVNVHA

SEQ ID NO: 190 - protein, 496 aa, Tick-borne encephalitis virus
SRCTHLENRDFVTGTQGTTRVTLVLELGGCVTIIAEGKTSMDVWLDAIYQENPAKTREYCLHAKLSDTKVAARCPTMGPATLAEEHQGGTVCKRDQSDRGWGNHCGLFGKGSIVACVKAACEAKKKATGHVYDANKIVYTVKVEPHTGDYVAANETHSGRKTASFTISSEKTILTMGEYGDVSLLCRVASGVDLAQTVILELDKTVEHLPTAWQVHRDWFNDLALPWKHEGAQNWNNAERLVEFGAPHAVKMDVYNLGDQTGVLLKALAGVPVAHIEGTKYHLKSGHVTCEVGLEKLKMKGLTYTMCDKTKFTWKRAPTDSGHDTVVMEVTFSGTKPCRIPVRAVAHGSPDVNVAMLITPNPTIENNGGGFIEMQLPPGDNIIYVGELSHQWFQKGSSIGRVFQKTKKGIERLTVIGEHAWDFGSAGGFLSSIGKAVHTVLGGAFNSIFGGVVFLPKLLLGVALAWLGLNMRNPTMSMSFLLAGGLVLAMTLGVGA

SEQ ID NO: 191 - protein, 500 aa, Usutu virus
FNCLGMSNRDFLEGVSGATWVDVVLEGDSCITIMAKDKPTIDIKMMETEATNLAEVRSYCYLATVSDVSTVSNCPTTGEAHNPKRAEDTYVCKSGVTDRGWGNGCGLFGKGSIDTCANFTCSLKAVGRMIQPENVKYEVGIFIHGSTSSDTHGNYSSQLGASQAGRFTITPNSPAITVKMGDYGEISVECEPRNGLNTEAYYIMSVGTKHFLVHREWFNDLALPWTSPASSNWRNREILLEFEEPHATKQSVVALGSQEGALHQALAGAIPVSFSGSVKLTSGHLKCRVKMEKLTLKGTTYSMCTEKFSFAKNPADTGHGTVVLELQYTGSDGPCKIPISIVASLSDLTPIGRMVTANPYVASSEANAKVLVEMEPPFGDSYIVVGRGDKQINHHWHKAGSSIGKAFITTIKGAQRLAALGDTAWDFGSVGGIFNSVGKAVHQVFGGAFRTLFGGMSWITQGLMGALLLWMGVNARDRSIALVMLATGGVLLFLATNVHA

SEQ ID NO: 192 - protein, 497 aa, Powassan virus
TRCTHLENRDFVTGVQGTTRVSLVLELGGCVTITAEGKPSIDVWLEDIFQESPAETREYCLHAKLSNTKVEARCPTTGPATLPEEHQADMVCKRDQSDRGWGNHCGFFGKGSIVACAKFECEEAKKAVGHVYDSTKITYVVKAEPHTGDYQAANETNENRKTAQFTVASEKVILNLGDYGDVSLTCKVASGIDVAQTVVMSLGSSKDHLPSAWQVHRDWFEDLALPWKHKDNQDWNIVEKLVEFGPPHAVKMDIFNLGDQTAVLLKSLAGVPLASVDNQKYHLKSGHVTCDVGLEKLKLKGTTYSMCDKTKFKWKRVPVDSGHDTVVMEVSYTGSDKPCRIPVRAVAHGVPTTNVAMLITPNPTIETSGGGFIEMQLPLGDNIIYVGDLSQQWFQKGSTIGRMFEKTRKGLERLSVVGEHAWDFGSVGGILSSVGKAIHTVLGGAFNTLFGGVGFIPKMLLGVALVWLGLNARNPTMSMTFLAVGALTLMMTMGVGA